European Patent Specification EP 3 377 898 B1, published May 1, 2024. Title: THERMOSTABLE GLUCOSE BIOSENSORS AND USES THEREOF. Applicant: Duke University. The sequence listing filed with the application follows.

SEQUENCE LISTING (158 sequences)

SEQ ID NO: 1 - protein, 414 aa, Thermus thermophilus
MRKWLLAIGMVLGLSALAQGGKLEIFSWWAGDEGPALEALIRLYKQKYPGVEVINATVTGGAGVNARAVLKTRMLGGDPPDTFQVHAGMELIGTWVVANRMEDLSALFRQEGWLQAFPKGLIDLISYKGGIWSVPVNIHRSNVMWYLPAKLKEWGVNPPRTWDEFLATCQTLKQKGLEAPLALGENWTQQHLWESVALAVLGPDDWNNLWNGKLKFTDPKAVRAWEVFGRVLDCANKDAAGLSWQQAVDRVVQGKAAFNVMGDWAAGYMTTTLKLKPGTDFAWAPSPGTQGVFMMLSDSFGLPKGAKNRQNAINWLRLVGSKEGQDTFNPLKGSIAARLDSDPSKYNAYGQSAMRDWRSNRIVGSLVHGAVAPESFMSQFGTVMEIFLQTRNPQAAANAAQAIADQVGLGRLGQ

SEQ ID NO: 2 - protein, 411 aa, Thermus scotoductus
MRKWLLAIGVALGLSALAQTGKLEIFSWWAGDEGPALEALIRLYKQKYPGVEVINATVTGGAGVNAKAVLKTRMLGGDPPDTFQVHAGQELIGTWVVADRMEDLTSLFRQEGWLQAFPKGLIDLLSYKGGIWSVPVNIHRSNVMWYIPAKLKEWGVTPPKTWAEFLATCQTLKRKGLEAPLALGENWTQQHLWESVALATLGADGWNNLWSGKLKFTDPKAVAVWETFGKVLDCANKDAAGLSWQQAVDRVVQGKAAFNIMGDWAAGYMSTTLKLKPGTDFAWTPSPGTSGIFMMLSDSFGLPKGAKNRQNAINWLKLVGSKEGQDTFNPLKGSIAARLDSDPAKYNAYGQSAMKDWKSNRIVGSLVHGAVAPESFMSQFGTVMEIFLQSRNPQAAANAAQAIANQVGLGR

SEQ ID NO: 3 - protein, 413 aa, Deinococcus maricopensis
MKRIKAALLVTTAALLASSASAAGKLEIFSWWSGDEGPALEALVKLYKQKYPSVDVVNATVAGGAGTNAKAVLKTRMLGGDPPDSFQAHAGQELIGTWVVANRMEDLSSLFKSEGWTTKFPKDLLPLISSKGGIWSVPVNVHRSNVMWYIPANLKKWGVTAPKTWDQFLTTCKTLKTKNVTPLALGENWTQQHLWESVAVGTLGAQGWQNLWSGKLKFTDPKVVKVWDTFGKVLDCTNKDASGLSWQQATDRVVNGQAAFNIMGDWAAGYLSTTKKLKPGTGFGWAPSPSTSGTFIFLADSFGLPKGAKDRAEALSWLKLLGSKQGQDTFNPLKGSIAARVDSDLSKYSTYSQSAAKDWKSNKIVGSLTHGAVAPESFTSTFGTVIDAFVASRNAQVAAATTQQLADKAGLGK

SEQ ID NO: 4 - protein, 417 aa, Thermotoga neapolitana
MFFMRRFVGLFLMVVLLSAVVTASQLEIFSWWTAGGEAEALEALIKVFNKYYPDVEVINATVAGGAGTNAKAVLKTRILGGNPPDSFQVHAGMELIDTYVIPGYMTPITNLLEQWGVMDKFPKGILEMCSYEGEIYSIPVNVHRGNVVFYNKKIAEEIGMNEPPKTWDEFIMYLQKAKEKGYVGLALGDKNKWTALHLFETILLGVLGPNDYNGLWKGEVSFNDPRIRRAFEIMNKLLDYVNEDHAALAWQDATRLVYEGKALANVMGDWAEGYLKSVGWEPGKDFGWFAVPETQNAFMVVSDTFGLPKNAPHKENAVKWLKVVASVEGQDAFNPIKGSIPARLDADRSKYDIYLQWSMEDFATKALTPSIAHGSAAPEGFVTTLNDIINRFVTTRDIDSALEELLMAAEDEGYLVE

SEQ ID NO: 5 - protein, 411 aa, Kosmotoga olearia
MRKFFVLLMILSMAFVAFSANQLEIFSWWTGGGEEEGLLALFDVFHKYYPDVEIINATVAGGAGTNAKAVLKTRMLGGNPPDSFQVHGGMELIDTYVVTGMMEPITDLLEEWGIIDKFPEDILKICSYKGEVYSIPVNVHRGNVVFYNKAILEEVGIEKVPSTWPEFIEVLKKIKKAGYIPLALGDKNKWTATHLFEDILLSTLGPYNYNGLWNGRTSFEHQGVKEALEIFKELMNYVNPNHASLTWQDATLLVFEGKAAFNVMGDWAEGYLKTLGWTPGKEFGWMVVPGTKGSFMVVTDTFGLPKNAPHRENAIKWLKIISSVEGQDTFNPIKGSIPARIDADRSLYDDYLIWSMDDFATNALCPSIIHGSAAPEAFVTALNDTINMFITRKDVKKALKEIIYAAEDYLE

SEQ ID NO: 6 - protein, 436 aa, Xanthomonas campestris
MVKKWFALMIALSVLVIGLVACGSSEDSSNEPSEEPETSDSEEATGEASGTLEIFSWWTGAGEEDGLLALIELFEEKHPEIEVDNAAVAGGAGTNAKAVLTSRMQGNDPPGTFQVHGGAELNDSWVAAGQMDPLNDLFEAEGWADKFPEELIELVSKDGNIYSVPVNIHRGNVLWYNTEIFEEHGLEVPTTFEEFFDVADALQEAGVTPLALGDREPWAATHLFETVLLGTLGADDYNKLWSGEVGMDDPRVEEAAEIFIRMLDYVNEDHSSRNWQDASQLVAQGEAAMNVMGDWAKGYFVNDLNLAVKEDFGWAATPGTEGTFMVITDTFGLPTGVENPEVVKSFLAVLGSQEGQDAFNPLKGSIPARVDADVSKYDEYGQETIEDFKSAELSPSLAHGSAANEGFLTQVNQAINIFVTQKDVDSFVDSLKQYQP

SEQ ID NO: 7 - protein, 487 aa, Staphylothermus marinus
MSYSAITKSTAIIITLLVIIGILAGIAWWGWSRTPAPATTITTPPTTPTTTTTTTATPPQAELVIYHWWTAGGEREAINAVFQVFKQKYPNIQIVENPVAGGAGSVMKSVIIGLLAAGTPPDTFQVHAGAELKEYVDAGYLAPIDDIWSKLGLDKVIPSTLQVMCKFNGHYYAVPIDVHRSNVLWYNPKIFNELGIINKFGDPRNWSVDTLLQVARYIKQQRPDIAPIALASRNKWPVTHLFEVLLANAGGPETYVKFFTGKFNYNDPNDPVVQTVKKVLTVMATMAKEGLFNSNHPELTWDQAAALVAEGKAAMFIHGDWVAGYYIANNYKYGKDWAAAPFPKNIFILLSDAFELPKNAPHPEAAKDWLMVVGSKEAQEKFNLIKGSIPARTDVSPKYPDPYRPETAEDFQKSTLIPSAVHGGIAKEAFMTDLHNILTSMLTAVSVGTPVDNAVNTALAQILQSVKTSGLASFWKGYTIDYFITKR

SEQ ID NO: 8 - protein, 430 aa, Arthrobacter sp.
MRAPNKLRISLAVTAAASLIAVSGCAANTPAGSSSGGGTDKLEITSWWTSGSEADALNVLIDGVKAAKPGLSVDNAAVSGGGGANARQALAARLQAGSPPDAWQVHPAGQLKSYVDGGQVADLTDLWTEGDWASQMPKDVAEAQQVDGKYYTVPIGVHRGNVLWTNPAVLSKANVTIDADAGIDGLISSLEQVQASGTTPLCLGDKDIFASSQLLESLIMSRAGADNWTKLFTSEYSFDAPEVKQALEDYKTILSFANKDHSAITWDEAAKKMADGECAVNLMGDWAYGELLNAGKKPGTDFAWVAFPGKEDIFDYVGDGFSIPANNIPHAEAARAWLKTLMDPKIQTEFAAKKGSIPAVTSADISGLSEYQQEAAKSLASGAVVSSLAHAQAAGAEFAQTYADAVSTFNGSGNTDAFIASMTQAQKTQL

SEQ ID NO: 9 - protein, 400 aa, Artificial Sequence
  ttGBP1 (with signal peptide replaced with M and a HHHHHH at C-terminus)
MKLEIFSWWAGDEGPALEALIRLYKQKYPGVEVINATVTGGAGVNARAVLKTRMLGGDPPDTFQVHAGMELIGTWVVANRMEDLSALFRQEGWLQAFPKGLIDLISYKGGIWSVPVNIHRSNVMWYLPAKLKGWGVNPPRTWDKFLATAQTLKQKGLEAPLALGENWTQQHLWESVALAVLGPDDWNNLWNGKLKFTDPKAVRAWEVFGRVLDAANKDAAGLSWQQAVDRVVQGKAAFNIMGDWAAGYMTTTLKLKPGTDFAWAPSPGTQGVFMMLSDSFGLPKGAKNRQNAINWLRLVGSKEGQDTSNPLKGSIAARLDSDPSKYNAYGQSAMRDWRSNRIVGSLVHGAVAPESFMSQFGTVMEIFLQTRNPQAAANAAQAIADQVGLGRLGQHHHHHH

SEQ ID NO: 10 - protein, 400 aa, Artificial Sequence
  tsGBP2  (with signal peptide replaced with M and a GGSHHHHHH at C-terminus)
MKLEIFSWWAGDEGPALEALIRLYKQKYPGVEVINATVTGGAGVNAKAVLKTRMLGGDPPDTFQVHAGQELIGTWVVADRMEDLTSLFRQEGWLQAFPKGLIDLLSYKGGIWSVPVNIHRSNVMWYIPAKLKEWGVTPPKTWAEFLATAQTLKRKGLEAPLALGENWTQQHLWESVALATLGADGWNNLWSGKLKFTDPKAVAVWETFGKVLDAANKDAAGLSWQQAVDRVVQGKAAFNIMGDWAAGYMSTTLKLKPGTDFAWTPSPGTSGIFMMLSDSFGLPKGAKNRQNAINWLKLVGSKEGQDTFNPLKGSIAARLDSDPAKYNAYGQSAMKDWKSNRIVGSLVHGAVAPESFMSQFGTVMEIFLQSRNPQAAANAAQAIANQVGLGRGGSHHHHHH

SEQ ID NO: 11 - protein, 399 aa, Artificial Sequence
  dmGBP3 (with signal peptide replaced with M and a GGSHHHHHH at C-terminus)
MKLEIFSWWSGDEGPALEALVKLYKQKYPSVDVVNATVAGGAGTNAKAVLKTRMLGGDPPDSFQAHAGQELIGTWVVANRMEDLSSLFKSEGWTTKFPKDLLPLISSKGGIWSVPVNVHRSNVMWYIPANLKKWGVTAPKTWDQFLTTAKTLKTKNVTPLALGENWTQQHLWESVAVGTLGAQGWQNLWSGKLKFTDPKVVKVWDTFGKVLDATNKDASGLSWQQATDRVVNGQAAFNIMGDWAAGYLSTTKKLKPGTGFGWAPSPSTSGTFIFLADSFGLPKGAKDRAEALSWLKLLGSKQGQDTFNPLKGSIAARVDSDLSKYSTYSQSAAKDWKSNKIVGSLTHGAVAPESFTSTFGTVIDAFVASRNAQVAAATTQQLADKAGLGKGGSHHHHHH

SEQ ID NO: 12 - protein, 402 aa, Artificial Sequence
  tnGBP4 (with signal peptide replaced with M and a GGSHHHHHH at C-terminus)
MLEIFSWWTAGGEAEALEALIKVFNKYYPDVEVINATVAGGAGTNAKAVLKTRILGGNPPDSFQVHAGMELIDTYVIPGYMTPITNLLEQWGVMDKFPKGILEMASYEGEIYSIPVNVHRGNVVFYNKKIAEEIGMNEPPKTWDEFIMYLQKAKEKGYVGLALGDKNKWTALHLFETILLGVLGPNDYNGLWKGEVSFNDPRIRRAFEIMNKLLDYVNEDHAALAWQDATRLVYEGKALANVMGDWAEGYLKSVGWEPGKDFGWFAVPETQNAFMVVSDTFGLPKNAPHKENAVKWLKVVASVEGQDAFNPIKGSIPARLDADRSKYDIYLQWSMEDFATKALTPSIAHGSAAPEGFVTTLNDIINRFVTTRDIDSALEELLMAAEDEGYLVEGGSHHHHHH

SEQ ID NO: 13 - protein, 399 aa, Artificial Sequence
  koGBP5 (with signal peptide replaced with M and a GGSHHHHHH at C-terminus)
MLEIFSWWTGGGEEEGLLALFDVFHKYYPDVEIINATVAGGAGTNAKAVLKTRMLGGNPPDSFQVHGGMELIDTYVVTGMMEPITDLLEEWGIIDKFPEDILKIASYKGEVYSIPVNVHRGNVVFYNKAILEEVGIEKVPSTWPEFIEVLKKIKKAGYIPLALGDKNKWTATHLFEDILLSTLGPYNYNGLWNGRTSFEHQGVKEALEIFKELMNYVNPNHASLTWQDATLLVFEGKAAFNVMGDWAEGYLKTLGWTPGKEFGWMVVPGTKGSFMVVTDTFGLPKNAPHRENAIKWLKIISSVEGQDTFNPIKGSIPARIDADRSLYDDYLIWSMDDFATNALCPSIIHGSAAPEAFVTALNDTINMFITRKDVKKALKEIIYAAEDYLEGGSHHHHHH

SEQ ID NO: 14 - protein, 395 aa, Artificial Sequence
  bhGBP6 (with signal peptide replaced with M and a GGSHHHHHH at C-terminus)
MLEIFSWWTGAGEEDGLLALIELFEEKHPEIEVDNAAVAGGAGTNAKAVLTSRMQGNDPPGTFQVHGGAELNDSWVAAGQMDPLNDLFEAEGWADKFPEELIELVSKDGNIYSVPVNIHRGNVLWYNTEIFEEHGLEVPTTFEEFFDVADALQEAGVTPLALGDREPWAATHLFETVLLGTLGADDYNKLWSGEVGMDDPRVEEAAEIFIRMLDYVNEDHSSRNWQDASQLVAQGEAAMNVMGDWAKGYFVNDLNLAVKEDFGWAATPGTEGTFMVITDTFGLPTGVENPEVVKSFLAVLGSQEGQDAFNPLKGSIPARVDADVSKYDEYGQETIEDFKSAELSPSLAHGSAANEGFLTQVNQAINIFVTQKDVDSFVDSLKQYQPGGSHHHHHH

SEQ ID NO: 15 - protein, 436 aa, Artificial Sequence
  smGBP7 (with signal peptide replaced with M and a GGSHHHHHH at C-terminus)
MELVIYHWWTAGGEREAINAVFQVFKQKYPNIQIVENPVAGGAGSVMKSVIIGLLAAGTPPDTFQVHAGAELKEYVDAGYLAPIDDIWSKLGLDKVIPSTLQVMAKFNGHYYAVPIDVHRSNVLWYNPKIFNELGIINKFGDPRNWSVDTLLQVARYIKQQRPDIAPIALASRNKWPVTHLFEVLLANAGGPETYVKFFTGKFNYNDPNDPVVQTVKKVLTVMATMAKEGLFNSNHPELTWDQAAALVAEGKAAMFIHGDWVAGYYIANNYKYGKDWAAAPFPKNIFILLSDAFELPKNAPHPEAAKDWLMVVGSKEAQEKFNLIKGSIPARTDVSPKYPDPYRPETAEDFQKSTLIPSAVHGGIAKEAFMTDLHNILTSMLTAVSVGTPVDNAVNTALAQILQSVKTSGLASFWKGYTIDYFITKRGGSHHHHHH

SEQ ID NO: 16 - protein, 400 aa, Artificial Sequence
  asGBP8 (with signal peptide replaced with M and a GGSHHHHHH at C-terminus)
MKLEITSWWTSGSEADALNVLIDGVKAAKPGLSVDNAAVSGGGGANARQALAARLQAGSPPDAWQVHPAGQLKSYVDGGQVADLTDLWTEGDWASQMPKDVAEAQQVDGKYYTVPIGVHRGNVLWTNPAVLSKANVTIDADAGIDGLISSLEQVQASGTTPLALGDKDIFASSQLLESLIMSRAGADNWTKLFTSEYSFDAPEVKQALEDYKTILSFANKDHSAITWDEAAKKMADGEAAVNLMGDWAYGELLNAGKKPGTDFAWVAFPGKEDIFDYVGDGFSIPANNIPHAEAARAWLKTLMDPKIQTEFAAKKGSIPAVTSADISGLSEYQQEAAKSLASGAVVSSLAHAQAAGAEFAQTYADAVSTFNGSGNTDAFIASMTQAQKTQLGGSHHHHHH

SEQ ID NO: 17 - protein, 400 aa, Artificial Sequence
  tsGBP2_C8 (8C substitution mutant with signal peptide replaced with M and a GGSHHHHHH at C-terminus)
MKLEIFSCWAGDEGPALEALIRLYKQKYPGVEVINATVTGGAGVNAKAVLKTRMLGGDPPDTFQVHAGQELIGTWVVADRMEDLTSLFRQEGWLQAFPKGLIDLLSYKGGIWSVPVNIHRSNVMWYIPAKLKEWGVTPPKTWAEFLATAQTLKRKGLEAPLALGENWTQQHLWESVALATLGADGWNNLWSGKLKFTDPKAVAVWETFGKVLDAANKDAAGLSWQQAVDRVVQGKAAFNIMGDWAAGYMSTTLKLKPGTDFAWTPSPGTSGIFMMLSDSFGLPKGAKNRQNAINWLKLVGSKEGQDTFNPLKGSIAARLDSDPAKYNAYGQSAMKDWKSNRIVGSLVHGAVAPESFMSQFGTVMEIFLQSRNPQAAANAAQAIANQVGLGRGGSHHHHHH

SEQ ID NO: 18 - protein, 400 aa, Artificial Sequence
  tsGBP2_C9 (9C substitution mutant with signal peptide replaced with M and a GGSHHHHHH at C-terminus)
MKLEIFSWCAGDEGPALEALIRLYKQKYPGVEVINATVTGGAGVNAKAVLKTRMLGGDPPDTFQVHAGQELIGTWVVADRMEDLTSLFRQEGWLQAFPKGLIDLLSYKGGIWSVPVNIHRSNVMWYIPAKLKEWGVTPPKTWAEFLATAQTLKRKGLEAPLALGENWTQQHLWESVALATLGADGWNNLWSGKLKFTDPKAVAVWETFGKVLDAANKDAAGLSWQQAVDRVVQGKAAFNIMGDWAAGYMSTTLKLKPGTDFAWTPSPGTSGIFMMLSDSFGLPKGAKNRQNAINWLKLVGSKEGQDTFNPLKGSIAARLDSDPAKYNAYGQSAMKDWKSNRIVGSLVHGAVAPESFMSQFGTVMEIFLQSRNPQAAANAAQAIANQVGLGRGGSHHHHHH

SEQ ID NO: 19 - protein, 400 aa, Artificial Sequence
  tsGBP2_C12 (12C substitution mutant with signal peptide replaced with M and a GGSHHHHHH at C-terminus)
MKLEIFSWWAGCEGPALEALIRLYKQKYPGVEVINATVTGGAGVNAKAVLKTRMLGGDPPDTFQVHAGQELIGTWVVADRMEDLTSLFRQEGWLQAFPKGLIDLLSYKGGIWSVPVNIHRSNVMWYIPAKLKEWGVTPPKTWAEFLATAQTLKRKGLEAPLALGENWTQQHLWESVALATLGADGWNNLWSGKLKFTDPKAVAVWETFGKVLDAANKDAAGLSWQQAVDRVVQGKAAFNIMGDWAAGYMSTTLKLKPGTDFAWTPSPGTSGIFMMLSDSFGLPKGAKNRQNAINWLKLVGSKEGQDTFNPLKGSIAARLDSDPAKYNAYGQSAMKDWKSNRIVGSLVHGAVAPESFMSQFGTVMEIFLQSRNPQAAANAAQAIANQVGLGRGGSHHHHHH

SEQ ID NO: 20 - protein, 400 aa, Artificial Sequence
  tsGBP2_C13 (13C substitution mutant with signal peptide replaced with M and a GGSHHHHHH at C-terminus)
MKLEIFSWWAGDCGPALEALIRLYKQKYPGVEVINATVTGGAGVNAKAVLKTRMLGGDPPDTFQVHAGQELIGTWVVADRMEDLTSLFRQEGWLQAFPKGLIDLLSYKGGIWSVPVNIHRSNVMWYIPAKLKEWGVTPPKTWAEFLATAQTLKRKGLEAPLALGENWTQQHLWESVALATLGADGWNNLWSGKLKFTDPKAVAVWETFGKVLDAANKDAAGLSWQQAVDRVVQGKAAFNIMGDWAAGYMSTTLKLKPGTDFAWTPSPGTSGIFMMLSDSFGLPKGAKNRQNAINWLKLVGSKEGQDTFNPLKGSIAARLDSDPAKYNAYGQSAMKDWKSNRIVGSLVHGAVAPESFMSQFGTVMEIFLQSRNPQAAANAAQAIANQVGLGRGGSHHHHHH

SEQ ID NO: 21 - protein, 400 aa, Artificial Sequence
  tsGBP2_C41 (41C substitution mutant with signal peptide replaced with M and a GGSHHHHHH at C-terminus)
MKLEIFSWWAGDEGPALEALIRLYKQKYPGVEVINATVTGCAGVNAKAVLKTRMLGGDPPDTFQVHAGQELIGTWVVADRMEDLTSLFRQEGWLQAFPKGLIDLLSYKGGIWSVPVNIHRSNVMWYIPAKLKEWGVTPPKTWAEFLATAQTLKRKGLEAPLALGENWTQQHLWESVALATLGADGWNNLWSGKLKFTDPKAVAVWETFGKVLDAANKDAAGLSWQQAVDRVVQGKAAFNIMGDWAAGYMSTTLKLKPGTDFAWTPSPGTSGIFMMLSDSFGLPKGAKNRQNAINWLKLVGSKEGQDTFNPLKGSIAARLDSDPAKYNAYGQSAMKDWKSNRIVGSLVHGAVAPESFMSQFGTVMEIFLQSRNPQAAANAAQAIANQVGLGRGGSHHHHHH

SEQ ID NO: 22 - protein, 400 aa, Artificial Sequence
  tsGBP2_C42 (42C substitution mutant with signal peptide replaced with M and a GGSHHHHHH at C-terminus)
MKLEIFSWWAGDEGPALEALIRLYKQKYPGVEVINATVTGGCGVNAKAVLKTRMLGGDPPDTFQVHAGQELIGTWVVADRMEDLTSLFRQEGWLQAFPKGLIDLLSYKGGIWSVPVNIHRSNVMWYIPAKLKEWGVTPPKTWAEFLATAQTLKRKGLEAPLALGENWTQQHLWESVALATLGADGWNNLWSGKLKFTDPKAVAVWETFGKVLDAANKDAAGLSWQQAVDRVVQGKAAFNIMGDWAAGYMSTTLKLKPGTDFAWTPSPGTSGIFMMLSDSFGLPKGAKNRQNAINWLKLVGSKEGQDTFNPLKGSIAARLDSDPAKYNAYGQSAMKDWKSNRIVGSLVHGAVAPESFMSQFGTVMEIFLQSRNPQAAANAAQAIANQVGLGRGGSHHHHHH

SEQ ID NO: 23 - protein, 400 aa, Artificial Sequence
  tsGBP2_C64 (64C substitution mutant with signal peptide replaced with M and a GGSHHHHHH at C-terminus)
MKLEIFSWWAGDEGPALEALIRLYKQKYPGVEVINATVTGGAGVNAKAVLKTRMLGGDPPDTFCVHAGQELIGTWVVADRMEDLTSLFRQEGWLQAFPKGLIDLLSYKGGIWSVPVNIHRSNVMWYIPAKLKEWGVTPPKTWAEFLATAQTLKRKGLEAPLALGENWTQQHLWESVALATLGADGWNNLWSGKLKFTDPKAVAVWETFGKVLDAANKDAAGLSWQQAVDRVVQGKAAFNIMGDWAAGYMSTTLKLKPGTDFAWTPSPGTSGIFMMLSDSFGLPKGAKNRQNAINWLKLVGSKEGQDTFNPLKGSIAARLDSDPAKYNAYGQSAMKDWKSNRIVGSLVHGAVAPESFMSQFGTVMEIFLQSRNPQAAANAAQAIANQVGLGRGGSHHHHHH

SEQ ID NO: 24 - protein, 400 aa, Artificial Sequence
  tsGBP2_C66 (66C substitution mutant with signal peptide replaced with M and a GGSHHHHHH at C-terminus)
MKLEIFSWWAGDEGPALEALIRLYKQKYPGVEVINATVTGGAGVNAKAVLKTRMLGGDPPDTFQVCAGQELIGTWVVADRMEDLTSLFRQEGWLQAFPKGLIDLLSYKGGIWSVPVNIHRSNVMWYIPAKLKEWGVTPPKTWAEFLATAQTLKRKGLEAPLALGENWTQQHLWESVALATLGADGWNNLWSGKLKFTDPKAVAVWETFGKVLDAANKDAAGLSWQQAVDRVVQGKAAFNIMGDWAAGYMSTTLKLKPGTDFAWTPSPGTSGIFMMLSDSFGLPKGAKNRQNAINWLKLVGSKEGQDTFNPLKGSIAARLDSDPAKYNAYGQSAMKDWKSNRIVGSLVHGAVAPESFMSQFGTVMEIFLQSRNPQAAANAAQAIANQVGLGRGGSHHHHHH

SEQ ID NO: 25 - protein, 400 aa, Artificial Sequence
  tsGBP2_C119 (119C substitution mutant with signal peptide replaced with M and a GGSHHHHHH at C-terminus)
MKLEIFSWWAGDEGPALEALIRLYKQKYPGVEVINATVTGGAGVNAKAVLKTRMLGGDPPDTFQVHAGQELIGTWVVADRMEDLTSLFRQEGWLQAFPKGLIDLLSYKGGIWSVPVNICRSNVMWYIPAKLKEWGVTPPKTWAEFLATAQTLKRKGLEAPLALGENWTQQHLWESVALATLGADGWNNLWSGKLKFTDPKAVAVWETFGKVLDAANKDAAGLSWQQAVDRVVQGKAAFNIMGDWAAGYMSTTLKLKPGTDFAWTPSPGTSGIFMMLSDSFGLPKGAKNRQNAINWLKLVGSKEGQDTFNPLKGSIAARLDSDPAKYNAYGQSAMKDWKSNRIVGSLVHGAVAPESFMSQFGTVMEIFLQSRNPQAAANAAQAIANQVGLGRGGSHHHHHH

SEQ ID NO: 26 - protein, 400 aa, Artificial Sequence
  tsGBP2_C167 (167C substitution mutant with signal peptide replaced with M and a GGSHHHHHH at C-terminus)
MKLEIFSWWAGDEGPALEALIRLYKQKYPGVEVINATVTGGAGVNAKAVLKTRMLGGDPPDTFQVHAGQELIGTWVVADRMEDLTSLFRQEGWLQAFPKGLIDLLSYKGGIWSVPVNIHRSNVMWYIPAKLKEWGVTPPKTWAEFLATAQTLKRKGLEAPLALGENCTQQHLWESVALATLGADGWNNLWSGKLKFTDPKAVAVWETFGKVLDAANKDAAGLSWQQAVDRVVQGKAAFNIMGDWAAGYMSTTLKLKPGTDFAWTPSPGTSGIFMMLSDSFGLPKGAKNRQNAINWLKLVGSKEGQDTFNPLKGSIAARLDSDPAKYNAYGQSAMKDWKSNRIVGSLVHGAVAPESFMSQFGTVMEIFLQSRNPQAAANAAQAIANQVGLGRGGSHHHHHH

SEQ ID NO: 27 - protein, 400 aa, Artificial Sequence
  tsGBP2_C223 (223C substitution mutant with signal peptide replaced with M and a GGSHHHHHH at C-terminus)
MKLEIFSWWAGDEGPALEALIRLYKQKYPGVEVINATVTGGAGVNAKAVLKTRMLGGDPPDTFQVHAGQELIGTWVVADRMEDLTSLFRQEGWLQAFPKGLIDLLSYKGGIWSVPVNIHRSNVMWYIPAKLKEWGVTPPKTWAEFLATAQTLKRKGLEAPLALGENWTQQHLWESVALATLGADGWNNLWSGKLKFTDPKAVAVWETFGKVLDAANKDAAGLCWQQAVDRVVQGKAAFNIMGDWAAGYMSTTLKLKPGTDFAWTPSPGTSGIFMMLSDSFGLPKGAKNRQNAINWLKLVGSKEGQDTFNPLKGSIAARLDSDPAKYNAYGQSAMKDWKSNRIVGSLVHGAVAPESFMSQFGTVMEIFLQSRNPQAAANAAQAIANQVGLGRGGSHHHHHH

SEQ ID NO: 28 - protein, 400 aa, Artificial Sequence
  tsGBP2_C224 (224C substitution mutant with signal peptide replaced with M and a GGSHHHHHH at C-terminus)
MKLEIFSWWAGDEGPALEALIRLYKQKYPGVEVINATVTGGAGVNAKAVLKTRMLGGDPPDTFQVHAGQELIGTWVVADRMEDLTSLFRQEGWLQAFPKGLIDLLSYKGGIWSVPVNIHRSNVMWYIPAKLKEWGVTPPKTWAEFLATAQTLKRKGLEAPLALGENWTQQHLWESVALATLGADGWNNLWSGKLKFTDPKAVAVWETFGKVLDAANKDAAGLSCQQAVDRVVQGKAAFNIMGDWAAGYMSTTLKLKPGTDFAWTPSPGTSGIFMMLSDSFGLPKGAKNRQNAINWLKLVGSKEGQDTFNPLKGSIAARLDSDPAKYNAYGQSAMKDWKSNRIVGSLVHGAVAPESFMSQFGTVMEIFLQSRNPQAAANAAQAIANQVGLGRGGSHHHHHH

SEQ ID NO: 29 - protein, 400 aa, Artificial Sequence
  tsGBP2_C225 (225C substitution mutant with signal peptide replaced with M and a GGSHHHHHH at C-terminus)
MKLEIFSWWAGDEGPALEALIRLYKQKYPGVEVINATVTGGAGVNAKAVLKTRMLGGDPPDTFQVHAGQELIGTWVVADRMEDLTSLFRQEGWLQAFPKGLIDLLSYKGGIWSVPVNIHRSNVMWYIPAKLKEWGVTPPKTWAEFLATAQTLKRKGLEAPLALGENWTQQHLWESVALATLGADGWNNLWSGKLKFTDPKAVAVWETFGKVLDAANKDAAGLSWCQAVDRVVQGKAAFNIMGDWAAGYMSTTLKLKPGTDFAWTPSPGTSGIFMMLSDSFGLPKGAKNRQNAINWLKLVGSKEGQDTFNPLKGSIAARLDSDPAKYNAYGQSAMKDWKSNRIVGSLVHGAVAPESFMSQFGTVMEIFLQSRNPQAAANAAQAIANQVGLGRGGSHHHHHH

SEQ ID NO: 30 - protein, 400 aa, Artificial Sequence
  tsGBP2_C244 (244C substitution mutant with signal peptide replaced with M and a GGSHHHHHH at C-terminus)
MKLEIFSWWAGDEGPALEALIRLYKQKYPGVEVINATVTGGAGVNAKAVLKTRMLGGDPPDTFQVHAGQELIGTWVVADRMEDLTSLFRQEGWLQAFPKGLIDLLSYKGGIWSVPVNIHRSNVMWYIPAKLKEWGVTPPKTWAEFLATAQTLKRKGLEAPLALGENWTQQHLWESVALATLGADGWNNLWSGKLKFTDPKAVAVWETFGKVLDAANKDAAGLSWQQAVDRVVQGKAAFNIMGDCAAGYMSTTLKLKPGTDFAWTPSPGTSGIFMMLSDSFGLPKGAKNRQNAINWLKLVGSKEGQDTFNPLKGSIAARLDSDPAKYNAYGQSAMKDWKSNRIVGSLVHGAVAPESFMSQFGTVMEIFLQSRNPQAAANAAQAIANQVGLGRGGSHHHHHH

SEQ ID NO: 31 - protein, 400 aa, Artificial Sequence
  tsGBP2_C277 (cysteine substitution mutant with signal peptide replaced with M and a GGSHHHHHH at C-terminus)
MKLEIFSWWAGDEGPALEALIRLYKQKYPGVEVINATVTGGAGVNAKAVLKTRMLGGDPPDTFQVHAGQELIGTWVVADRMEDLTSLFRQEGWLQAFPKGLIDLLSYKGGIWSVPVNIHRSNVMWYIPAKLKEWGVTPPKTWAEFLATAQTLKRKGLEAPLALGENWTQQHLWESVALATLGADGWNNLWSGKLKFTDPKAVAVWETFGKVLDAANKDAAGLSWQQAVDRVVQGKAAFNIMGDWAAGYMSTTLKLKPGTDFAWTPSPGTSGIFMMLCDSFGLPKGAKNRQNAINWLKLVGSKEGQDTFNPLKGSIAARLDSDPAKYNAYGQSAMKDWKSNRIVGSLVHGAVAPESFMSQFGTVMEIFLQSRNPQAAANAAQAIANQVGLGRGGSHHHHHH

SEQ ID NO: 32 - protein, 400 aa, Artificial Sequence
  tsGBP2_C278 (278C substitution mutant with signal peptide replaced with M and a GGSHHHHHH at C-terminus)
MKLEIFSWWAGDEGPALEALIRLYKQKYPGVEVINATVTGGAGVNAKAVLKTRMLGGDPPDTFQVHAGQELIGTWVVADRMEDLTSLFRQEGWLQAFPKGLIDLLSYKGGIWSVPVNIHRSNVMWYIPAKLKEWGVTPPKTWAEFLATAQTLKRKGLEAPLALGENWTQQHLWESVALATLGADGWNNLWSGKLKFTDPKAVAVWETFGKVLDAANKDAAGLSWQQAVDRVVQGKAAFNIMGDWAAGYMSTTLKLKPGTDFAWTPSPGTSGIFMMLSCSFGLPKGAKNRQNAINWLKLVGSKEGQDTFNPLKGSIAARLDSDPAKYNAYGQSAMKDWKSNRIVGSLVHGAVAPESFMSQFGTVMEIFLQSRNPQAAANAAQAIANQVGLGRGGSHHHHHH

SEQ ID NO: 33 - protein, 400 aa, Artificial Sequence
  tsGBP2_C312 (312C substitution mutant with signal peptide replaced with M and a GGSHHHHHH at C-terminus)
MKLEIFSWWAGDEGPALEALIRLYKQKYPGVEVINATVTGGAGVNAKAVLKTRMLGGDPPDTFQVHAGQELIGTWVVADRMEDLTSLFRQEGWLQAFPKGLIDLLSYKGGIWSVPVNIHRSNVMWYIPAKLKEWGVTPPKTWAEFLATAQTLKRKGLEAPLALGENWTQQHLWESVALATLGADGWNNLWSGKLKFTDPKAVAVWETFGKVLDAANKDAAGLSWQQAVDRVVQGKAAFNIMGDWAAGYMSTTLKLKPGTDFAWTPSPGTSGIFMMLSDSFGLPKGAKNRQNAINWLKLVGSKEGQDTFNPLCGSIAARLDSDPAKYNAYGQSAMKDWKSNRIVGSLVHGAVAPESFMSQFGTVMEIFLQSRNPQAAANAAQAIANQVGLGRGGSHHHHHH

SEQ ID NO: 34 - protein, 400 aa, Artificial Sequence
  tsGBP2_C337 (337C substitution mutant with signal peptide replaced with M and a GGSHHHHHH at C-terminus)
MKLEIFSWWAGDEGPALEALIRLYKQKYPGVEVINATVTGGAGVNAKAVLKTRMLGGDPPDTFQVHAGQELIGTWVVADRMEDLTSLFRQEGWLQAFPKGLIDLLSYKGGIWSVPVNIHRSNVMWYIPAKLKEWGVTPPKTWAEFLATAQTLKRKGLEAPLALGENWTQQHLWESVALATLGADGWNNLWSGKLKFTDPKAVAVWETFGKVLDAANKDAAGLSWQQAVDRVVQGKAAFNIMGDWAAGYMSTTLKLKPGTDFAWTPSPGTSGIFMMLSDSFGLPKGAKNRQNAINWLKLVGSKEGQDTFNPLKGSIAARLDSDPAKYNAYGQSAMKDCKSNRIVGSLVHGAVAPESFMSQFGTVMEIFLQSRNPQAAANAAQAIANQVGLGRGGSHHHHHH

SEQ ID NO: 35 - protein, 400 aa, Artificial Sequence
  tsGBP2_C348 (348C substitution mutant with signal peptide replaced with M and a GGSHHHHHH at C-terminus)
MKLEIFSWWAGDEGPALEALIRLYKQKYPGVEVINATVTGGAGVNAKAVLKTRMLGGDPPDTFQVHAGQELIGTWVVADRMEDLTSLFRQEGWLQAFPKGLIDLLSYKGGIWSVPVNIHRSNVMWYIPAKLKEWGVTPPKTWAEFLATAQTLKRKGLEAPLALGENWTQQHLWESVALATLGADGWNNLWSGKLKFTDPKAVAVWETFGKVLDAANKDAAGLSWQQAVDRVVQGKAAFNIMGDWAAGYMSTTLKLKPGTDFAWTPSPGTSGIFMMLSDSFGLPKGAKNRQNAINWLKLVGSKEGQDTFNPLKGSIAARLDSDPAKYNAYGQSAMKDWKSNRIVGSLVCGAVAPESFMSQFGTVMEIFLQSRNPQAAANAAQAIANQVGLGRGGSHHHHHH

SEQ ID NO: 36 - protein, 400 aa, Artificial Sequence
  tsGBP2_C357 (357C substitution mutant with signal peptide replaced with M and a GGSHHHHHH at C-terminus)
MKLEIFSWWAGDEGPALEALIRLYKQKYPGVEVINATVTGGAGVNAKAVLKTRMLGGDPPDTFQVHAGQELIGTWVVADRMEDLTSLFRQEGWLQAFPKGLIDLLSYKGGIWSVPVNIHRSNVMWYIPAKLKEWGVTPPKTWAEFLATAQTLKRKGLEAPLALGENWTQQHLWESVALATLGADGWNNLWSGKLKFTDPKAVAVWETFGKVLDAANKDAAGLSWQQAVDRVVQGKAAFNIMGDWAAGYMSTTLKLKPGTDFAWTPSPGTSGIFMMLSDSFGLPKGAKNRQNAINWLKLVGSKEGQDTFNPLKGSIAARLDSDPAKYNAYGQSAMKDWKSNRIVGSLVHGAVAPESFCSQFGTVMEIFLQSRNPQAAANAAQAIANQVGLGRGGSHHHHHH

SEQ ID NO: 37 - protein, 400 aa, Artificial Sequence
  tsGBP2.13C.W8F (13C, 8F double substitution mutant)
MKLEIFSFWAGDCGPALEALIRLYKQKYPGVEVINATVTGGAGVNAKAVLKTRMLGGDPPDTFQVHAGQELIGTWVVADRMEDLTSLFRQEGWLQAFPKGLIDLLSYKGGIWSVPVNIHRSNVMWYIPAKLKEWGVTPPKTWAEFLATAQTLKRKGLEAPLALGENWTQQHLWESVALATLGADGWNNLWSGKLKFTDPKAVAVWETFGKVLDAANKDAAGLSWQQAVDRVVQGKAAFNIMGDWAAGYMSTTLKLKPGTDFAWTPSPGTSGIFMMLSDSFGLPKGAKNRQNAINWLKLVGSKEGQDTFNPLKGSIAARLDSDPAKYNAYGQSAMKDWKSNRIVGSLVHGAVAPESFMSQFGTVMEIFLQSRNPQAAANAAQAIANQVGLGRGGSHHHHHH

SEQ ID NO: 38 - protein, 400 aa, Artificial Sequence
  tsGBP2.13C.W8M (13C, 8M double substitution mutant with signal peptide replaced with M and a GGSHHHHHH at C-terminus)
MKLEIFSMWAGDCGPALEALIRLYKQKYPGVEVINATVTGGAGVNAKAVLKTRMLGGDPPDTFQVHAGQELIGTWVVADRMEDLTSLFRQEGWLQAFPKGLIDLLSYKGGIWSVPVNIHRSNVMWYIPAKLKEWGVTPPKTWAEFLATAQTLKRKGLEAPLALGENWTQQHLWESVALATLGADGWNNLWSGKLKFTDPKAVAVWETFGKVLDAANKDAAGLSWQQAVDRVVQGKAAFNIMGDWAAGYMSTTLKLKPGTDFAWTPSPGTSGIFMMLSDSFGLPKGAKNRQNAINWLKLVGSKEGQDTFNPLKGSIAARLDSDPAKYNAYGQSAMKDWKSNRIVGSLVHGAVAPESFMSQFGTVMEIFLQSRNPQAAANAAQAIANQVGLGRGGSHHHHHH

SEQ ID NO: 39 - protein, 400 aa, Artificial Sequence
  tsGBP2.13C.W8Y (13C, 8Y double substitution mutant with signal peptide replaced with M and a GGSHHHHHH at C-terminus)
MKLEIFSYWAGDCGPALEALIRLYKQKYPGVEVINATVTGGAGVNAKAVLKTRMLGGDPPDTFQVHAGQELIGTWVVADRMEDLTSLFRQEGWLQAFPKGLIDLLSYKGGIWSVPVNIHRSNVMWYIPAKLKEWGVTPPKTWAEFLATAQTLKRKGLEAPLALGENWTQQHLWESVALATLGADGWNNLWSGKLKFTDPKAVAVWETFGKVLDAANKDAAGLSWQQAVDRVVQGKAAFNIMGDWAAGYMSTTLKLKPGTDFAWTPSPGTSGIFMMLSDSFGLPKGAKNRQNAINWLKLVGSKEGQDTFNPLKGSIAARLDSDPAKYNAYGQSAMKDWKSNRIVGSLVHGAVAPESFMSQFGTVMEIFLQSRNPQAAANAAQAIANQVGLGRGGSHHHHHH

SEQ ID NO: 40 - protein, 400 aa, Artificial Sequence
  tsGBP2.13C.W9F (13C 9F double substitution mutant with signal peptide replaced with M and a GGSHHHHHH at C-terminus)
MKLEIFSWFAGDCGPALEALIRLYKQKYPGVEVINATVTGGAGVNAKAVLKTRMLGGDPPDTFQVHAGQELIGTWVVADRMEDLTSLFRQEGWLQAFPKGLIDLLSYKGGIWSVPVNIHRSNVMWYIPAKLKEWGVTPPKTWAEFLATAQTLKRKGLEAPLALGENWTQQHLWESVALATLGADGWNNLWSGKLKFTDPKAVAVWETFGKVLDAANKDAAGLSWQQAVDRVVQGKAAFNIMGDWAAGYMSTTLKLKPGTDFAWTPSPGTSGIFMMLSDSFGLPKGAKNRQNAINWLKLVGSKEGQDTFNPLKGSIAARLDSDPAKYNAYGQSAMKDWKSNRIVGSLVHGAVAPESFMSQFGTVMEIFLQSRNPQAAANAAQAIANQVGLGRGGSHHHHHH

SEQ ID NO: 41 - protein, 400 aa, Artificial Sequence
  tsGBP2.13C.W9M (13C 9M double substitution mutant with signal peptide replaced with M and a GGSHHHHHH at C-terminus)
MKLEIFSWMAGDCGPALEALIRLYKQKYPGVEVINATVTGGAGVNAKAVLKTRMLGGDPPDTFQVHAGQELIGTWVVADRMEDLTSLFRQEGWLQAFPKGLIDLLSYKGGIWSVPVNIHRSNVMWYIPAKLKEWGVTPPKTWAEFLATAQTLKRKGLEAPLALGENWTQQHLWESVALATLGADGWNNLWSGKLKFTDPKAVAVWETFGKVLDAANKDAAGLSWQQAVDRVVQGKAAFNIMGDWAAGYMSTTLKLKPGTDFAWTPSPGTSGIFMMLSDSFGLPKGAKNRQNAINWLKLVGSKEGQDTFNPLKGSIAARLDSDPAKYNAYGQSAMKDWKSNRIVGSLVHGAVAPESFMSQFGTVMEIFLQSRNPQAAANAAQAIANQVGLGRGGSHHHHHH

SEQ ID NO: 42 - protein, 400 aa, Artificial Sequence
  tsGBP2.13C.W9Y (13C, 9Y double substitution mutant with signal peptide replaced with M and a GGSHHHHHH at C-terminus)
MKLEIFSWYAGDCGPALEALIRLYKQKYPGVEVINATVTGGAGVNAKAVLKTRMLGGDPPDTFQVHAGQELIGTWVVADRMEDLTSLFRQEGWLQAFPKGLIDLLSYKGGIWSVPVNIHRSNVMWYIPAKLKEWGVTPPKTWAEFLATAQTLKRKGLEAPLALGENWTQQHLWESVALATLGADGWNNLWSGKLKFTDPKAVAVWETFGKVLDAANKDAAGLSWQQAVDRVVQGKAAFNIMGDWAAGYMSTTLKLKPGTDFAWTPSPGTSGIFMMLSDSFGLPKGAKNRQNAINWLKLVGSKEGQDTFNPLKGSIAARLDSDPAKYNAYGQSAMKDWKSNRIVGSLVHGAVAPESFMSQFGTVMEIFLQSRNPQAAANAAQAIANQVGLGRGGSHHHHHH

SEQ ID NO: 43 - protein, 400 aa, Artificial Sequence
  tsGBP2.13C.Q64N (13C, 64N double substitution mutant with signal peptide replaced with M and a GGSHHHHHH at C-terminus)
MKLEIFSWWAGDCGPALEALIRLYKQKYPGVEVINATVTGGAGVNAKAVLKTRMLGGDPPDTFNVHAGQELIGTWVVADRMEDLTSLFRQEGWLQAFPKGLIDLLSYKGGIWSVPVNIHRSNVMWYIPAKLKEWGVTPPKTWAEFLATAQTLKRKGLEAPLALGENWTQQHLWESVALATLGADGWNNLWSGKLKFTDPKAVAVWETFGKVLDAANKDAAGLSWQQAVDRVVQGKAAFNIMGDWAAGYMSTTLKLKPGTDFAWTPSPGTSGIFMMLSDSFGLPKGAKNRQNAINWLKLVGSKEGQDTFNPLKGSIAARLDSDPAKYNAYGQSAMKDWKSNRIVGSLVHGAVAPESFMSQFGTVMEIFLQSRNPQAAANAAQAIANQVGLGRGGSHHHHHH

SEQ ID NO: 44 - protein, 400 aa, Artificial Sequence
  tsGBP2.13C.Q64E (13C, 64E double substitution mutant with signal peptide replaced with M and a GGSHHHHHH at C-terminus)
MKLEIFSWWAGDCGPALEALIRLYKQKYPGVEVINATVTGGAGVNAKAVLKTRMLGGDPPDTFEVHAGQELIGTWVVADRMEDLTSLFRQEGWLQAFPKGLIDLLSYKGGIWSVPVNIHRSNVMWYIPAKLKEWGVTPPKTWAEFLATAQTLKRKGLEAPLALGENWTQQHLWESVALATLGADGWNNLWSGKLKFTDPKAVAVWETFGKVLDAANKDAAGLSWQQAVDRVVQGKAAFNIMGDWAAGYMSTTLKLKPGTDFAWTPSPGTSGIFMMLSDSFGLPKGAKNRQNAINWLKLVGSKEGQDTFNPLKGSIAARLDSDPAKYNAYGQSAMKDWKSNRIVGSLVHGAVAPESFMSQFGTVMEIFLQSRNPQAAANAAQAIANQVGLGRGGSHHHHHH

SEQ ID NO: 45 - protein, 400 aa, Artificial Sequence
  tsGBP2.13C.Q64M (13C, 64M double substitution mutant with signal peptide replaced with M and a GGSHHHHHH at C-terminus)
MKLEIFSWWAGDCGPALEALIRLYKQKYPGVEVINATVTGGAGVNAKAVLKTRMLGGDPPDTFMVHAGQELIGTWVVADRMEDLTSLFRQEGWLQAFPKGLIDLLSYKGGIWSVPVNIHRSNVMWYIPAKLKEWGVTPPKTWAEFLATAQTLKRKGLEAPLALGENWTQQHLWESVALATLGADGWNNLWSGKLKFTDPKAVAVWETFGKVLDAANKDAAGLSWQQAVDRVVQGKAAFNIMGDWAAGYMSTTLKLKPGTDFAWTPSPGTSGIFMMLSDSFGLPKGAKNRQNAINWLKLVGSKEGQDTFNPLKGSIAARLDSDPAKYNAYGQSAMKDWKSNRIVGSLVHGAVAPESFMSQFGTVMEIFLQSRNPQAAANAAQAIANQVGLGRGGSHHHHHH

SEQ ID NO: 46 - protein, 400 aa, Artificial Sequence
  tsGBP2.13C.H66Q (13C, 66Q double substitution mutant with signal peptide replaced with M and a GGSHHHHHH at C-terminus)
MKLEIFSWWAGDCGPALEALIRLYKQKYPGVEVINATVTGGAGVNAKAVLKTRMLGGDPPDTFQVQAGQELIGTWVVADRMEDLTSLFRQEGWLQAFPKGLIDLLSYKGGIWSVPVNIHRSNVMWYIPAKLKEWGVTPPKTWAEFLATAQTLKRKGLEAPLALGENWTQQHLWESVALATLGADGWNNLWSGKLKFTDPKAVAVWETFGKVLDAANKDAAGLSWQQAVDRVVQGKAAFNIMGDWAAGYMSTTLKLKPGTDFAWTPSPGTSGIFMMLSDSFGLPKGAKNRQNAINWLKLVGSKEGQDTFNPLKGSIAARLDSDPAKYNAYGQSAMKDWKSNRIVGSLVHGAVAPESFMSQFGTVMEIFLQSRNPQAAANAAQAIANQVGLGRGGSHHHHHH

SEQ ID NO: 47 - protein, 400 aa, Artificial Sequence
  tsGBP2.13C.W244M (13C, 244M double substitution mutant with signal peptide replaced with M and a GGSHHHHHH at C-terminus)
MKLEIFSWWAGDCGPALEALIRLYKQKYPGVEVINATVTGGAGVNAKAVLKTRMLGGDPPDTFQVHAGQELIGTWVVADRMEDLTSLFRQEGWLQAFPKGLIDLLSYKGGIWSVPVNIHRSNVMWYIPAKLKEWGVTPPKTWAEFLATAQTLKRKGLEAPLALGENWTQQHLWESVALATLGADGWNNLWSGKLKFTDPKAVAVWETFGKVLDAANKDAAGLSWQQAVDRVVQGKAAFNIMGDMAAGYMSTTLKLKPGTDFAWTPSPGTSGIFMMLSDSFGLPKGAKNRQNAINWLKLVGSKEGQDTFNPLKGSIAARLDSDPAKYNAYGQSAMKDWKSNRIVGSLVHGAVAPESFMSQFGTVMEIFLQSRNPQAAANAAQAIANQVGLGRGGSHHHHHH

SEQ ID NO: 48 - protein, 400 aa, Artificial Sequence
  tsGBP2.13C.W244F (13C, 244F double substitution mutant with signal peptide replaced with M and a GGSHHHHHH at C-terminus)
MKLEIFSWWAGDCGPALEALIRLYKQKYPGVEVINATVTGGAGVNAKAVLKTRMLGGDPPDTFQVHAGQELIGTWVVADRMEDLTSLFRQEGWLQAFPKGLIDLLSYKGGIWSVPVNIHRSNVMWYIPAKLKEWGVTPPKTWAEFLATAQTLKRKGLEAPLALGENWTQQHLWESVALATLGADGWNNLWSGKLKFTDPKAVAVWETFGKVLDAANKDAAGLSWQQAVDRVVQGKAAFNIMGDFAAGYMSTTLKLKPGTDFAWTPSPGTSGIFMMLSDSFGLPKGAKNRQNAINWLKLVGSKEGQDTFNPLKGSIAARLDSDPAKYNAYGQSAMKDWKSNRIVGSLVHGAVAPESFMSQFGTVMEIFLQSRNPQAAANAAQAIANQVGLGRGGSHHHHHH

SEQ ID NO: 49 - protein, 400 aa, Artificial Sequence
  tsGBP2.13C.W244Y (13C, 244Y double substitution mutant with signal peptide replaced with M and a GGSHHHHHH at C-terminus)
MKLEIFSWWAGDCGPALEALIRLYKQKYPGVEVINATVTGGAGVNAKAVLKTRMLGGDPPDTFQVHAGQELIGTWVVADRMEDLTSLFRQEGWLQAFPKGLIDLLSYKGGIWSVPVNIHRSNVMWYIPAKLKEWGVTPPKTWAEFLATAQTLKRKGLEAPLALGENWTQQHLWESVALATLGADGWNNLWSGKLKFTDPKAVAVWETFGKVLDAANKDAAGLSWQQAVDRVVQGKAAFNIMGDYAAGYMSTTLKLKPGTDFAWTPSPGTSGIFMMLSDSFGLPKGAKNRQNAINWLKLVGSKEGQDTFNPLKGSIAARLDSDPAKYNAYGQSAMKDWKSNRIVGSLVHGAVAPESFMSQFGTVMEIFLQSRNPQAAANAAQAIANQVGLGRGGSHHHHHH

SEQ ID NO: 50 - protein, 400 aa, Artificial Sequence
  tsGBP2.13C.D278N (13C, 278N double substitution mutant with signal peptide replaced with M and a GGSHHHHHH at C-terminus)
MKLEIFSWWAGDCGPALEALIRLYKQKYPGVEVINATVTGGAGVNAKAVLKTRMLGGDPPDTFQVHAGQELIGTWVVADRMEDLTSLFRQEGWLQAFPKGLIDLLSYKGGIWSVPVNIHRSNVMWYIPAKLKEWGVTPPKTWAEFLATAQTLKRKGLEAPLALGENWTQQHLWESVALATLGADGWNNLWSGKLKFTDPKAVAVWETFGKVLDAANKDAAGLSWQQAVDRVVQGKAAFNIMGDWAAGYMSTTLKLKPGTDFAWTPSPGTSGIFMMLSNSFGLPKGAKNRQNAINWLKLVGSKEGQDTFNPLKGSIAARLDSDPAKYNAYGQSAMKDWKSNRIVGSLVHGAVAPESFMSQFGTVMEIFLQSRNPQAAANAAQAIANQVGLGRGGSHHHHHH

SEQ ID NO: 51 - protein, 400 aa, Artificial Sequence
  tsGBP2.13C.D278S (13C, 278S double substitution mutant with signal peptide replaced with M and a GGSHHHHHH at C-terminus)
MKLEIFSWWAGDCGPALEALIRLYKQKYPGVEVINATVTGGAGVNAKAVLKTRMLGGDPPDTFQVHAGQELIGTWVVADRMEDLTSLFRQEGWLQAFPKGLIDLLSYKGGIWSVPVNIHRSNVMWYIPAKLKEWGVTPPKTWAEFLATAQTLKRKGLEAPLALGENWTQQHLWESVALATLGADGWNNLWSGKLKFTDPKAVAVWETFGKVLDAANKDAAGLSWQQAVDRVVQGKAAFNIMGDWAAGYMSTTLKLKPGTDFAWTPSPGTSGIFMMLSSSFGLPKGAKNRQNAINWLKLVGSKEGQDTFNPLKGSIAARLDSDPAKYNAYGQSAMKDWKSNRIVGSLVHGAVAPESFMSQFGTVMEIFLQSRNPQAAANAAQAIANQVGLGRGGSHHHHHH

SEQ ID NO: 52 - protein, 400 aa, Artificial Sequence
  tsGBP2.13C.D278L (13C, 278L double substitution mutant with signal peptide replaced with M and a GGSHHHHHH at C-terminus)
MKLEIFSWWAGDCGPALEALIRLYKQKYPGVEVINATVTGGAGVNAKAVLKTRMLGGDPPDTFQVHAGQELIGTWVVADRMEDLTSLFRQEGWLQAFPKGLIDLLSYKGGIWSVPVNIHRSNVMWYIPAKLKEWGVTPPKTWAEFLATAQTLKRKGLEAPLALGENWTQQHLWESVALATLGADGWNNLWSGKLKFTDPKAVAVWETFGKVLDAANKDAAGLSWQQAVDRVVQGKAAFNIMGDWAAGYMSTTLKLKPGTDFAWTPSPGTSGIFMMLSLSFGLPKGAKNRQNAINWLKLVGSKEGQDTFNPLKGSIAARLDSDPAKYNAYGQSAMKDWKSNRIVGSLVHGAVAPESFMSQFGTVMEIFLQSRNPQAAANAAQAIANQVGLGRGGSHHHHHH

SEQ ID NO: 53 - protein, 400 aa, Artificial Sequence
  tsGBP2.13C.K312M (13C, 312M double substitution mutant with signal peptide replaced with M and a GGSHHHHHH at C-terminus)
MKLEIFSWWAGDCGPALEALIRLYKQKYPGVEVINATVTGGAGVNAKAVLKTRMLGGDPPDTFQVHAGQELIGTWVVADRMEDLTSLFRQEGWLQAFPKGLIDLLSYKGGIWSVPVNIHRSNVMWYIPAKLKEWGVTPPKTWAEFLATAQTLKRKGLEAPLALGENWTQQHLWESVALATLGADGWNNLWSGKLKFTDPKAVAVWETFGKVLDAANKDAAGLSWQQAVDRVVQGKAAFNIMGDWAAGYMSTTLKLKPGTDFAWTPSPGTSGIFMMLSDSFGLPKGAKNRQNAINWLKLVGSKEGQDTFNPLMGSIAARLDSDPAKYNAYGQSAMKDWKSNRIVGSLVHGAVAPESFMSQFGTVMEIFLQSRNPQAAANAAQAIANQVGLGRGGSHHHHHH

SEQ ID NO: 54 - protein, 424 aa, Artificial Sequence
  tsGBP2.13C.bZif (13C substitution mutant, with bZif fusion, signal peptide replaced with M and a GGSHHHHHH at C-terminus)
MKLEIFSWWAGDCGPALEALIRLYKQKYPGVEVINATVTGGAGVNAKAVLKTRMLGGDPPDTFQVHAGQELIGTWVVADRMEDLTSLFRQEGWLQAFPKGLIDLLSYKGGIWSVPVNIHRSNVMWYIPAKLKEWGVTPPKTWAEFLATAQTLKRKGLEAPLALGENWTQQHLWESVALATLGADGWNNLWSGKLKFTDPKAVAVWETFGKVLDAANKDAAGLSWQQAVDRVVQGKAAFNIMGDWAAGYMSTTLKLKPGTDFAWTPSPGTSGIFMMLSDSFGLPKGAKNRQNAINWLKLVGSKEGQDTFNPLKGSIAARLDSDPAKYNAYGQSAMKDWKSNRIVGSLVHGAVAPESFMSQFGTVMEIFLQSRNPQAAANAAQAIANQVGLGRGGSGGSTGEKPYKCPECGKSFSRSGGSHHHHHH

SEQ ID NO: 55 - protein, 424 aa, Artificial Sequence
  tsGBP2.244C.bZif  (244C substitution mutant, with bZif fusion with signal peptide replaced with M and a GGSHHHHHH at C-terminus)
MKLEIFSWWAGDEGPALEALIRLYKQKYPGVEVINATVTGGAGVNAKAVLKTRMLGGDPPDTFQVHAGQELIGTWVVADRMEDLTSLFRQEGWLQAFPKGLIDLLSYKGGIWSVPVNIHRSNVMWYIPAKLKEWGVTPPKTWAEFLATAQTLKRKGLEAPLALGENWTQQHLWESVALATLGADGWNNLWSGKLKFTDPKAVAVWETFGKVLDAANKDAAGLSWQQAVDRVVQGKAAFNIMGDCAAGYMSTTLKLKPGTDFAWTPSPGTSGIFMMLSDSFGLPKGAKNRQNAINWLKLVGSKEGQDTFNPLKGSIAARLDSDPAKYNAYGQSAMKDWKSNRIVGSLVHGAVAPESFMSQFGTVMEIFLQSRNPQAAANAAQAIANQVGLGRGGSGGSTGEKPYKCPECGKSFSRSGGSHHHHHH

SEQ ID NO: 56 - protein, 424 aa, Artificial Sequence
  tsGBP2.13C_244F.bZif  (13C, 244F double substitution mutant, with bZif fusion, signal peptide replaced with M and a GGSHHHHHH at C-terminus)
MKLEIFSWWAGDCGPALEALIRLYKQKYPGVEVINATVTGGAGVNAKAVLKTRMLGGDPPDTFQVHAGQELIGTWVVADRMEDLTSLFRQEGWLQAFPKGLIDLLSYKGGIWSVPVNIHRSNVMWYIPAKLKEWGVTPPKTWAEFLATAQTLKRKGLEAPLALGENWTQQHLWESVALATLGADGWNNLWSGKLKFTDPKAVAVWETFGKVLDAANKDAAGLSWQQAVDRVVQGKAAFNIMGDFAAGYMSTTLKLKPGTDFAWTPSPGTSGIFMMLSDSFGLPKGAKNRQNAINWLKLVGSKEGQDTFNPLKGSIAARLDSDPAKYNAYGQSAMKDWKSNRIVGSLVHGAVAPESFMSQFGTVMEIFLQSRNPQAAANAAQAIANQVGLGRGGSGGSTGEKPYKCPECGKSFSRSGGSHHHHHH

SEQ ID NO: 57 - DNA, 1604 bp, Artificial Sequence
  Exemplary ttGBP1 expression sequence, optimized using OrfOpt
gccagtaagcttcggtcacgcttgggactgccataggctggcccggtgatgccggccacgatgcgtccggcgtagaggatcgagatctcgatcccgcgaaattaatacgactcactatagggagaccacaacggtttccctctagaaataattttgtttaactttaagaaggagatataccatgaaattagaaattttttcttggtgggcaggtgatgaaggcccggccttagaggccttgatccgcttatataaacaaaaatacccgggtgtagaagtgattaatgcaaccgtgacaggcggtgcaggcgtcaatgcgcgggcagttctcaaaacccgtatgttaggcggtgatccaccagacaccttccaagtccatgctgggatggaattaatcggcacatgggtcgtcgcgaaccgcatggaggacctctcggcgctgtttcggcaggaaggctggcttcaggcattccctaaaggcctcatcgacctgatttcttataagggcgggatttggtccgtacctgtaaatatccaccggagtaacgtaatgtggtatctgccggcaaaattaaaaggctggggcgtaaacccaccacgtacttgggacaaatttcttgcgacggcgcagaccttaaagcaaaaaggtttagaggcaccactggccctcggggaaaattggacacagcagcacttgtgggagtcggtcgccttggcagtattgggtccagatgattggaataacttatggaacggcaaactcaagtttactgatccaaaagccgtccgtgcatgggaggtgttcggccgcgtcctcgacgcagctaataaagatgcagcaggcttgagctggcagcaagccgtcgatcgcgtcgtacaggggaaagccgcattcaacattatgggggattgggcggctgggtacatgactacgacgttaaaattaaaaccaggtacagatttcgcttgggccccatcaccaggtacccaaggcgtattcatgatgttaagtgactcattcggtctccctaaaggtgccaaaaatcgtcagaatgctattaactggctgcgtctcgtaggttcaaaggaagggcaagatacatctaaccctctcaaaggtagtattgcagcacgtcttgacagcgacccttcgaagtataacgcctatggccaatcggcaatgcgtgactggcgcagtaaccgtatcgtagggtccctcgttcacggcgccgttgcaccagaatcgtttatgagtcaattcggtaccgtaatggaaatcttcctccaaacccgcaatccacaagcagctgctaatgcagcacaggccatcgccgaccaagtaggcctcggtcgtttaggtcaacatcatcatcatcatcattaatgaaagggcgatatccagcacactggcggccgttactagtggatccggctgctaacaaagcccgaaaggaagctgagttggctgctgccaccgctgagcaataactagcataaccccttggggcctctaaacgggtcttgaggggttttttgctgaaaggaggaactatatccggagcgactcccacggcacgttggcaagctcggaattcggcgtaatc

SEQ ID NO: 58 - DNA, 1577 bp, Artificial Sequence
  Exemplary tsGBP2 expression sequence, optimized using OrfOpt
cggtcacgcttgggactgccataggctggcccggtgatgccggccacgatgcgtccggcgtagaggatcgagatctcgatcccgcgaaattaatacgactcactatagggagaccacaacggtttccctctagaaataattttgtttaactttaagaaggagatataccatgaaattagaaattttttcttggtgggcaggtgatgaaggcccagctctcgaagccttgatccggttgtataaacagaaatacccaggtgtagaggtcattaatgctaccgtcaccgggggtgccggtgtcaacgccaaagccgtccttaaaacgcgtatgctcggcggggacccaccagatacctttcaagtacatgcagggcaggagctgatcggcacatgggtcgtcgccgaccgtatggaagatcttacctcattgtttcggcaggagggctggcttcaagcgttcccaaaaggtttaatcgatctcctcagttacaaaggtggcatttggtcagtcccagtcaacatccaccgttctaacgtaatgtggtacatcccggcaaaattaaaagaatggggcgtgaccccgccaaaaacatgggcagaatttttagcgacagcgcaaacattaaagcggaaaggccttgaggcaccattggcactcggtgagaattggacacagcaacatctctgggaaagcgtcgccctcgccacactgggtgccgatggttggaataatctctggagtggtaagctcaaattcacggatccaaaagcagtcgccgtatgggaaacattcggtaaggtattagatgcagcgaacaaggatgcagccgggctttcatggcaacaagcagtagaccgtgtagtacaggggaaagctgcattcaatatcatgggggactgggcagcaggttacatgagtacgaccttaaaactgaagccaggtaccgacttcgcatggacaccttctccgggcacttcagggatctttatgatgctgtctgatagtttcggcttgccaaagggggcgaagaatcgtcaaaatgctattaactggttgaaactcgtcgggtcaaaagaggggcaggacaccttcaacccgctcaaaggttccatcgctgctcgtctcgattctgatcctgccaaatataatgcatacggccaaagtgcaatgaaggactggaagtcaaatcggatcgtaggctccctcgtccacggcgcagtcgcgccagaatccttcatgtcgcagtttgggacggtaatggagattttcttgcaatcccgtaacccgcaggcagccgctaatgccgcacaagctatcgccaatcaggtcggtttaggtcgtgggggttcacatcatcatcatcatcattaatgaaagggcgatatccagcacactggcggccgttactagtggatccggctgctaacaaagcccgaaaggaagctgagttggctgctgccaccgctgagcaataactagcataaccccttggggcctctaaacgggtcttgaggggttttttgctgaaaggaggaactatatccggagcgactcccacggcacgttggcaagctcg

SEQ ID NO: 59 - DNA, 1574 bp, Artificial Sequence
  Exemplary dmGBP3 expression sequence, optimized using OrfOpt
cggtcacgcttgggactgccataggctggcccggtgatgccggccacgatgcgtccggcgtagaggatcgagatctcgatcccgcgaaattaatacgactcactatagggagaccacaacggtttccctctagaaataattttgtttaactttaagaaggagatataccatgaaactcgaaatttttagttggtggtcaggtgacgaaggcccagcactcgaggcactcgtgaagttatataagcaaaagtatccatcggtagacgtggtcaatgcgacggtagcagggggcgcagggacaaatgcaaaagcggtgctgaaaactcgtatgctcgggggcgacccaccggattcattccaggcccacgccggccaagaattgatcgggacatgggtagtggcaaatcgtatggaagatttaagttccctgttcaaatccgaaggttggaccacaaaattcccaaaagatttattaccacttatctcttcgaaagggggcatctggtcagtcccagtaaacgtccatcgcagtaacgtcatgtggtacatcccggctaatctgaagaaatggggcgtgaccgcacctaaaacctgggaccagttcttaactaccgcgaagaccttgaagaccaagaacgtaactccattagcactcggggaaaactggactcaacaacacttatgggaatcagtggcggtcggtacattaggggcccagggttggcagaacttatggtcggggaagttaaagtttacagacccaaaggtggtgaaagtatgggacacattcggcaaggtcttggatgcaacaaacaaggatgcatcgggtctcagttggcagcaggcgacggaccgtgtagtaaatggccaggcagcgtttaacattatgggggattgggccgcaggttatctcagtacgaccaagaaattgaaaccggggacaggcttcggctgggcgccgtccccatcaacatcaggcacgttcattttcttggctgatagctttgggttgccgaaaggtgccaaggatcgcgcggaagccctctcatggttaaaacttttaggctcaaaacagggtcaggacacatttaatcctttaaagggcagtatcgcggctcgggtcgacagtgatttatctaaatactccacatatagccaatcggcagccaaggactggaagagcaataaaattgtggggtcgttgacgcatggggcagtcgcaccagaatcctttacttctacctttggcaccgtaatcgatgcctttgtagcaagtcggaatgctcaggtcgcagccgctactacacaacagctcgcagataaagccggtctgggcaaaggtggtagtcatcatcatcatcatcattaatgaaagggcgatatccagcacactggcggccgttactagtggatccggctgctaacaaagcccgaaaggaagctgagttggctgctgccaccgctgagcaataactagcataaccccttggggcctctaaacgggtcttgaggggttttttgctgaaaggaggaactatatccggagcgactcccacggcacgttggcaagctcg

SEQ ID NO: 60 - DNA, 1583 bp, Artificial Sequence
  Exemplary tnGBP4 expression sequence, optimized using OrfOpt
cggtcacgcttgggactgccataggctggcccggtgatgccggccacgatgcgtccggcgtagaggatcgagatctcgatcccgcgaaattaatacgactcactatagggagaccacaacggtttccctctagaaataattttgtttaactttaagaaggagatataccatgttagaaattttttcttggtggacagcaggtggcgaagccgaagccttagaagcactcattaaagtcttcaataagtactatccggatgtagaggtcatcaatgcgacagtcgcaggcggtgctggtactaacgccaaagcagtcttaaagacccgcattcttggtggtaaccctccggattcattccaagttcacgctggcatggaactcatcgacacatacgttattccaggttacatgacaccaatcaccaatctcttagagcaatggggcgtcatggacaagtttccgaaaggcattctcgagatggcttcctatgaaggcgaaatttactcaattccggtaaatgtacatcgcggtaatgtggtcttttacaataagaaaattgcagaggaaattggcatgaacgaaccaccaaaaacgtgggacgaatttatcatgtatctccagaaagccaaagagaaaggctatgtagggcttgcactgggtgacaagaataagtggacagccctccacctgttcgaaacaatcctcttaggcgtgttaggcccaaatgattataatggtctttggaaaggggaagttagctttaacgaccctcgtattcgccgcgcattcgaaattatgaacaagttgttggactacgtaaacgaagatcatgcagcactcgcctggcaggatgcaactcgtttagtatacgaaggcaaagccttggctaacgtcatgggtgattgggcggaggggtacttaaaaagcgtcgggtgggaaccgggtaaagatttcgggtggttcgccgtgccagaaacccaaaacgctttcatggtagtctccgatacgtttggtctcccgaaaaacgcacctcataaagaaaatgcagtaaaatggttaaaggtggtagcctcagtagagggccaggatgcatttaatcctatcaagggctcaattccggcccgtctcgacgcagaccgctcaaaatatgatatctacttgcaatggtccatggaagattttgccacgaaggcactcaccccaagcatcgcccatgggagtgcagccccggaaggttttgtaacaacattaaatgacattattaaccggtttgtaaccacccgcgatatcgactccgccctggaagaactgctcatggcagccgaggacgaagggtacttggtagaaggtggtagtcatcatcatcatcatcattaatgaaagggcgatatccagcacactggcggccgttactagtggatccggctgctaacaaagcccgaaaggaagctgagttggctgctgccaccgctgagcaataactagcataaccccttggggcctctaaacgggtcttgaggggttttttgctgaaaggaggaactatatccggagcgactcccacggcacgttggcaagctcg

SEQ ID NO: 61 - DNA, 1574 bp, Artificial Sequence
  Exemplary koGBP5 expression sequence, optimized using OrfOpt
cggtcacgcttgggactgccataggctggcccggtgatgccggccacgatgcgtccggcgtagaggatcgagatctcgatcccgcgaaattaatacgactcactatagggagaccacaacggtttccctctagaaataattttgtttaactttaagaaggagatataccatgttagaaatttttagttggtggacaggtggtggcgaagaagaagggctcttggctttattcgacgtattccacaaatactacccagatgtcgagatcatcaacgccaccgtcgctgggggtgcagggactaacgccaaggcagtattgaagactcgtatgttaggggggaacccgccagacagctttcaggtacacggcggcatggaactcatcgatacctacgtagtaacagggatgatggagccaattacagacttattagaggaatggggtattattgacaaatttccagaggatatcttgaaaattgcgtcctataaaggggaagtgtacagtattccagtcaacgtccatcgtggtaacgtcgtcttctacaataaagctatcctcgaagaggtcgggatcgaaaaggtgcctagtacatggccggaatttattgaagtcctcaaaaaaatcaagaaggcaggttatatccctcttgcattgggtgataagaataaatggactgcgacgcacctgttcgaggacattttactgtcaactctcggtccatacaattacaacggcctgtggaacggtcgtacgtcatttgaacatcagggcgtgaaggaggccttagagatcttcaaagaattgatgaactacgtaaacccaaatcatgcttcgctgacatggcaagacgccacgctcttggtatttgaaggtaaagcagcattcaacgttatgggcgattgggccgagggttatcttaaaacattagggtggaccccaggcaaagagttcggttggatggtagtcccgggtacgaaaggttctttcatggtagtcaccgacaccttcggtctgcctaaaaatgcgccacaccgcgagaacgcaatcaaatggttaaagatcatcagttccgtggaaggccaagacacattcaaccctatcaagggttcaattccagcacgtattgacgccgatcgcagcttgtacgatgactatctgatctggtctatggacgatttcgctacaaatgcgttgtgtcctagcattatccacgggtccgctgccccagaagccttcgttactgcgctcaacgatacgattaatatgttcatcacacgcaaggacgttaaaaaagcattaaaggaaattatctatgcagcagaagattatttagaaggtggtagtcatcatcatcatcatcattaatgaaagggcgatatccagcacactggcggccgttactagtggatccggctgctaacaaagcccgaaaggaagctgagttggctgctgccaccgctgagcaataactagcataaccccttggggcctctaaacgggtcttgaggggttttttgctgaaaggaggaactatatccggagcgactcccacggcacgttggcaagctcg

SEQ ID NO: 62 - DNA, 1562 bp, Artificial Sequence
  Exemplary bhGBP6 expression sequence, optimized using OrfOpt
cggtcacgcttgggactgccataggctggcccggtgatgccggccacgatgcgtccggcgtagaggatcgagatctcgatcccgcgaaattaatacgactcactatagggagaccacaacggtttccctctagaaataattttgtttaactttaagaaggagatataccatgttagaaatttttagttggtggacaggtgcaggcgaggaagacgggctcttagccctcattgaattattcgaggagaagcacccagagattgaggtcgacaacgccgcggtagccggtggggccgggaccaatgcaaaagccgtactgacatcgcggatgcaaggtaatgatccaccaggcacgtttcaggttcacggtggcgccgagctcaacgacagctgggtagcggccggccaaatggacccattgaacgatttattcgaagccgaggggtgggcggacaagttccctgaggagcttatcgaattggtctccaaggatggcaacatttatagcgtcccagtgaacattcaccggggtaacgttctctggtataacactgaaattttcgaggagcatggcttagaagtaccgacgacatttgaagaatttttcgatgtagcggacgccttacaagaagcaggtgtaacccctctggccttaggcgaccgcgaaccatgggccgccacacatttgttcgagaccgtattactcggcacactcggtgcagatgattataacaagctgtggagtggtgaagtaggcatggatgacccgcgtgtagaagaggcagcagagattttcatccgtatgctcgattatgttaatgaggaccacagtagtcgtaactggcaagacgcttcacaactcgtggcacagggggaagcagccatgaatgtgatgggcgattgggcgaaaggctactttgttaacgacctgaatctcgcggtaaaagaggattttggttgggcggccactccaggtacagaggggacattcatggtgatcacagacacattcggtttgccgaccggtgtagagaacccagaggtcgtcaaaagtttcctcgcggtcttaggctcacaagaaggccaggatgccttcaatccattaaaaggttccattccagctcgtgttgacgcagatgtttccaagtacgacgaatatggtcaagaaaccattgaagattttaagtccgcggagctgtcaccatcgctcgcgcacggcagtgcagcaaacgaggggttcttgacccaagtgaatcaggctatcaacatttttgtaacacagaaggacgtagattcattcgtagactcgttgaaacaatatcaaccaggtggtagtcatcatcatcatcatcattaatgaaagggcgatatccagcacactggcggccgttactagtggatccggctgctaacaaagcccgaaaggaagctgagttggctgctgccaccgctgagcaataactagcataaccccttggggcctctaaacgggtcttgaggggttttttgctgaaaggaggaactatatccggagcgactcccacggcacgttggcaagctcg

SEQ ID NO: 63 - DNA, 1685 bp, Artificial Sequence
  Exemplary smGBP7 expression sequence, optimized using OrfOpt
cggtcacgcttgggactgccataggctggcccggtgatgccggccacgatgcgtccggcgtagaggatcgagatctcgatcccgcgaaattaatacgactcactatagggagaccacaacggtttccctctagaaataattttgtttaactttaagaaggagatataccatggaattagtaatttatcattggtggacagcaggcggggaacgtgaggcaatcaacgccgtcttccaggtctttaagcaaaagtacccgaacattcaaatcgtggaaaatccagtagccggcggtgcaggctcggtcatgaagagtgtaattatcggcctcctcgccgcaggtaccccaccagacacatttcaggtacacgcaggtgcagagttaaaagagtatgtggacgccggttatctcgccccaatcgacgacatttggtcgaagctgggtctggacaaggtaatcccgagtaccctccaagtcatggcaaaatttaacgggcattactatgcagtcccaattgacgtgcaccggtccaatgtactctggtacaaccctaagatcttcaacgaactcggtatcatcaacaaattcggtgaccctcgtaactggtctgtagatacgctcctccaagtagcacgttacattaagcaacaacgccctgacatcgcaccaattgcactggcgtcgcgtaataagtggccagtaacgcatctcttcgaggtccttttagccaacgcaggcggtccagagacttacgtcaaattctttaccggtaaatttaattacaatgaccctaatgacccagttgtacagacagtaaagaaagtcctcaccgtgatggcgaccatggcaaaggaaggtttgtttaacagcaaccatccggaactcacctgggatcaagcagcagcgcttgtagctgaaggcaaggcagcaatgttcattcacggggattgggtcgccggctactatatcgccaataactataaatacggtaaggattgggctgcggcaccgttcccgaaaaacatcttcatcctgctttcagatgccttcgaattgccaaaaaacgcccctcaccctgaggccgccaaggattggctcatggttgtcggtagtaaggaagcacaagagaaattcaatctcatcaaggggtcgatcccagcacgcactgacgtctccccaaaatacccagatccgtaccggccagagacagcggaagacttccagaaatcaacattgattccttcagctgttcacggcggtatcgctaaagaagcctttatgacagatttacacaacattttgacatcgatgctgacggccgtctcggtaggtactccggtggacaatgcggtgaatacagcattagcccaaatccttcagtcagtaaaaacgtccggcttggcgtcgttttggaaaggttacacaattgactactttatcacaaagcgtggcggttctcatcatcatcatcatcattaatgaaagggcgatatccagcacactggcggccgttactagtggatccggctgctaacaaagcccgaaaggaagctgagttggctgctgccaccgctgagcaataactagcataaccccttggggcctctaaacgggtcttgaggggttttttgctgaaaggaggaactatatccggagcgactcccacggcacgttggcaagctcg

SEQ ID NO: 64 - DNA, 1577 bp, Artificial Sequence
  Exemplary asGBP8 expression sequence, optimized using OrfOpt
cggtcacgcttgggactgccataggctggcccggtgatgccggccacgatgcgtccggcgtagaggatcgagatctcgatcccgcgaaattaatacgactcactatagggagaccacaacggtttccctctagaaataattttgtttaactttaagaaggagatataccatgaaattagaaattacaagttggtggacttccgggagtgaggcagatgcccttaacgtactcatcgacggtgtcaaagccgcaaaaccgggtctcagcgtagacaacgcagcggtctcagggggcggcggcgccaacgcccgccaggcactcgcagcacgtctccaagcaggcagtccacctgacgcctggcaagttcatccagcaggtcaattaaagtcctatgtagacgggggccaggtggccgacctcactgatttatggactgaaggcgattgggcctcgcaaatgccgaaagacgtagccgaggcgcaacaggtagacggtaaatactacacagtaccaatcggtgtgcaccgcggtaatgtactctggacaaatccagccgtactcagcaaagcgaatgtaaccattgacgcagacgcgggtatcgacgggctcatctcttcattggaacaagtacaagcaagtgggactaccccgttggctttaggtgacaaagacattttcgcaagttcccagctgttagagtccctgattatgtcgcgggctggtgccgataactggacaaaactctttacaagtgagtattccttcgatgcaccagaagtcaaacaagcccttgaagactataaaacgatcctcagctttgcaaataaggaccatagcgccatcacctgggacgaggcagctaagaagatggccgacggtgaagccgcagtaaacttgatgggcgattgggcgtacggcgaactcttgaacgcagggaagaaaccagggaccgatttcgcatgggtggcatttccgggcaaagaggacatcttcgattatgtaggtgacggttttagtatcccggcaaacaatattccacacgcggaggcagctcgggcgtggctgaagaccttaatggatccaaaaatccaaaccgaatttgccgccaaaaaagggtcgattccagccgtcacaagtgccgacatttccggcctgagtgaataccagcaggaagctgccaaatctctcgccagtggtgccgtagtcagttctttagcgcatgcacaagcagccggtgcagagttcgcccaaacatacgcagatgcagtaagcactttcaacggtagcggcaatactgacgcgttcatcgcttccatgacccaggcccagaaaacacagttaggtggttcacatcatcatcatcatcattaatgaaagggcgatatccagcacactggcggccgttactagtggatccggctgctaacaaagcccgaaaggaagctgagttggctgctgccaccgctgagcaataactagcataaccccttggggcctctaaacgggtcttgaggggttttttgctgaaaggaggaactatatccggagcgactcccacggcacgttggcaagctcg

SEQ ID NO: 65 - DNA, 1577 bp, Artificial Sequence
  Exemplary tsGBP2_C8 expression sequence, optimized using OrfOpt
cggtcacgcttgggactgccataggctggcccggtgatgccggccacgatgcgtccggcgtagaggatcgagatctcgatcccgcgaaattaatacgactcactatagggagaccacaacggtttccctctagaaataattttgtttaactttaagaaggagatataccatgaaattagaaattttttcttgctgggcaggtgatgaaggcccagctctcgaagccttgatccggttgtataaacagaaatacccaggtgtagaggtcattaatgctaccgtcaccgggggtgccggtgtcaacgccaaagccgtccttaaaacgcgtatgctcggcggggacccaccagatacctttcaagtacatgcagggcaggagctgatcggcacatgggtcgtcgccgaccgtatggaagatcttacctcattgtttcggcaggagggctggcttcaagcgttcccaaaaggtttaatcgatctcctcagttacaaaggtggcatttggtcagtcccagtcaacatccaccgttctaacgtaatgtggtacatcccggcaaaattaaaagaatggggcgtgaccccgccaaaaacatgggcagaatttttagcgacagcgcaaacattaaagcggaaaggccttgaggcaccattggcactcggtgagaattggacacagcaacatctctgggaaagcgtcgccctcgccacactgggtgccgatggttggaataatctctggagtggtaagctcaaattcacggatccaaaagcagtcgccgtatgggaaacattcggtaaggtattagatgcagcgaacaaggatgcagccgggctttcatggcaacaagcagtagaccgtgtagtacaggggaaagctgcattcaatatcatgggggactgggcagcaggttacatgagtacgaccttaaaactgaagccaggtaccgacttcgcatggacaccttctccgggcacttcagggatctttatgatgctgtctgatagtttcggcttgccaaagggggcgaagaatcgtcaaaatgctattaactggttgaaactcgtcgggtcaaaagaggggcaggacaccttcaacccgctcaaaggttccatcgctgctcgtctcgattctgatcctgccaaatataatgcatacggccaaagtgcaatgaaggactggaagtcaaatcggatcgtaggctccctcgtccacggcgcagtcgcgccagaatccttcatgtcgcagtttgggacggtaatggagattttcttgcaatcccgtaacccgcaggcagccgctaatgccgcacaagctatcgccaatcaggtcggtttaggtcgtgggggttcacatcatcatcatcatcattaatgaaagggcgatatccagcacactggcggccgttactagtggatccggctgctaacaaagcccgaaaggaagctgagttggctgctgccaccgctgagcaataactagcataaccccttggggcctctaaacgggtcttgaggggttttttgctgaaaggaggaactatatccggagcgactcccacggcacgttggcaagctcg

SEQ ID NO: 66 - DNA, 1577 bp, Artificial Sequence
  Exemplary tsGBP2_C9 expression sequence, optimized using OrfOpt
cggtcacgcttgggactgccataggctggcccggtgatgccggccacgatgcgtccggcgtagaggatcgagatctcgatcccgcgaaattaatacgactcactatagggagaccacaacggtttccctctagaaataattttgtttaactttaagaaggagatataccatgaaattagaaattttttcttggtgcgcaggtgatgaaggcccagctctcgaagccttgatccggttgtataaacagaaatacccaggtgtagaggtcattaatgctaccgtcaccgggggtgccggtgtcaacgccaaagccgtccttaaaacgcgtatgctcggcggggacccaccagatacctttcaagtacatgcagggcaggagctgatcggcacatgggtcgtcgccgaccgtatggaagatcttacctcattgtttcggcaggagggctggcttcaagcgttcccaaaaggtttaatcgatctcctcagttacaaaggtggcatttggtcagtcccagtcaacatccaccgttctaacgtaatgtggtacatcccggcaaaattaaaagaatggggcgtgaccccgccaaaaacatgggcagaatttttagcgacagcgcaaacattaaagcggaaaggccttgaggcaccattggcactcggtgagaattggacacagcaacatctctgggaaagcgtcgccctcgccacactgggtgccgatggttggaataatctctggagtggtaagctcaaattcacggatccaaaagcagtcgccgtatgggaaacattcggtaaggtattagatgcagcgaacaaggatgcagccgggctttcatggcaacaagcagtagaccgtgtagtacaggggaaagctgcattcaatatcatgggggactgggcagcaggttacatgagtacgaccttaaaactgaagccaggtaccgacttcgcatggacaccttctccgggcacttcagggatctttatgatgctgtctgatagtttcggcttgccaaagggggcgaagaatcgtcaaaatgctattaactggttgaaactcgtcgggtcaaaagaggggcaggacaccttcaacccgctcaaaggttccatcgctgctcgtctcgattctgatcctgccaaatataatgcatacggccaaagtgcaatgaaggactggaagtcaaatcggatcgtaggctccctcgtccacggcgcagtcgcgccagaatccttcatgtcgcagtttgggacggtaatggagattttcttgcaatcccgtaacccgcaggcagccgctaatgccgcacaagctatcgccaatcaggtcggtttaggtcgtgggggttcacatcatcatcatcatcattaatgaaagggcgatatccagcacactggcggccgttactagtggatccggctgctaacaaagcccgaaaggaagctgagttggctgctgccaccgctgagcaataactagcataaccccttggggcctctaaacgggtcttgaggggttttttgctgaaaggaggaactatatccggagcgactcccacggcacgttggcaagctcg

SEQ ID NO: 67 - DNA, 1577 bp, Artificial Sequence
  Exemplary tsGBP2_C12 expression sequence, optimized using OrfOpt
cggtcacgcttgggactgccataggctggcccggtgatgccggccacgatgcgtccggcgtagaggatcgagatctcgatcccgcgaaattaatacgactcactatagggagaccacaacggtttccctctagaaataattttgtttaactttaagaaggagatataccatgaaattagaaattttttcttggtgggcaggttgcgaaggcccagctctcgaagccttgatccggttgtataaacagaaatacccaggtgtagaggtcattaatgctaccgtcaccgggggtgccggtgtcaacgccaaagccgtccttaaaacgcgtatgctcggcggggacccaccagatacctttcaagtacatgcagggcaggagctgatcggcacatgggtcgtcgccgaccgtatggaagatcttacctcattgtttcggcaggagggctggcttcaagcgttcccaaaaggtttaatcgatctcctcagttacaaaggtggcatttggtcagtcccagtcaacatccaccgttctaacgtaatgtggtacatcccggcaaaattaaaagaatggggcgtgaccccgccaaaaacatgggcagaatttttagcgacagcgcaaacattaaagcggaaaggccttgaggcaccattggcactcggtgagaattggacacagcaacatctctgggaaagcgtcgccctcgccacactgggtgccgatggttggaataatctctggagtggtaagctcaaattcacggatccaaaagcagtcgccgtatgggaaacattcggtaaggtattagatgcagcgaacaaggatgcagccgggctttcatggcaacaagcagtagaccgtgtagtacaggggaaagctgcattcaatatcatgggggactgggcagcaggttacatgagtacgaccttaaaactgaagccaggtaccgacttcgcatggacaccttctccgggcacttcagggatctttatgatgctgtctgatagtttcggcttgccaaagggggcgaagaatcgtcaaaatgctattaactggttgaaactcgtcgggtcaaaagaggggcaggacaccttcaacccgctcaaaggttccatcgctgctcgtctcgattctgatcctgccaaatataatgcatacggccaaagtgcaatgaaggactggaagtcaaatcggatcgtaggctccctcgtccacggcgcagtcgcgccagaatccttcatgtcgcagtttgggacggtaatggagattttcttgcaatcccgtaacccgcaggcagccgctaatgccgcacaagctatcgccaatcaggtcggtttaggtcgtgggggttcacatcatcatcatcatcattaatgaaagggcgatatccagcacactggcggccgttactagtggatccggctgctaacaaagcccgaaaggaagctgagttggctgctgccaccgctgagcaataactagcataaccccttggggcctctaaacgggtcttgaggggttttttgctgaaaggaggaactatatccggagcgactcccacggcacgttggcaagctcg

SEQ ID NO: 68 - DNA, 1577 bp, Artificial Sequence
  Exemplary tsGBP2_C13 expression sequence, optimized using OrfOpt
cggtcacgcttgggactgccataggctggcccggtgatgccggccacgatgcgtccggcgtagaggatcgagatctcgatcccgcgaaattaatacgactcactatagggagaccacaacggtttccctctagaaataattttgtttaactttaagaaggagatataccatgaaattagaaattttttcttggtgggcaggtgattgcggcccagctctcgaagccttgatccggttgtataaacagaaatacccaggtgtagaggtcattaatgctaccgtcaccgggggtgccggtgtcaacgccaaagccgtccttaaaacgcgtatgctcggcggggacccaccagatacctttcaagtacatgcagggcaggagctgatcggcacatgggtcgtcgccgaccgtatggaagatcttacctcattgtttcggcaggagggctggcttcaagcgttcccaaaaggtttaatcgatctcctcagttacaaaggtggcatttggtcagtcccagtcaacatccaccgttctaacgtaatgtggtacatcccggcaaaattaaaagaatggggcgtgaccccgccaaaaacatgggcagaatttttagcgacagcgcaaacattaaagcggaaaggccttgaggcaccattggcactcggtgagaattggacacagcaacatctctgggaaagcgtcgccctcgccacactgggtgccgatggttggaataatctctggagtggtaagctcaaattcacggatccaaaagcagtcgccgtatgggaaacattcggtaaggtattagatgcagcgaacaaggatgcagccgggctttcatggcaacaagcagtagaccgtgtagtacaggggaaagctgcattcaatatcatgggggactgggcagcaggttacatgagtacgaccttaaaactgaagccaggtaccgacttcgcatggacaccttctccgggcacttcagggatctttatgatgctgtctgatagtttcggcttgccaaagggggcgaagaatcgtcaaaatgctattaactggttgaaactcgtcgggtcaaaagaggggcaggacaccttcaacccgctcaaaggttccatcgctgctcgtctcgattctgatcctgccaaatataatgcatacggccaaagtgcaatgaaggactggaagtcaaatcggatcgtaggctccctcgtccacggcgcagtcgcgccagaatccttcatgtcgcagtttgggacggtaatggagattttcttgcaatcccgtaacccgcaggcagccgctaatgccgcacaagctatcgccaatcaggtcggtttaggtcgtgggggttcacatcatcatcatcatcattaatgaaagggcgatatccagcacactggcggccgttactagtggatccggctgctaacaaagcccgaaaggaagctgagttggctgctgccaccgctgagcaataactagcataaccccttggggcctctaaacgggtcttgaggggttttttgctgaaaggaggaactatatccggagcgactcccacggcacgttggcaagctcg

SEQ ID NO: 69 - DNA, 1577 bp, Artificial Sequence
  Exemplary tsGBP2_C41 expression sequence, optimized using OrfOpt
cggtcacgcttgggactgccataggctggcccggtgatgccggccacgatgcgtccggcgtagaggatcgagatctcgatcccgcgaaattaatacgactcactatagggagaccacaacggtttccctctagaaataattttgtttaactttaagaaggagatataccatgaaattagaaattttttcttggtgggcaggtgatgaaggcccagctctcgaagccttgatccggttgtataaacagaaatacccaggtgtagaggtcattaatgctaccgtcaccgggtgcgccggtgtcaacgccaaagccgtccttaaaacgcgtatgctcggcggggacccaccagatacctttcaagtacatgcagggcaggagctgatcggcacatgggtcgtcgccgaccgtatggaagatcttacctcattgtttcggcaggagggctggcttcaagcgttcccaaaaggtttaatcgatctcctcagttacaaaggtggcatttggtcagtcccagtcaacatccaccgttctaacgtaatgtggtacatcccggcaaaattaaaagaatggggcgtgaccccgccaaaaacatgggcagaatttttagcgacagcgcaaacattaaagcggaaaggccttgaggcaccattggcactcggtgagaattggacacagcaacatctctgggaaagcgtcgccctcgccacactgggtgccgatggttggaataatctctggagtggtaagctcaaattcacggatccaaaagcagtcgccgtatgggaaacattcggtaaggtattagatgcagcgaacaaggatgcagccgggctttcatggcaacaagcagtagaccgtgtagtacaggggaaagctgcattcaatatcatgggggactgggcagcaggttacatgagtacgaccttaaaactgaagccaggtaccgacttcgcatggacaccttctccgggcacttcagggatctttatgatgctgtctgatagtttcggcttgccaaagggggcgaagaatcgtcaaaatgctattaactggttgaaactcgtcgggtcaaaagaggggcaggacaccttcaacccgctcaaaggttccatcgctgctcgtctcgattctgatcctgccaaatataatgcatacggccaaagtgcaatgaaggactggaagtcaaatcggatcgtaggctccctcgtccacggcgcagtcgcgccagaatccttcatgtcgcagtttgggacggtaatggagattttcttgcaatcccgtaacccgcaggcagccgctaatgccgcacaagctatcgccaatcaggtcggtttaggtcgtgggggttcacatcatcatcatcatcattaatgaaagggcgatatccagcacactggcggccgttactagtggatccggctgctaacaaagcccgaaaggaagctgagttggctgctgccaccgctgagcaataactagcataaccccttggggcctctaaacgggtcttgaggggttttttgctgaaaggaggaactatatccggagcgactcccacggcacgttggcaagctcg

SEQ ID NO: 70 - DNA, 1577 bp, Artificial Sequence
  Exemplary tsGBP2_C42 expression sequence, optimized using OrfOpt
cggtcacgcttgggactgccataggctggcccggtgatgccggccacgatgcgtccggcgtagaggatcgagatctcgatcccgcgaaattaatacgactcactatagggagaccacaacggtttccctctagaaataattttgtttaactttaagaaggagatataccatgaaattagaaattttttcttggtgggcaggtgatgaaggcccagctctcgaagccttgatccggttgtataaacagaaatacccaggtgtagaggtcattaatgctaccgtcaccgggggttgcggtgtcaacgccaaagccgtccttaaaacgcgtatgctcggcggggacccaccagatacctttcaagtacatgcagggcaggagctgatcggcacatgggtcgtcgccgaccgtatggaagatcttacctcattgtttcggcaggagggctggcttcaagcgttcccaaaaggtttaatcgatctcctcagttacaaaggtggcatttggtcagtcccagtcaacatccaccgttctaacgtaatgtggtacatcccggcaaaattaaaagaatggggcgtgaccccgccaaaaacatgggcagaatttttagcgacagcgcaaacattaaagcggaaaggccttgaggcaccattggcactcggtgagaattggacacagcaacatctctgggaaagcgtcgccctcgccacactgggtgccgatggttggaataatctctggagtggtaagctcaaattcacggatccaaaagcagtcgccgtatgggaaacattcggtaaggtattagatgcagcgaacaaggatgcagccgggctttcatggcaacaagcagtagaccgtgtagtacaggggaaagctgcattcaatatcatgggggactgggcagcaggttacatgagtacgaccttaaaactgaagccaggtaccgacttcgcatggacaccttctccgggcacttcagggatctttatgatgctgtctgatagtttcggcttgccaaagggggcgaagaatcgtcaaaatgctattaactggttgaaactcgtcgggtcaaaagaggggcaggacaccttcaacccgctcaaaggttccatcgctgctcgtctcgattctgatcctgccaaatataatgcatacggccaaagtgcaatgaaggactggaagtcaaatcggatcgtaggctccctcgtccacggcgcagtcgcgccagaatccttcatgtcgcagtttgggacggtaatggagattttcttgcaatcccgtaacccgcaggcagccgctaatgccgcacaagctatcgccaatcaggtcggtttaggtcgtgggggttcacatcatcatcatcatcattaatgaaagggcgatatccagcacactggcggccgttactagtggatccggctgctaacaaagcccgaaaggaagctgagttggctgctgccaccgctgagcaataactagcataaccccttggggcctctaaacgggtcttgaggggttttttgctgaaaggaggaactatatccggagcgactcccacggcacgttggcaagctcg

SEQ ID NO: 71 - DNA, 1577 bp, Artificial Sequence
  Exemplary tsGBP2_C64 expression sequence, optimized using OrfOpt
cggtcacgcttgggactgccataggctggcccggtgatgccggccacgatgcgtccggcgtagaggatcgagatctcgatcccgcgaaattaatacgactcactatagggagaccacaacggtttccctctagaaataattttgtttaactttaagaaggagatataccatgaaattagaaattttttcttggtgggcaggtgatgaaggcccagctctcgaagccttgatccggttgtataaacagaaatacccaggtgtagaggtcattaatgctaccgtcaccgggggtgccggtgtcaacgccaaagccgtccttaaaacgcgtatgctcggcggggacccaccagataccttttgcgtacatgcagggcaggagctgatcggcacatgggtcgtcgccgaccgtatggaagatcttacctcattgtttcggcaggagggctggcttcaagcgttcccaaaaggtttaatcgatctcctcagttacaaaggtggcatttggtcagtcccagtcaacatccaccgttctaacgtaatgtggtacatcccggcaaaattaaaagaatggggcgtgaccccgccaaaaacatgggcagaatttttagcgacagcgcaaacattaaagcggaaaggccttgaggcaccattggcactcggtgagaattggacacagcaacatctctgggaaagcgtcgccctcgccacactgggtgccgatggttggaataatctctggagtggtaagctcaaattcacggatccaaaagcagtcgccgtatgggaaacattcggtaaggtattagatgcagcgaacaaggatgcagccgggctttcatggcaacaagcagtagaccgtgtagtacaggggaaagctgcattcaatatcatgggggactgggcagcaggttacatgagtacgaccttaaaactgaagccaggtaccgacttcgcatggacaccttctccgggcacttcagggatctttatgatgctgtctgatagtttcggcttgccaaagggggcgaagaatcgtcaaaatgctattaactggttgaaactcgtcgggtcaaaagaggggcaggacaccttcaacccgctcaaaggttccatcgctgctcgtctcgattctgatcctgccaaatataatgcatacggccaaagtgcaatgaaggactggaagtcaaatcggatcgtaggctccctcgtccacggcgcagtcgcgccagaatccttcatgtcgcagtttgggacggtaatggagattttcttgcaatcccgtaacccgcaggcagccgctaatgccgcacaagctatcgccaatcaggtcggtttaggtcgtgggggttcacatcatcatcatcatcattaatgaaagggcgatatccagcacactggcggccgttactagtggatccggctgctaacaaagcccgaaaggaagctgagttggctgctgccaccgctgagcaataactagcataaccccttggggcctctaaacgggtcttgaggggttttttgctgaaaggaggaactatatccggagcgactcccacggcacgttggcaagctcg

SEQ ID NO: 72 - DNA, 1577 bp, Artificial Sequence
  Exemplary tsGBP2_C66 expression sequence, optimized using OrfOpt
cggtcacgcttgggactgccataggctggcccggtgatgccggccacgatgcgtccggcgtagaggatcgagatctcgatcccgcgaaattaatacgactcactatagggagaccacaacggtttccctctagaaataattttgtttaactttaagaaggagatataccatgaaattagaaattttttcttggtgggcaggtgatgaaggcccagctctcgaagccttgatccggttgtataaacagaaatacccaggtgtagaggtcattaatgctaccgtcaccgggggtgccggtgtcaacgccaaagccgtccttaaaacgcgtatgctcggcggggacccaccagatacctttcaagtatgcgcagggcaggagctgatcggcacatgggtcgtcgccgaccgtatggaagatcttacctcattgtttcggcaggagggctggcttcaagcgttcccaaaaggtttaatcgatctcctcagttacaaaggtggcatttggtcagtcccagtcaacatccaccgttctaacgtaatgtggtacatcccggcaaaattaaaagaatggggcgtgaccccgccaaaaacatgggcagaatttttagcgacagcgcaaacattaaagcggaaaggccttgaggcaccattggcactcggtgagaattggacacagcaacatctctgggaaagcgtcgccctcgccacactgggtgccgatggttggaataatctctggagtggtaagctcaaattcacggatccaaaagcagtcgccgtatgggaaacattcggtaaggtattagatgcagcgaacaaggatgcagccgggctttcatggcaacaagcagtagaccgtgtagtacaggggaaagctgcattcaatatcatgggggactgggcagcaggttacatgagtacgaccttaaaactgaagccaggtaccgacttcgcatggacaccttctccgggcacttcagggatctttatgatgctgtctgatagtttcggcttgccaaagggggcgaagaatcgtcaaaatgctattaactggttgaaactcgtcgggtcaaaagaggggcaggacaccttcaacccgctcaaaggttccatcgctgctcgtctcgattctgatcctgccaaatataatgcatacggccaaagtgcaatgaaggactggaagtcaaatcggatcgtaggctccctcgtccacggcgcagtcgcgccagaatccttcatgtcgcagtttgggacggtaatggagattttcttgcaatcccgtaacccgcaggcagccgctaatgccgcacaagctatcgccaatcaggtcggtttaggtcgtgggggttcacatcatcatcatcatcattaatgaaagggcgatatccagcacactggcggccgttactagtggatccggctgctaacaaagcccgaaaggaagctgagttggctgctgccaccgctgagcaataactagcataaccccttggggcctctaaacgggtcttgaggggttttttgctgaaaggaggaactatatccggagcgactcccacggcacgttggcaagctcg

SEQ ID NO: 73 - DNA, 1577 bp, Artificial Sequence
  Exemplary tsGBP2_C119 expression sequence, optimized using OrfOpt
cggtcacgcttgggactgccataggctggcccggtgatgccggccacgatgcgtccggcgtagaggatcgagatctcgatcccgcgaaattaatacgactcactatagggagaccacaacggtttccctctagaaataattttgtttaactttaagaaggagatataccatgaaattagaaattttttcttggtgggcaggtgatgaaggcccagctctcgaagccttgatccggttgtataaacagaaatacccaggtgtagaggtcattaatgctaccgtcaccgggggtgccggtgtcaacgccaaagccgtccttaaaacgcgtatgctcggcggggacccaccagatacctttcaagtacatgcagggcaggagctgatcggcacatgggtcgtcgccgaccgtatggaagatcttacctcattgtttcggcaggagggctggcttcaagcgttcccaaaaggtttaatcgatctcctcagttacaaaggtggcatttggtcagtcccagtcaacatctgccgttctaacgtaatgtggtacatcccggcaaaattaaaagaatggggcgtgaccccgccaaaaacatgggcagaatttttagcgacagcgcaaacattaaagcggaaaggccttgaggcaccattggcactcggtgagaattggacacagcaacatctctgggaaagcgtcgccctcgccacactgggtgccgatggttggaataatctctggagtggtaagctcaaattcacggatccaaaagcagtcgccgtatgggaaacattcggtaaggtattagatgcagcgaacaaggatgcagccgggctttcatggcaacaagcagtagaccgtgtagtacaggggaaagctgcattcaatatcatgggggactgggcagcaggttacatgagtacgaccttaaaactgaagccaggtaccgacttcgcatggacaccttctccgggcacttcagggatctttatgatgctgtctgatagtttcggcttgccaaagggggcgaagaatcgtcaaaatgctattaactggttgaaactcgtcgggtcaaaagaggggcaggacaccttcaacccgctcaaaggttccatcgctgctcgtctcgattctgatcctgccaaatataatgcatacggccaaagtgcaatgaaggactggaagtcaaatcggatcgtaggctccctcgtccacggcgcagtcgcgccagaatccttcatgtcgcagtttgggacggtaatggagattttcttgcaatcccgtaacccgcaggcagccgctaatgccgcacaagctatcgccaatcaggtcggtttaggtcgtgggggttcacatcatcatcatcatcattaatgaaagggcgatatccagcacactggcggccgttactagtggatccggctgctaacaaagcccgaaaggaagctgagttggctgctgccaccgctgagcaataactagcataaccccttggggcctctaaacgggtcttgaggggttttttgctgaaaggaggaactatatccggagcgactcccacggcacgttggcaagctcg

SEQ ID NO: 74 - DNA, 1577 bp, Artificial Sequence
  Exemplary tsGBP2_C167 expression sequence, optimized using OrfOpt
cggtcacgcttgggactgccataggctggcccggtgatgccggccacgatgcgtccggcgtagaggatcgagatctcgatcccgcgaaattaatacgactcactatagggagaccacaacggtttccctctagaaataattttgtttaactttaagaaggagatataccatgaaattagaaattttttcttggtgggcaggtgatgaaggcccagctctcgaagccttgatccggttgtataaacagaaatacccaggtgtagaggtcattaatgctaccgtcaccgggggtgccggtgtcaacgccaaagccgtccttaaaacgcgtatgctcggcggggacccaccagatacctttcaagtacatgcagggcaggagctgatcggcacatgggtcgtcgccgaccgtatggaagatcttacctcattgtttcggcaggagggctggcttcaagcgttcccaaaaggtttaatcgatctcctcagttacaaaggtggcatttggtcagtcccagtcaacatccaccgttctaacgtaatgtggtacatcccggcaaaattaaaagaatggggcgtgaccccgccaaaaacatgggcagaatttttagcgacagcgcaaacattaaagcggaaaggccttgaggcaccattggcactcggtgagaattgcacacagcaacatctctgggaaagcgtcgccctcgccacactgggtgccgatggttggaataatctctggagtggtaagctcaaattcacggatccaaaagcagtcgccgtatgggaaacattcggtaaggtattagatgcagcgaacaaggatgcagccgggctttcatggcaacaagcagtagaccgtgtagtacaggggaaagctgcattcaatatcatgggggactgggcagcaggttacatgagtacgaccttaaaactgaagccaggtaccgacttcgcatggacaccttctccgggcacttcagggatctttatgatgctgtctgatagtttcggcttgccaaagggggcgaagaatcgtcaaaatgctattaactggttgaaactcgtcgggtcaaaagaggggcaggacaccttcaacccgctcaaaggttccatcgctgctcgtctcgattctgatcctgccaaatataatgcatacggccaaagtgcaatgaaggactggaagtcaaatcggatcgtaggctccctcgtccacggcgcagtcgcgccagaatccttcatgtcgcagtttgggacggtaatggagattttcttgcaatcccgtaacccgcaggcagccgctaatgccgcacaagctatcgccaatcaggtcggtttaggtcgtgggggttcacatcatcatcatcatcattaatgaaagggcgatatccagcacactggcggccgttactagtggatccggctgctaacaaagcccgaaaggaagctgagttggctgctgccaccgctgagcaataactagcataaccccttggggcctctaaacgggtcttgaggggttttttgctgaaaggaggaactatatccggagcgactcccacggcacgttggcaagctcg

SEQ ID NO: 75 - DNA, 1577 bp, Artificial Sequence
  Exemplary tsGBP2_C223 expression sequence, optimized using OrfOpt
cggtcacgcttgggactgccataggctggcccggtgatgccggccacgatgcgtccggcgtagaggatcgagatctcgatcccgcgaaattaatacgactcactatagggagaccacaacggtttccctctagaaataattttgtttaactttaagaaggagatataccatgaaattagaaattttttcttggtgggcaggtgatgaaggcccagctctcgaagccttgatccggttgtataaacagaaatacccaggtgtagaggtcattaatgctaccgtcaccgggggtgccggtgtcaacgccaaagccgtccttaaaacgcgtatgctcggcggggacccaccagatacctttcaagtacatgcagggcaggagctgatcggcacatgggtcgtcgccgaccgtatggaagatcttacctcattgtttcggcaggagggctggcttcaagcgttcccaaaaggtttaatcgatctcctcagttacaaaggtggcatttggtcagtcccagtcaacatccaccgttctaacgtaatgtggtacatcccggcaaaattaaaagaatggggcgtgaccccgccaaaaacatgggcagaatttttagcgacagcgcaaacattaaagcggaaaggccttgaggcaccattggcactcggtgagaattggacacagcaacatctctgggaaagcgtcgccctcgccacactgggtgccgatggttggaataatctctggagtggtaagctcaaattcacggatccaaaagcagtcgccgtatgggaaacattcggtaaggtattagatgcagcgaacaaggatgcagccgggctttgctggcaacaagcagtagaccgtgtagtacaggggaaagctgcattcaatatcatgggggactgggcagcaggttacatgagtacgaccttaaaactgaagccaggtaccgacttcgcatggacaccttctccgggcacttcagggatctttatgatgctgtctgatagtttcggcttgccaaagggggcgaagaatcgtcaaaatgctattaactggttgaaactcgtcgggtcaaaagaggggcaggacaccttcaacccgctcaaaggttccatcgctgctcgtctcgattctgatcctgccaaatataatgcatacggccaaagtgcaatgaaggactggaagtcaaatcggatcgtaggctccctcgtccacggcgcagtcgcgccagaatccttcatgtcgcagtttgggacggtaatggagattttcttgcaatcccgtaacccgcaggcagccgctaatgccgcacaagctatcgccaatcaggtcggtttaggtcgtgggggttcacatcatcatcatcatcattaatgaaagggcgatatccagcacactggcggccgttactagtggatccggctgctaacaaagcccgaaaggaagctgagttggctgctgccaccgctgagcaataactagcataaccccttggggcctctaaacgggtcttgaggggttttttgctgaaaggaggaactatatccggagcgactcccacggcacgttggcaagctcg

SEQ ID NO: 76 - DNA, 1577 bp, Artificial Sequence
  Exemplary tsGBP2_C224 expression sequence, optimized using OrfOpt
cggtcacgcttgggactgccataggctggcccggtgatgccggccacgatgcgtccggcgtagaggatcgagatctcgatcccgcgaaattaatacgactcactatagggagaccacaacggtttccctctagaaataattttgtttaactttaagaaggagatataccatgaaattagaaattttttcttggtgggcaggtgatgaaggcccagctctcgaagccttgatccggttgtataaacagaaatacccaggtgtagaggtcattaatgctaccgtcaccgggggtgccggtgtcaacgccaaagccgtccttaaaacgcgtatgctcggcggggacccaccagatacctttcaagtacatgcagggcaggagctgatcggcacatgggtcgtcgccgaccgtatggaagatcttacctcattgtttcggcaggagggctggcttcaagcgttcccaaaaggtttaatcgatctcctcagttacaaaggtggcatttggtcagtcccagtcaacatccaccgttctaacgtaatgtggtacatcccggcaaaattaaaagaatggggcgtgaccccgccaaaaacatgggcagaatttttagcgacagcgcaaacattaaagcggaaaggccttgaggcaccattggcactcggtgagaattggacacagcaacatctctgggaaagcgtcgccctcgccacactgggtgccgatggttggaataatctctggagtggtaagctcaaattcacggatccaaaagcagtcgccgtatgggaaacattcggtaaggtattagatgcagcgaacaaggatgcagccgggctttcatgccaacaagcagtagaccgtgtagtacaggggaaagctgcattcaatatcatgggggactgggcagcaggttacatgagtacgaccttaaaactgaagccaggtaccgacttcgcatggacaccttctccgggcacttcagggatctttatgatgctgtctgatagtttcggcttgccaaagggggcgaagaatcgtcaaaatgctattaactggttgaaactcgtcgggtcaaaagaggggcaggacaccttcaacccgctcaaaggttccatcgctgctcgtctcgattctgatcctgccaaatataatgcatacggccaaagtgcaatgaaggactggaagtcaaatcggatcgtaggctccctcgtccacggcgcagtcgcgccagaatccttcatgtcgcagtttgggacggtaatggagattttcttgcaatcccgtaacccgcaggcagccgctaatgccgcacaagctatcgccaatcaggtcggtttaggtcgtgggggttcacatcatcatcatcatcattaatgaaagggcgatatccagcacactggcggccgttactagtggatccggctgctaacaaagcccgaaaggaagctgagttggctgctgccaccgctgagcaataactagcataaccccttggggcctctaaacgggtcttgaggggttttttgctgaaaggaggaactatatccggagcgactcccacggcacgttggcaagctcg

SEQ ID NO: 77 - DNA, 1577 bp, Artificial Sequence
  Exemplary tsGBP2_C225 expression sequence, optimized using OrfOpt
cggtcacgcttgggactgccataggctggcccggtgatgccggccacgatgcgtccggcgtagaggatcgagatctcgatcccgcgaaattaatacgactcactatagggagaccacaacggtttccctctagaaataattttgtttaactttaagaaggagatataccatgaaattagaaattttttcttggtgggcaggtgatgaaggcccagctctcgaagccttgatccggttgtataaacagaaatacccaggtgtagaggtcattaatgctaccgtcaccgggggtgccggtgtcaacgccaaagccgtccttaaaacgcgtatgctcggcggggacccaccagatacctttcaagtacatgcagggcaggagctgatcggcacatgggtcgtcgccgaccgtatggaagatcttacctcattgtttcggcaggagggctggcttcaagcgttcccaaaaggtttaatcgatctcctcagttacaaaggtggcatttggtcagtcccagtcaacatccaccgttctaacgtaatgtggtacatcccggcaaaattaaaagaatggggcgtgaccccgccaaaaacatgggcagaatttttagcgacagcgcaaacattaaagcggaaaggccttgaggcaccattggcactcggtgagaattggacacagcaacatctctgggaaagcgtcgccctcgccacactgggtgccgatggttggaataatctctggagtggtaagctcaaattcacggatccaaaagcagtcgccgtatgggaaacattcggtaaggtattagatgcagcgaacaaggatgcagccgggctttcatggtgccaagcagtagaccgtgtagtacaggggaaagctgcattcaatatcatgggggactgggcagcaggttacatgagtacgaccttaaaactgaagccaggtaccgacttcgcatggacaccttctccgggcacttcagggatctttatgatgctgtctgatagtttcggcttgccaaagggggcgaagaatcgtcaaaatgctattaactggttgaaactcgtcgggtcaaaagaggggcaggacaccttcaacccgctcaaaggttccatcgctgctcgtctcgattctgatcctgccaaatataatgcatacggccaaagtgcaatgaaggactggaagtcaaatcggatcgtaggctccctcgtccacggcgcagtcgcgccagaatccttcatgtcgcagtttgggacggtaatggagattttcttgcaatcccgtaacccgcaggcagccgctaatgccgcacaagctatcgccaatcaggtcggtttaggtcgtgggggttcacatcatcatcatcatcattaatgaaagggcgatatccagcacactggcggccgttactagtggatccggctgctaacaaagcccgaaaggaagctgagttggctgctgccaccgctgagcaataactagcataaccccttggggcctctaaacgggtcttgaggggttttttgctgaaaggaggaactatatccggagcgactcccacggcacgttggcaagctcg

SEQ ID NO: 78 - DNA, 1577 bp, Artificial Sequence
  Exemplary tsGBP2_C244 expression sequence, optimized using OrfOpt
cggtcacgcttgggactgccataggctggcccggtgatgccggccacgatgcgtccggcgtagaggatcgagatctcgatcccgcgaaattaatacgactcactatagggagaccacaacggtttccctctagaaataattttgtttaactttaagaaggagatataccatgaaattagaaattttttcttggtgggcaggtgatgaaggcccagctctcgaagccttgatccggttgtataaacagaaatacccaggtgtagaggtcattaatgctaccgtcaccgggggtgccggtgtcaacgccaaagccgtccttaaaacgcgtatgctcggcggggacccaccagatacctttcaagtacatgcagggcaggagctgatcggcacatgggtcgtcgccgaccgtatggaagatcttacctcattgtttcggcaggagggctggcttcaagcgttcccaaaaggtttaatcgatctcctcagttacaaaggtggcatttggtcagtcccagtcaacatccaccgttctaacgtaatgtggtacatcccggcaaaattaaaagaatggggcgtgaccccgccaaaaacatgggcagaatttttagcgacagcgcaaacattaaagcggaaaggccttgaggcaccattggcactcggtgagaattggacacagcaacatctctgggaaagcgtcgccctcgccacactgggtgccgatggttggaataatctctggagtggtaagctcaaattcacggatccaaaagcagtcgccgtatgggaaacattcggtaaggtattagatgcagcgaacaaggatgcagccgggctttcatggcaacaagcagtagaccgtgtagtacaggggaaagctgcattcaatatcatgggggactgcgcagcaggttacatgagtacgaccttaaaactgaagccaggtaccgacttcgcatggacaccttctccgggcacttcagggatctttatgatgctgtctgatagtttcggcttgccaaagggggcgaagaatcgtcaaaatgctattaactggttgaaactcgtcgggtcaaaagaggggcaggacaccttcaacccgctcaaaggttccatcgctgctcgtctcgattctgatcctgccaaatataatgcatacggccaaagtgcaatgaaggactggaagtcaaatcggatcgtaggctccctcgtccacggcgcagtcgcgccagaatccttcatgtcgcagtttgggacggtaatggagattttcttgcaatcccgtaacccgcaggcagccgctaatgccgcacaagctatcgccaatcaggtcggtttaggtcgtgggggttcacatcatcatcatcatcattaatgaaagggcgatatccagcacactggcggccgttactagtggatccggctgctaacaaagcccgaaaggaagctgagttggctgctgccaccgctgagcaataactagcataaccccttggggcctctaaacgggtcttgaggggttttttgctgaaaggaggaactatatccggagcgactcccacggcacgttggcaagctcg

SEQ ID NO: 79 - DNA, 1577 bp, Artificial Sequence
  Exemplary tsGBP2_C277 expression sequence, optimized using OrfOpt
cggtcacgcttgggactgccataggctggcccggtgatgccggccacgatgcgtccggcgtagaggatcgagatctcgatcccgcgaaattaatacgactcactatagggagaccacaacggtttccctctagaaataattttgtttaactttaagaaggagatataccatgaaattagaaattttttcttggtgggcaggtgatgaaggcccagctctcgaagccttgatccggttgtataaacagaaatacccaggtgtagaggtcattaatgctaccgtcaccgggggtgccggtgtcaacgccaaagccgtccttaaaacgcgtatgctcggcggggacccaccagatacctttcaagtacatgcagggcaggagctgatcggcacatgggtcgtcgccgaccgtatggaagatcttacctcattgtttcggcaggagggctggcttcaagcgttcccaaaaggtttaatcgatctcctcagttacaaaggtggcatttggtcagtcccagtcaacatccaccgttctaacgtaatgtggtacatcccggcaaaattaaaagaatggggcgtgaccccgccaaaaacatgggcagaatttttagcgacagcgcaaacattaaagcggaaaggccttgaggcaccattggcactcggtgagaattggacacagcaacatctctgggaaagcgtcgccctcgccacactgggtgccgatggttggaataatctctggagtggtaagctcaaattcacggatccaaaagcagtcgccgtatgggaaacattcggtaaggtattagatgcagcgaacaaggatgcagccgggctttcatggcaacaagcagtagaccgtgtagtacaggggaaagctgcattcaatatcatgggggactgggcagcaggttacatgagtacgaccttaaaactgaagccaggtaccgacttcgcatggacaccttctccgggcacttcagggatctttatgatgctgtgcgatagtttcggcttgccaaagggggcgaagaatcgtcaaaatgctattaactggttgaaactcgtcgggtcaaaagaggggcaggacaccttcaacccgctcaaaggttccatcgctgctcgtctcgattctgatcctgccaaatataatgcatacggccaaagtgcaatgaaggactggaagtcaaatcggatcgtaggctccctcgtccacggcgcagtcgcgccagaatccttcatgtcgcagtttgggacggtaatggagattttcttgcaatcccgtaacccgcaggcagccgctaatgccgcacaagctatcgccaatcaggtcggtttaggtcgtgggggttcacatcatcatcatcatcattaatgaaagggcgatatccagcacactggcggccgttactagtggatccggctgctaacaaagcccgaaaggaagctgagttggctgctgccaccgctgagcaataactagcataaccccttggggcctctaaacgggtcttgaggggttttttgctgaaaggaggaactatatccggagcgactcccacggcacgttggcaagctcg

SEQ ID NO: 80 - DNA, 1577 bp, Artificial Sequence
  Exemplary tsGBP2_C278 expression sequence, optimized using OrfOpt
cggtcacgcttgggactgccataggctggcccggtgatgccggccacgatgcgtccggcgtagaggatcgagatctcgatcccgcgaaattaatacgactcactatagggagaccacaacggtttccctctagaaataattttgtttaactttaagaaggagatataccatgaaattagaaattttttcttggtgggcaggtgatgaaggcccagctctcgaagccttgatccggttgtataaacagaaatacccaggtgtagaggtcattaatgctaccgtcaccgggggtgccggtgtcaacgccaaagccgtccttaaaacgcgtatgctcggcggggacccaccagatacctttcaagtacatgcagggcaggagctgatcggcacatgggtcgtcgccgaccgtatggaagatcttacctcattgtttcggcaggagggctggcttcaagcgttcccaaaaggtttaatcgatctcctcagttacaaaggtggcatttggtcagtcccagtcaacatccaccgttctaacgtaatgtggtacatcccggcaaaattaaaagaatggggcgtgaccccgccaaaaacatgggcagaatttttagcgacagcgcaaacattaaagcggaaaggccttgaggcaccattggcactcggtgagaattggacacagcaacatctctgggaaagcgtcgccctcgccacactgggtgccgatggttggaataatctctggagtggtaagctcaaattcacggatccaaaagcagtcgccgtatgggaaacattcggtaaggtattagatgcagcgaacaaggatgcagccgggctttcatggcaacaagcagtagaccgtgtagtacaggggaaagctgcattcaatatcatgggggactgggcagcaggttacatgagtacgaccttaaaactgaagccaggtaccgacttcgcatggacaccttctccgggcacttcagggatctttatgatgctgtcttgcagtttcggcttgccaaagggggcgaagaatcgtcaaaatgctattaactggttgaaactcgtcgggtcaaaagaggggcaggacaccttcaacccgctcaaaggttccatcgctgctcgtctcgattctgatcctgccaaatataatgcatacggccaaagtgcaatgaaggactggaagtcaaatcggatcgtaggctccctcgtccacggcgcagtcgcgccagaatccttcatgtcgcagtttgggacggtaatggagattttcttgcaatcccgtaacccgcaggcagccgctaatgccgcacaagctatcgccaatcaggtcggtttaggtcgtgggggttcacatcatcatcatcatcattaatgaaagggcgatatccagcacactggcggccgttactagtggatccggctgctaacaaagcccgaaaggaagctgagttggctgctgccaccgctgagcaataactagcataaccccttggggcctctaaacgggtcttgaggggttttttgctgaaaggaggaactatatccggagcgactcccacggcacgttggcaagctcg

SEQ ID NO: 81 - DNA, 1577 bp, Artificial Sequence
  Exemplary tsGBP2_C312 expression sequence, optimized using OrfOpt
cggtcacgcttgggactgccataggctggcccggtgatgccggccacgatgcgtccggcgtagaggatcgagatctcgatcccgcgaaattaatacgactcactatagggagaccacaacggtttccctctagaaataattttgtttaactttaagaaggagatataccatgaaattagaaattttttcttggtgggcaggtgatgaaggcccagctctcgaagccttgatccggttgtataaacagaaatacccaggtgtagaggtcattaatgctaccgtcaccgggggtgccggtgtcaacgccaaagccgtccttaaaacgcgtatgctcggcggggacccaccagatacctttcaagtacatgcagggcaggagctgatcggcacatgggtcgtcgccgaccgtatggaagatcttacctcattgtttcggcaggagggctggcttcaagcgttcccaaaaggtttaatcgatctcctcagttacaaaggtggcatttggtcagtcccagtcaacatccaccgttctaacgtaatgtggtacatcccggcaaaattaaaagaatggggcgtgaccccgccaaaaacatgggcagaatttttagcgacagcgcaaacattaaagcggaaaggccttgaggcaccattggcactcggtgagaattggacacagcaacatctctgggaaagcgtcgccctcgccacactgggtgccgatggttggaataatctctggagtggtaagctcaaattcacggatccaaaagcagtcgccgtatgggaaacattcggtaaggtattagatgcagcgaacaaggatgcagccgggctttcatggcaacaagcagtagaccgtgtagtacaggggaaagctgcattcaatatcatgggggactgggcagcaggttacatgagtacgaccttaaaactgaagccaggtaccgacttcgcatggacaccttctccgggcacttcagggatctttatgatgctgtctgatagtttcggcttgccaaagggggcgaagaatcgtcaaaatgctattaactggttgaaactcgtcgggtcaaaagaggggcaggacaccttcaacccgctctgcggttccatcgctgctcgtctcgattctgatcctgccaaatataatgcatacggccaaagtgcaatgaaggactggaagtcaaatcggatcgtaggctccctcgtccacggcgcagtcgcgccagaatccttcatgtcgcagtttgggacggtaatggagattttcttgcaatcccgtaacccgcaggcagccgctaatgccgcacaagctatcgccaatcaggtcggtttaggtcgtgggggttcacatcatcatcatcatcattaatgaaagggcgatatccagcacactggcggccgttactagtggatccggctgctaacaaagcccgaaaggaagctgagttggctgctgccaccgctgagcaataactagcataaccccttggggcctctaaacgggtcttgaggggttttttgctgaaaggaggaactatatccggagcgactcccacggcacgttggcaagctcg

SEQ ID NO: 82 - DNA, 1577 bp, Artificial Sequence
  Exemplary tsGBP2_C337 expression sequence, optimized using OrfOpt
cggtcacgcttgggactgccataggctggcccggtgatgccggccacgatgcgtccggcgtagaggatcgagatctcgatcccgcgaaattaatacgactcactatagggagaccacaacggtttccctctagaaataattttgtttaactttaagaaggagatataccatgaaattagaaattttttcttggtgggcaggtgatgaaggcccagctctcgaagccttgatccggttgtataaacagaaatacccaggtgtagaggtcattaatgctaccgtcaccgggggtgccggtgtcaacgccaaagccgtccttaaaacgcgtatgctcggcggggacccaccagatacctttcaagtacatgcagggcaggagctgatcggcacatgggtcgtcgccgaccgtatggaagatcttacctcattgtttcggcaggagggctggcttcaagcgttcccaaaaggtttaatcgatctcctcagttacaaaggtggcatttggtcagtcccagtcaacatccaccgttctaacgtaatgtggtacatcccggcaaaattaaaagaatggggcgtgaccccgccaaaaacatgggcagaatttttagcgacagcgcaaacattaaagcggaaaggccttgaggcaccattggcactcggtgagaattggacacagcaacatctctgggaaagcgtcgccctcgccacactgggtgccgatggttggaataatctctggagtggtaagctcaaattcacggatccaaaagcagtcgccgtatgggaaacattcggtaaggtattagatgcagcgaacaaggatgcagccgggctttcatggcaacaagcagtagaccgtgtagtacaggggaaagctgcattcaatatcatgggggactgggcagcaggttacatgagtacgaccttaaaactgaagccaggtaccgacttcgcatggacaccttctccgggcacttcagggatctttatgatgctgtctgatagtttcggcttgccaaagggggcgaagaatcgtcaaaatgctattaactggttgaaactcgtcgggtcaaaagaggggcaggacaccttcaacccgctcaaaggttccatcgctgctcgtctcgattctgatcctgccaaatataatgcatacggccaaagtgcaatgaaggactgcaagtcaaatcggatcgtaggctccctcgtccacggcgcagtcgcgccagaatccttcatgtcgcagtttgggacggtaatggagattttcttgcaatcccgtaacccgcaggcagccgctaatgccgcacaagctatcgccaatcaggtcggtttaggtcgtgggggttcacatcatcatcatcatcattaatgaaagggcgatatccagcacactggcggccgttactagtggatccggctgctaacaaagcccgaaaggaagctgagttggctgctgccaccgctgagcaataactagcataaccccttggggcctctaaacgggtcttgaggggttttttgctgaaaggaggaactatatccggagcgactcccacggcacgttggcaagctcg

SEQ ID NO: 83 - DNA, 1577 bp, Artificial Sequence
  Exemplary tsGBP2_C348 expression sequence, optimized using OrfOpt
cggtcacgcttgggactgccataggctggcccggtgatgccggccacgatgcgtccggcgtagaggatcgagatctcgatcccgcgaaattaatacgactcactatagggagaccacaacggtttccctctagaaataattttgtttaactttaagaaggagatataccatgaaattagaaattttttcttggtgggcaggtgatgaaggcccagctctcgaagccttgatccggttgtataaacagaaatacccaggtgtagaggtcattaatgctaccgtcaccgggggtgccggtgtcaacgccaaagccgtccttaaaacgcgtatgctcggcggggacccaccagatacctttcaagtacatgcagggcaggagctgatcggcacatgggtcgtcgccgaccgtatggaagatcttacctcattgtttcggcaggagggctggcttcaagcgttcccaaaaggtttaatcgatctcctcagttacaaaggtggcatttggtcagtcccagtcaacatccaccgttctaacgtaatgtggtacatcccggcaaaattaaaagaatggggcgtgaccccgccaaaaacatgggcagaatttttagcgacagcgcaaacattaaagcggaaaggccttgaggcaccattggcactcggtgagaattggacacagcaacatctctgggaaagcgtcgccctcgccacactgggtgccgatggttggaataatctctggagtggtaagctcaaattcacggatccaaaagcagtcgccgtatgggaaacattcggtaaggtattagatgcagcgaacaaggatgcagccgggctttcatggcaacaagcagtagaccgtgtagtacaggggaaagctgcattcaatatcatgggggactgggcagcaggttacatgagtacgaccttaaaactgaagccaggtaccgacttcgcatggacaccttctccgggcacttcagggatctttatgatgctgtctgatagtttcggcttgccaaagggggcgaagaatcgtcaaaatgctattaactggttgaaactcgtcgggtcaaaagaggggcaggacaccttcaacccgctcaaaggttccatcgctgctcgtctcgattctgatcctgccaaatataatgcatacggccaaagtgcaatgaaggactggaagtcaaatcggatcgtaggctccctcgtctgcggcgcagtcgcgccagaatccttcatgtcgcagtttgggacggtaatggagattttcttgcaatcccgtaacccgcaggcagccgctaatgccgcacaagctatcgccaatcaggtcggtttaggtcgtgggggttcacatcatcatcatcatcattaatgaaagggcgatatccagcacactggcggccgttactagtggatccggctgctaacaaagcccgaaaggaagctgagttggctgctgccaccgctgagcaataactagcataaccccttggggcctctaaacgggtcttgaggggttttttgctgaaaggaggaactatatccggagcgactcccacggcacgttggcaagctcg

SEQ ID NO: 84 - DNA, 1577 bp, Artificial Sequence
  Exemplary tsGBP2_C357 expression sequence, optimized using OrfOpt
cggtcacgcttgggactgccataggctggcccggtgatgccggccacgatgcgtccggcgtagaggatcgagatctcgatcccgcgaaattaatacgactcactatagggagaccacaacggtttccctctagaaataattttgtttaactttaagaaggagatataccatgaaattagaaattttttcttggtgggcaggtgatgaaggcccagctctcgaagccttgatccggttgtataaacagaaatacccaggtgtagaggtcattaatgctaccgtcaccgggggtgccggtgtcaacgccaaagccgtccttaaaacgcgtatgctcggcggggacccaccagatacctttcaagtacatgcagggcaggagctgatcggcacatgggtcgtcgccgaccgtatggaagatcttacctcattgtttcggcaggagggctggcttcaagcgttcccaaaaggtttaatcgatctcctcagttacaaaggtggcatttggtcagtcccagtcaacatccaccgttctaacgtaatgtggtacatcccggcaaaattaaaagaatggggcgtgaccccgccaaaaacatgggcagaatttttagcgacagcgcaaacattaaagcggaaaggccttgaggcaccattggcactcggtgagaattggacacagcaacatctctgggaaagcgtcgccctcgccacactgggtgccgatggttggaataatctctggagtggtaagctcaaattcacggatccaaaagcagtcgccgtatgggaaacattcggtaaggtattagatgcagcgaacaaggatgcagccgggctttcatggcaacaagcagtagaccgtgtagtacaggggaaagctgcattcaatatcatgggggactgggcagcaggttacatgagtacgaccttaaaactgaagccaggtaccgacttcgcatggacaccttctccgggcacttcagggatctttatgatgctgtctgatagtttcggcttgccaaagggggcgaagaatcgtcaaaatgctattaactggttgaaactcgtcgggtcaaaagaggggcaggacaccttcaacccgctcaaaggttccatcgctgctcgtctcgattctgatcctgccaaatataatgcatacggccaaagtgcaatgaaggactggaagtcaaatcggatcgtaggctccctcgtccacggcgcagtcgcgccagaatccttctgctcgcagtttgggacggtaatggagattttcttgcaatcccgtaacccgcaggcagccgctaatgccgcacaagctatcgccaatcaggtcggtttaggtcgtgggggttcacatcatcatcatcatcattaatgaaagggcgatatccagcacactggcggccgttactagtggatccggctgctaacaaagcccgaaaggaagctgagttggctgctgccaccgctgagcaataactagcataaccccttggggcctctaaacgggtcttgaggggttttttgctgaaaggaggaactatatccggagcgactcccacggcacgttggcaagctcg

SEQ ID NO: 85 - DNA, 1577 bp, Artificial Sequence
  Exemplary tsGBP2.13C.W8F expression sequence, optimized using OrfOpt
cggtcacgcttgggactgccataggctggcccggtgatgccggccacgatgcgtccggcgtagaggatcgagatctcgatcccgcgaaattaatacgactcactatagggagaccacaacggtttccctctagaaataattttgtttaactttaagaaggagatataccatgaaattagaaattttttctttttgggcaggtgattgtggcccagctctcgaagccttgatccggttgtataaacagaaatacccaggtgtagaggtcattaatgctaccgtcaccgggggtgccggtgtcaacgccaaagccgtccttaaaacgcgtatgctcggcggggacccaccagatacctttcaagtacatgcagggcaggagctgatcggcacatgggtcgtcgccgaccgtatggaagatcttacctcattgtttcggcaggagggctggcttcaagcgttcccaaaaggtttaatcgatctcctcagttacaaaggtggcatttggtcagtcccagtcaacatccaccgttctaacgtaatgtggtacatcccggcaaaattaaaagaatggggcgtgaccccgccaaaaacatgggcagaatttttagcgacagcgcaaacattaaagcggaaaggccttgaggcaccattggcactcggtgagaattggacacagcaacatctctgggaaagcgtcgccctcgccacactgggtgccgatggttggaataatctctggagtggtaagctcaaattcacggatccaaaagcagtcgccgtatgggaaacattcggtaaggtattagatgcagcgaacaaggatgcagccgggctttcatggcaacaagcagtagaccgtgtagtacaggggaaagctgcattcaatatcatgggggactgggcagcaggttacatgagtacgaccttaaaactgaagccaggtaccgacttcgcatggacaccttctccgggcacttcagggatctttatgatgctgtctgatagtttcggcttgccaaagggggcgaagaatcgtcaaaatgctattaactggttgaaactcgtcgggtcaaaagaggggcaggacaccttcaacccgctcaaaggttccatcgctgctcgtctcgattctgatcctgccaaatataatgcatacggccaaagtgcaatgaaggactggaagtcaaatcggatcgtaggctccctcgtccacggcgcagtcgcgccagaatccttcatgtcgcagtttgggacggtaatggagattttcttgcaatcccgtaacccgcaggcagccgctaatgccgcacaagctatcgccaatcaggtcggtttaggtcgtgggggttcacatcatcatcatcatcattaatgaaagggcgatatccagcacactggcggccgttactagtggatccggctgctaacaaagcccgaaaggaagctgagttggctgctgccaccgctgagcaataactagcataaccccttggggcctctaaacgggtcttgaggggttttttgctgaaaggaggaactatatccggagcgactcccacggcacgttggcaagctcg

SEQ ID NO: 86 - DNA, 1577 bp, Artificial Sequence
  Exemplary tsGBP2.13C.W8M expression sequence, optimized using OrfOpt
cggtcacgcttgggactgccataggctggcccggtgatgccggccacgatgcgtccggcgtagaggatcgagatctcgatcccgcgaaattaatacgactcactatagggagaccacaacggtttccctctagaaataattttgtttaactttaagaaggagatataccatgaaattagaaattttttctatgtgggcaggtgattgtggcccagctctcgaagccttgatccggttgtataaacagaaatacccaggtgtagaggtcattaatgctaccgtcaccgggggtgccggtgtcaacgccaaagccgtccttaaaacgcgtatgctcggcggggacccaccagatacctttcaagtacatgcagggcaggagctgatcggcacatgggtcgtcgccgaccgtatggaagatcttacctcattgtttcggcaggagggctggcttcaagcgttcccaaaaggtttaatcgatctcctcagttacaaaggtggcatttggtcagtcccagtcaacatccaccgttctaacgtaatgtggtacatcccggcaaaattaaaagaatggggcgtgaccccgccaaaaacatgggcagaatttttagcgacagcgcaaacattaaagcggaaaggccttgaggcaccattggcactcggtgagaattggacacagcaacatctctgggaaagcgtcgccctcgccacactgggtgccgatggttggaataatctctggagtggtaagctcaaattcacggatccaaaagcagtcgccgtatgggaaacattcggtaaggtattagatgcagcgaacaaggatgcagccgggctttcatggcaacaagcagtagaccgtgtagtacaggggaaagctgcattcaatatcatgggggactgggcagcaggttacatgagtacgaccttaaaactgaagccaggtaccgacttcgcatggacaccttctccgggcacttcagggatctttatgatgctgtctgatagtttcggcttgccaaagggggcgaagaatcgtcaaaatgctattaactggttgaaactcgtcgggtcaaaagaggggcaggacaccttcaacccgctcaaaggttccatcgctgctcgtctcgattctgatcctgccaaatataatgcatacggccaaagtgcaatgaaggactggaagtcaaatcggatcgtaggctccctcgtccacggcgcagtcgcgccagaatccttcatgtcgcagtttgggacggtaatggagattttcttgcaatcccgtaacccgcaggcagccgctaatgccgcacaagctatcgccaatcaggtcggtttaggtcgtgggggttcacatcatcatcatcatcattaatgaaagggcgatatccagcacactggcggccgttactagtggatccggctgctaacaaagcccgaaaggaagctgagttggctgctgccaccgctgagcaataactagcataaccccttggggcctctaaacgggtcttgaggggttttttgctgaaaggaggaactatatccggagcgactcccacggcacgttggcaagctcg

SEQ ID NO: 87 - DNA, 1577 bp, Artificial Sequence
  Exemplary tsGBP2.13C.W8Y expression sequence, optimized using OrfOpt
cggtcacgcttgggactgccataggctggcccggtgatgccggccacgatgcgtccggcgtagaggatcgagatctcgatcccgcgaaattaatacgactcactatagggagaccacaacggtttccctctagaaataattttgtttaactttaagaaggagatataccatgaaattagaaattttttcttattgggcaggtgattgtggcccagctctcgaagccttgatccggttgtataaacagaaatacccaggtgtagaggtcattaatgctaccgtcaccgggggtgccggtgtcaacgccaaagccgtccttaaaacgcgtatgctcggcggggacccaccagatacctttcaagtacatgcagggcaggagctgatcggcacatgggtcgtcgccgaccgtatggaagatcttacctcattgtttcggcaggagggctggcttcaagcgttcccaaaaggtttaatcgatctcctcagttacaaaggtggcatttggtcagtcccagtcaacatccaccgttctaacgtaatgtggtacatcccggcaaaattaaaagaatggggcgtgaccccgccaaaaacatgggcagaatttttagcgacagcgcaaacattaaagcggaaaggccttgaggcaccattggcactcggtgagaattggacacagcaacatctctgggaaagcgtcgccctcgccacactgggtgccgatggttggaataatctctggagtggtaagctcaaattcacggatccaaaagcagtcgccgtatgggaaacattcggtaaggtattagatgcagcgaacaaggatgcagccgggctttcatggcaacaagcagtagaccgtgtagtacaggggaaagctgcattcaatatcatgggggactgggcagcaggttacatgagtacgaccttaaaactgaagccaggtaccgacttcgcatggacaccttctccgggcacttcagggatctttatgatgctgtctgatagtttcggcttgccaaagggggcgaagaatcgtcaaaatgctattaactggttgaaactcgtcgggtcaaaagaggggcaggacaccttcaacccgctcaaaggttccatcgctgctcgtctcgattctgatcctgccaaatataatgcatacggccaaagtgcaatgaaggactggaagtcaaatcggatcgtaggctccctcgtccacggcgcagtcgcgccagaatccttcatgtcgcagtttgggacggtaatggagattttcttgcaatcccgtaacccgcaggcagccgctaatgccgcacaagctatcgccaatcaggtcggtttaggtcgtgggggttcacatcatcatcatcatcattaatgaaagggcgatatccagcacactggcggccgttactagtggatccggctgctaacaaagcccgaaaggaagctgagttggctgctgccaccgctgagcaataactagcataaccccttggggcctctaaacgggtcttgaggggttttttgctgaaaggaggaactatatccggagcgactcccacggcacgttggcaagctcg

SEQ ID NO: 88 - DNA, 1577 bp, Artificial Sequence
  Exemplary tsGBP2.13C.W9F expression sequence, optimized using OrfOpt
cggtcacgcttgggactgccataggctggcccggtgatgccggccacgatgcgtccggcgtagaggatcgagatctcgatcccgcgaaattaatacgactcactatagggagaccacaacggtttccctctagaaataattttgtttaactttaagaaggagatataccatgaaattagaaattttttcttggtttgcaggtgattgtggcccagctctcgaagccttgatccggttgtataaacagaaatacccaggtgtagaggtcattaatgctaccgtcaccgggggtgccggtgtcaacgccaaagccgtccttaaaacgcgtatgctcggcggggacccaccagatacctttcaagtacatgcagggcaggagctgatcggcacatgggtcgtcgccgaccgtatggaagatcttacctcattgtttcggcaggagggctggcttcaagcgttcccaaaaggtttaatcgatctcctcagttacaaaggtggcatttggtcagtcccagtcaacatccaccgttctaacgtaatgtggtacatcccggcaaaattaaaagaatggggcgtgaccccgccaaaaacatgggcagaatttttagcgacagcgcaaacattaaagcggaaaggccttgaggcaccattggcactcggtgagaattggacacagcaacatctctgggaaagcgtcgccctcgccacactgggtgccgatggttggaataatctctggagtggtaagctcaaattcacggatccaaaagcagtcgccgtatgggaaacattcggtaaggtattagatgcagcgaacaaggatgcagccgggctttcatggcaacaagcagtagaccgtgtagtacaggggaaagctgcattcaatatcatgggggactgggcagcaggttacatgagtacgaccttaaaactgaagccaggtaccgacttcgcatggacaccttctccgggcacttcagggatctttatgatgctgtctgatagtttcggcttgccaaagggggcgaagaatcgtcaaaatgctattaactggttgaaactcgtcgggtcaaaagaggggcaggacaccttcaacccgctcaaaggttccatcgctgctcgtctcgattctgatcctgccaaatataatgcatacggccaaagtgcaatgaaggactggaagtcaaatcggatcgtaggctccctcgtccacggcgcagtcgcgccagaatccttcatgtcgcagtttgggacggtaatggagattttcttgcaatcccgtaacccgcaggcagccgctaatgccgcacaagctatcgccaatcaggtcggtttaggtcgtgggggttcacatcatcatcatcatcattaatgaaagggcgatatccagcacactggcggccgttactagtggatccggctgctaacaaagcccgaaaggaagctgagttggctgctgccaccgctgagcaataactagcataaccccttggggcctctaaacgggtcttgaggggttttttgctgaaaggaggaactatatccggagcgactcccacggcacgttggcaagctcg

SEQ ID NO: 89 - DNA, 1577 bp, Artificial Sequence
  Exemplary tsGBP2.13C.W9M expression sequence, optimized using OrfOpt
cggtcacgcttgggactgccataggctggcccggtgatgccggccacgatgcgtccggcgtagaggatcgagatctcgatcccgcgaaattaatacgactcactatagggagaccacaacggtttccctctagaaataattttgtttaactttaagaaggagatataccatgaaattagaaattttttcttggatggcaggtgattgtggcccagctctcgaagccttgatccggttgtataaacagaaatacccaggtgtagaggtcattaatgctaccgtcaccgggggtgccggtgtcaacgccaaagccgtccttaaaacgcgtatgctcggcggggacccaccagatacctttcaagtacatgcagggcaggagctgatcggcacatgggtcgtcgccgaccgtatggaagatcttacctcattgtttcggcaggagggctggcttcaagcgttcccaaaaggtttaatcgatctcctcagttacaaaggtggcatttggtcagtcccagtcaacatccaccgttctaacgtaatgtggtacatcccggcaaaattaaaagaatggggcgtgaccccgccaaaaacatgggcagaatttttagcgacagcgcaaacattaaagcggaaaggccttgaggcaccattggcactcggtgagaattggacacagcaacatctctgggaaagcgtcgccctcgccacactgggtgccgatggttggaataatctctggagtggtaagctcaaattcacggatccaaaagcagtcgccgtatgggaaacattcggtaaggtattagatgcagcgaacaaggatgcagccgggctttcatggcaacaagcagtagaccgtgtagtacaggggaaagctgcattcaatatcatgggggactgggcagcaggttacatgagtacgaccttaaaactgaagccaggtaccgacttcgcatggacaccttctccgggcacttcagggatctttatgatgctgtctgatagtttcggcttgccaaagggggcgaagaatcgtcaaaatgctattaactggttgaaactcgtcgggtcaaaagaggggcaggacaccttcaacccgctcaaaggttccatcgctgctcgtctcgattctgatcctgccaaatataatgcatacggccaaagtgcaatgaaggactggaagtcaaatcggatcgtaggctccctcgtccacggcgcagtcgcgccagaatccttcatgtcgcagtttgggacggtaatggagattttcttgcaatcccgtaacccgcaggcagccgctaatgccgcacaagctatcgccaatcaggtcggtttaggtcgtgggggttcacatcatcatcatcatcattaatgaaagggcgatatccagcacactggcggccgttactagtggatccggctgctaacaaagcccgaaaggaagctgagttggctgctgccaccgctgagcaataactagcataaccccttggggcctctaaacgggtcttgaggggttttttgctgaaaggaggaactatatccggagcgactcccacggcacgttggcaagctcg

SEQ ID NO: 90 - DNA, 1577 bp, Artificial Sequence
  Exemplary tsGBP2.13C.W9Y expression sequence, optimized using OrfOpt
cggtcacgcttgggactgccataggctggcccggtgatgccggccacgatgcgtccggcgtagaggatcgagatctcgatcccgcgaaattaatacgactcactatagggagaccacaacggtttccctctagaaataattttgtttaactttaagaaggagatataccatgaaattagaaattttttcttggtatgcaggtgattgtggcccagctctcgaagccttgatccggttgtataaacagaaatacccaggtgtagaggtcattaatgctaccgtcaccgggggtgccggtgtcaacgccaaagccgtccttaaaacgcgtatgctcggcggggacccaccagatacctttcaagtacatgcagggcaggagctgatcggcacatgggtcgtcgccgaccgtatggaagatcttacctcattgtttcggcaggagggctggcttcaagcgttcccaaaaggtttaatcgatctcctcagttacaaaggtggcatttggtcagtcccagtcaacatccaccgttctaacgtaatgtggtacatcccggcaaaattaaaagaatggggcgtgaccccgccaaaaacatgggcagaatttttagcgacagcgcaaacattaaagcggaaaggccttgaggcaccattggcactcggtgagaattggacacagcaacatctctgggaaagcgtcgccctcgccacactgggtgccgatggttggaataatctctggagtggtaagctcaaattcacggatccaaaagcagtcgccgtatgggaaacattcggtaaggtattagatgcagcgaacaaggatgcagccgggctttcatggcaacaagcagtagaccgtgtagtacaggggaaagctgcattcaatatcatgggggactgggcagcaggttacatgagtacgaccttaaaactgaagccaggtaccgacttcgcatggacaccttctccgggcacttcagggatctttatgatgctgtctgatagtttcggcttgccaaagggggcgaagaatcgtcaaaatgctattaactggttgaaactcgtcgggtcaaaagaggggcaggacaccttcaacccgctcaaaggttccatcgctgctcgtctcgattctgatcctgccaaatataatgcatacggccaaagtgcaatgaaggactggaagtcaaatcggatcgtaggctccctcgtccacggcgcagtcgcgccagaatccttcatgtcgcagtttgggacggtaatggagattttcttgcaatcccgtaacccgcaggcagccgctaatgccgcacaagctatcgccaatcaggtcggtttaggtcgtgggggttcacatcatcatcatcatcattaatgaaagggcgatatccagcacactggcggccgttactagtggatccggctgctaacaaagcccgaaaggaagctgagttggctgctgccaccgctgagcaataactagcataaccccttggggcctctaaacgggtcttgaggggttttttgctgaaaggaggaactatatccggagcgactcccacggcacgttggcaagctcg

SEQ ID NO: 91 - DNA, 1577 bp, Artificial Sequence
  Exemplary tsGBP2.13C.Q64N expression sequence, optimized using OrfOpt
cggtcacgcttgggactgccataggctggcccggtgatgccggccacgatgcgtccggcgtagaggatcgagatctcgatcccgcgaaattaatacgactcactatagggagaccacaacggtttccctctagaaataattttgtttaactttaagaaggagatataccatgaaattagaaattttttcttggtgggcaggtgattgtggcccagctctcgaagccttgatccggttgtataaacagaaatacccaggtgtagaggtcattaatgctaccgtcaccgggggtgccggtgtcaacgccaaagccgtccttaaaacgcgtatgctcggcggggacccaccagatacctttaacgtacatgcagggcaggagctgatcggcacatgggtcgtcgccgaccgtatggaagatcttacctcattgtttcggcaggagggctggcttcaagcgttcccaaaaggtttaatcgatctcctcagttacaaaggtggcatttggtcagtcccagtcaacatccaccgttctaacgtaatgtggtacatcccggcaaaattaaaagaatggggcgtgaccccgccaaaaacatgggcagaatttttagcgacagcgcaaacattaaagcggaaaggccttgaggcaccattggcactcggtgagaattggacacagcaacatctctgggaaagcgtcgccctcgccacactgggtgccgatggttggaataatctctggagtggtaagctcaaattcacggatccaaaagcagtcgccgtatgggaaacattcggtaaggtattagatgcagcgaacaaggatgcagccgggctttcatggcaacaagcagtagaccgtgtagtacaggggaaagctgcattcaatatcatgggggactgggcagcaggttacatgagtacgaccttaaaactgaagccaggtaccgacttcgcatggacaccttctccgggcacttcagggatctttatgatgctgtctgatagtttcggcttgccaaagggggcgaagaatcgtcaaaatgctattaactggttgaaactcgtcgggtcaaaagaggggcaggacaccttcaacccgctcaaaggttccatcgctgctcgtctcgattctgatcctgccaaatataatgcatacggccaaagtgcaatgaaggactggaagtcaaatcggatcgtaggctccctcgtccacggcgcagtcgcgccagaatccttcatgtcgcagtttgggacggtaatggagattttcttgcaatcccgtaacccgcaggcagccgctaatgccgcacaagctatcgccaatcaggtcggtttaggtcgtgggggttcacatcatcatcatcatcattaatgaaagggcgatatccagcacactggcggccgttactagtggatccggctgctaacaaagcccgaaaggaagctgagttggctgctgccaccgctgagcaataactagcataaccccttggggcctctaaacgggtcttgaggggttttttgctgaaaggaggaactatatccggagcgactcccacggcacgttggcaagctcg

SEQ ID NO: 92 - DNA, 1577 bp, Artificial Sequence
  Exemplary tsGBP2.13C.Q64E expression sequence, optimized using OrfOpt
cggtcacgcttgggactgccataggctggcccggtgatgccggccacgatgcgtccggcgtagaggatcgagatctcgatcccgcgaaattaatacgactcactatagggagaccacaacggtttccctctagaaataattttgtttaactttaagaaggagatataccatgaaattagaaattttttcttggtgggcaggtgattgtggcccagctctcgaagccttgatccggttgtataaacagaaatacccaggtgtagaggtcattaatgctaccgtcaccgggggtgccggtgtcaacgccaaagccgtccttaaaacgcgtatgctcggcggggacccaccagatacctttgaagtacatgcagggcaggagctgatcggcacatgggtcgtcgccgaccgtatggaagatcttacctcattgtttcggcaggagggctggcttcaagcgttcccaaaaggtttaatcgatctcctcagttacaaaggtggcatttggtcagtcccagtcaacatccaccgttctaacgtaatgtggtacatcccggcaaaattaaaagaatggggcgtgaccccgccaaaaacatgggcagaatttttagcgacagcgcaaacattaaagcggaaaggccttgaggcaccattggcactcggtgagaattggacacagcaacatctctgggaaagcgtcgccctcgccacactgggtgccgatggttggaataatctctggagtggtaagctcaaattcacggatccaaaagcagtcgccgtatgggaaacattcggtaaggtattagatgcagcgaacaaggatgcagccgggctttcatggcaacaagcagtagaccgtgtagtacaggggaaagctgcattcaatatcatgggggactgggcagcaggttacatgagtacgaccttaaaactgaagccaggtaccgacttcgcatggacaccttctccgggcacttcagggatctttatgatgctgtctgatagtttcggcttgccaaagggggcgaagaatcgtcaaaatgctattaactggttgaaactcgtcgggtcaaaagaggggcaggacaccttcaacccgctcaaaggttccatcgctgctcgtctcgattctgatcctgccaaatataatgcatacggccaaagtgcaatgaaggactggaagtcaaatcggatcgtaggctccctcgtccacggcgcagtcgcgccagaatccttcatgtcgcagtttgggacggtaatggagattttcttgcaatcccgtaacccgcaggcagccgctaatgccgcacaagctatcgccaatcaggtcggtttaggtcgtgggggttcacatcatcatcatcatcattaatgaaagggcgatatccagcacactggcggccgttactagtggatccggctgctaacaaagcccgaaaggaagctgagttggctgctgccaccgctgagcaataactagcataaccccttggggcctctaaacgggtcttgaggggttttttgctgaaaggaggaactatatccggagcgactcccacggcacgttggcaagctcg

SEQ ID NO: 93 - DNA, 1577 bp, Artificial Sequence
  Exemplary tsGBP2.13C.Q64M expression sequence, optimized using OrfOpt
cggtcacgcttgggactgccataggctggcccggtgatgccggccacgatgcgtccggcgtagaggatcgagatctcgatcccgcgaaattaatacgactcactatagggagaccacaacggtttccctctagaaataattttgtttaactttaagaaggagatataccatgaaattagaaattttttcttggtgggcaggtgattgtggcccagctctcgaagccttgatccggttgtataaacagaaatacccaggtgtagaggtcattaatgctaccgtcaccgggggtgccggtgtcaacgccaaagccgtccttaaaacgcgtatgctcggcggggacccaccagatacctttatggtacatgcagggcaggagctgatcggcacatgggtcgtcgccgaccgtatggaagatcttacctcattgtttcggcaggagggctggcttcaagcgttcccaaaaggtttaatcgatctcctcagttacaaaggtggcatttggtcagtcccagtcaacatccaccgttctaacgtaatgtggtacatcccggcaaaattaaaagaatggggcgtgaccccgccaaaaacatgggcagaatttttagcgacagcgcaaacattaaagcggaaaggccttgaggcaccattggcactcggtgagaattggacacagcaacatctctgggaaagcgtcgccctcgccacactgggtgccgatggttggaataatctctggagtggtaagctcaaattcacggatccaaaagcagtcgccgtatgggaaacattcggtaaggtattagatgcagcgaacaaggatgcagccgggctttcatggcaacaagcagtagaccgtgtagtacaggggaaagctgcattcaatatcatgggggactgggcagcaggttacatgagtacgaccttaaaactgaagccaggtaccgacttcgcatggacaccttctccgggcacttcagggatctttatgatgctgtctgatagtttcggcttgccaaagggggcgaagaatcgtcaaaatgctattaactggttgaaactcgtcgggtcaaaagaggggcaggacaccttcaacccgctcaaaggttccatcgctgctcgtctcgattctgatcctgccaaatataatgcatacggccaaagtgcaatgaaggactggaagtcaaatcggatcgtaggctccctcgtccacggcgcagtcgcgccagaatccttcatgtcgcagtttgggacggtaatggagattttcttgcaatcccgtaacccgcaggcagccgctaatgccgcacaagctatcgccaatcaggtcggtttaggtcgtgggggttcacatcatcatcatcatcattaatgaaagggcgatatccagcacactggcggccgttactagtggatccggctgctaacaaagcccgaaaggaagctgagttggctgctgccaccgctgagcaataactagcataaccccttggggcctctaaacgggtcttgaggggttttttgctgaaaggaggaactatatccggagcgactcccacggcacgttggcaagctcg

SEQ ID NO: 94 - DNA, 1577 bp, Artificial Sequence
  Exemplary tsGBP2.13C.H66Q expression sequence, optimized using OrfOpt
cggtcacgcttgggactgccataggctggcccggtgatgccggccacgatgcgtccggcgtagaggatcgagatctcgatcccgcgaaattaatacgactcactatagggagaccacaacggtttccctctagaaataattttgtttaactttaagaaggagatataccatgaaattagaaattttttcttggtgggcaggtgattgtggcccagctctcgaagccttgatccggttgtataaacagaaatacccaggtgtagaggtcattaatgctaccgtcaccgggggtgccggtgtcaacgccaaagccgtccttaaaacgcgtatgctcggcggggacccaccagatacctttcaagtacaggcagggcaggagctgatcggcacatgggtcgtcgccgaccgtatggaagatcttacctcattgtttcggcaggagggctggcttcaagcgttcccaaaaggtttaatcgatctcctcagttacaaaggtggcatttggtcagtcccagtcaacatccaccgttctaacgtaatgtggtacatcccggcaaaattaaaagaatggggcgtgaccccgccaaaaacatgggcagaatttttagcgacagcgcaaacattaaagcggaaaggccttgaggcaccattggcactcggtgagaattggacacagcaacatctctgggaaagcgtcgccctcgccacactgggtgccgatggttggaataatctctggagtggtaagctcaaattcacggatccaaaagcagtcgccgtatgggaaacattcggtaaggtattagatgcagcgaacaaggatgcagccgggctttcatggcaacaagcagtagaccgtgtagtacaggggaaagctgcattcaatatcatgggggactgggcagcaggttacatgagtacgaccttaaaactgaagccaggtaccgacttcgcatggacaccttctccgggcacttcagggatctttatgatgctgtctgatagtttcggcttgccaaagggggcgaagaatcgtcaaaatgctattaactggttgaaactcgtcgggtcaaaagaggggcaggacaccttcaacccgctcaaaggttccatcgctgctcgtctcgattctgatcctgccaaatataatgcatacggccaaagtgcaatgaaggactggaagtcaaatcggatcgtaggctccctcgtccacggcgcagtcgcgccagaatccttcatgtcgcagtttgggacggtaatggagattttcttgcaatcccgtaacccgcaggcagccgctaatgccgcacaagctatcgccaatcaggtcggtttaggtcgtgggggttcacatcatcatcatcatcattaatgaaagggcgatatccagcacactggcggccgttactagtggatccggctgctaacaaagcccgaaaggaagctgagttggctgctgccaccgctgagcaataactagcataaccccttggggcctctaaacgggtcttgaggggttttttgctgaaaggaggaactatatccggagcgactcccacggcacgttggcaagctcg

SEQ ID NO: 95 - DNA, 1577 bp, Artificial Sequence
  Exemplary tsGBP2.13C.W244M expression sequence, optimized using OrfOpt
cggtcacgcttgggactgccataggctggcccggtgatgccggccacgatgcgtccggcgtagaggatcgagatctcgatcccgcgaaattaatacgactcactatagggagaccacaacggtttccctctagaaataattttgtttaactttaagaaggagatataccatgaaattagaaattttttcttggtgggcaggtgattgtggcccagctctcgaagccttgatccggttgtataaacagaaatacccaggtgtagaggtcattaatgctaccgtcaccgggggtgccggtgtcaacgccaaagccgtccttaaaacgcgtatgctcggcggggacccaccagatacctttcaagtacatgcagggcaggagctgatcggcacatgggtcgtcgccgaccgtatggaagatcttacctcattgtttcggcaggagggctggcttcaagcgttcccaaaaggtttaatcgatctcctcagttacaaaggtggcatttggtcagtcccagtcaacatccaccgttctaacgtaatgtggtacatcccggcaaaattaaaagaatggggcgtgaccccgccaaaaacatgggcagaatttttagcgacagcgcaaacattaaagcggaaaggccttgaggcaccattggcactcggtgagaattggacacagcaacatctctgggaaagcgtcgccctcgccacactgggtgccgatggttggaataatctctggagtggtaagctcaaattcacggatccaaaagcagtcgccgtatgggaaacattcggtaaggtattagatgcagcgaacaaggatgcagccgggctttcatggcaacaagcagtagaccgtgtagtacaggggaaagctgcattcaatatcatgggggacatggcagcaggttacatgagtacgaccttaaaactgaagccaggtaccgacttcgcatggacaccttctccgggcacttcagggatctttatgatgctgtctgatagtttcggcttgccaaagggggcgaagaatcgtcaaaatgctattaactggttgaaactcgtcgggtcaaaagaggggcaggacaccttcaacccgctcaaaggttccatcgctgctcgtctcgattctgatcctgccaaatataatgcatacggccaaagtgcaatgaaggactggaagtcaaatcggatcgtaggctccctcgtccacggcgcagtcgcgccagaatccttcatgtcgcagtttgggacggtaatggagattttcttgcaatcccgtaacccgcaggcagccgctaatgccgcacaagctatcgccaatcaggtcggtttaggtcgtgggggttcacatcatcatcatcatcattaatgaaagggcgatatccagcacactggcggccgttactagtggatccggctgctaacaaagcccgaaaggaagctgagttggctgctgccaccgctgagcaataactagcataaccccttggggcctctaaacgggtcttgaggggttttttgctgaaaggaggaactatatccggagcgactcccacggcacgttggcaagctcg

SEQ ID NO: 96 - DNA, 1577 bp, Artificial Sequence
  Exemplary tsGBP2.13C.W244F expression sequence, optimized using OrfOpt
cggtcacgcttgggactgccataggctggcccggtgatgccggccacgatgcgtccggcgtagaggatcgagatctcgatcccgcgaaattaatacgactcactatagggagaccacaacggtttccctctagaaataattttgtttaactttaagaaggagatataccatgaaattagaaattttttcttggtgggcaggtgattgtggcccagctctcgaagccttgatccggttgtataaacagaaatacccaggtgtagaggtcattaatgctaccgtcaccgggggtgccggtgtcaacgccaaagccgtccttaaaacgcgtatgctcggcggggacccaccagatacctttcaagtacatgcagggcaggagctgatcggcacatgggtcgtcgccgaccgtatggaagatcttacctcattgtttcggcaggagggctggcttcaagcgttcccaaaaggtttaatcgatctcctcagttacaaaggtggcatttggtcagtcccagtcaacatccaccgttctaacgtaatgtggtacatcccggcaaaattaaaagaatggggcgtgaccccgccaaaaacatgggcagaatttttagcgacagcgcaaacattaaagcggaaaggccttgaggcaccattggcactcggtgagaattggacacagcaacatctctgggaaagcgtcgccctcgccacactgggtgccgatggttggaataatctctggagtggtaagctcaaattcacggatccaaaagcagtcgccgtatgggaaacattcggtaaggtattagatgcagcgaacaaggatgcagccgggctttcatggcaacaagcagtagaccgtgtagtacaggggaaagctgcattcaatatcatgggggactttgcagcaggttacatgagtacgaccttaaaactgaagccaggtaccgacttcgcatggacaccttctccgggcacttcagggatctttatgatgctgtctgatagtttcggcttgccaaagggggcgaagaatcgtcaaaatgctattaactggttgaaactcgtcgggtcaaaagaggggcaggacaccttcaacccgctcaaaggttccatcgctgctcgtctcgattctgatcctgccaaatataatgcatacggccaaagtgcaatgaaggactggaagtcaaatcggatcgtaggctccctcgtccacggcgcagtcgcgccagaatccttcatgtcgcagtttgggacggtaatggagattttcttgcaatcccgtaacccgcaggcagccgctaatgccgcacaagctatcgccaatcaggtcggtttaggtcgtgggggttcacatcatcatcatcatcattaatgaaagggcgatatccagcacactggcggccgttactagtggatccggctgctaacaaagcccgaaaggaagctgagttggctgctgccaccgctgagcaataactagcataaccccttggggcctctaaacgggtcttgaggggttttttgctgaaaggaggaactatatccggagcgactcccacggcacgttggcaagctcg

SEQ ID NO: 97 - DNA, 1577 bp, Artificial Sequence
  Exemplary tsGBP2.13C.W244Y expression sequence, optimized using OrfOpt
cggtcacgcttgggactgccataggctggcccggtgatgccggccacgatgcgtccggcgtagaggatcgagatctcgatcccgcgaaattaatacgactcactatagggagaccacaacggtttccctctagaaataattttgtttaactttaagaaggagatataccatgaaattagaaattttttcttggtgggcaggtgattgtggcccagctctcgaagccttgatccggttgtataaacagaaatacccaggtgtagaggtcattaatgctaccgtcaccgggggtgccggtgtcaacgccaaagccgtccttaaaacgcgtatgctcggcggggacccaccagatacctttcaagtacatgcagggcaggagctgatcggcacatgggtcgtcgccgaccgtatggaagatcttacctcattgtttcggcaggagggctggcttcaagcgttcccaaaaggtttaatcgatctcctcagttacaaaggtggcatttggtcagtcccagtcaacatccaccgttctaacgtaatgtggtacatcccggcaaaattaaaagaatggggcgtgaccccgccaaaaacatgggcagaatttttagcgacagcgcaaacattaaagcggaaaggccttgaggcaccattggcactcggtgagaattggacacagcaacatctctgggaaagcgtcgccctcgccacactgggtgccgatggttggaataatctctggagtggtaagctcaaattcacggatccaaaagcagtcgccgtatgggaaacattcggtaaggtattagatgcagcgaacaaggatgcagccgggctttcatggcaacaagcagtagaccgtgtagtacaggggaaagctgcattcaatatcatgggggactatgcagcaggttacatgagtacgaccttaaaactgaagccaggtaccgacttcgcatggacaccttctccgggcacttcagggatctttatgatgctgtctgatagtttcggcttgccaaagggggcgaagaatcgtcaaaatgctattaactggttgaaactcgtcgggtcaaaagaggggcaggacaccttcaacccgctcaaaggttccatcgctgctcgtctcgattctgatcctgccaaatataatgcatacggccaaagtgcaatgaaggactggaagtcaaatcggatcgtaggctccctcgtccacggcgcagtcgcgccagaatccttcatgtcgcagtttgggacggtaatggagattttcttgcaatcccgtaacccgcaggcagccgctaatgccgcacaagctatcgccaatcaggtcggtttaggtcgtgggggttcacatcatcatcatcatcattaatgaaagggcgatatccagcacactggcggccgttactagtggatccggctgctaacaaagcccgaaaggaagctgagttggctgctgccaccgctgagcaataactagcataaccccttggggcctctaaacgggtcttgaggggttttttgctgaaaggaggaactatatccggagcgactcccacggcacgttggcaagctcg

SEQ ID NO: 98 - DNA, 1577 bp, Artificial Sequence
  Exemplary tsGBP2.13C.D278N expression sequence, optimized using OrfOpt
cggtcacgcttgggactgccataggctggcccggtgatgccggccacgatgcgtccggcgtagaggatcgagatctcgatcccgcgaaattaatacgactcactatagggagaccacaacggtttccctctagaaataattttgtttaactttaagaaggagatataccatgaaattagaaattttttcttggtgggcaggtgattgtggcccagctctcgaagccttgatccggttgtataaacagaaatacccaggtgtagaggtcattaatgctaccgtcaccgggggtgccggtgtcaacgccaaagccgtccttaaaacgcgtatgctcggcggggacccaccagatacctttcaagtacatgcagggcaggagctgatcggcacatgggtcgtcgccgaccgtatggaagatcttacctcattgtttcggcaggagggctggcttcaagcgttcccaaaaggtttaatcgatctcctcagttacaaaggtggcatttggtcagtcccagtcaacatccaccgttctaacgtaatgtggtacatcccggcaaaattaaaagaatggggcgtgaccccgccaaaaacatgggcagaatttttagcgacagcgcaaacattaaagcggaaaggccttgaggcaccattggcactcggtgagaattggacacagcaacatctctgggaaagcgtcgccctcgccacactgggtgccgatggttggaataatctctggagtggtaagctcaaattcacggatccaaaagcagtcgccgtatgggaaacattcggtaaggtattagatgcagcgaacaaggatgcagccgggctttcatggcaacaagcagtagaccgtgtagtacaggggaaagctgcattcaatatcatgggggactgggcagcaggttacatgagtacgaccttaaaactgaagccaggtaccgacttcgcatggacaccttctccgggcacttcagggatctttatgatgctgtctaacagtttcggcttgccaaagggggcgaagaatcgtcaaaatgctattaactggttgaaactcgtcgggtcaaaagaggggcaggacaccttcaacccgctcaaaggttccatcgctgctcgtctcgattctgatcctgccaaatataatgcatacggccaaagtgcaatgaaggactggaagtcaaatcggatcgtaggctccctcgtccacggcgcagtcgcgccagaatccttcatgtcgcagtttgggacggtaatggagattttcttgcaatcccgtaacccgcaggcagccgctaatgccgcacaagctatcgccaatcaggtcggtttaggtcgtgggggttcacatcatcatcatcatcattaatgaaagggcgatatccagcacactggcggccgttactagtggatccggctgctaacaaagcccgaaaggaagctgagttggctgctgccaccgctgagcaataactagcataaccccttggggcctctaaacgggtcttgaggggttttttgctgaaaggaggaactatatccggagcgactcccacggcacgttggcaagctcg

SEQ ID NO: 99 - DNA, 1577 bp, Artificial Sequence
  Exemplary tsGBP2.13C.D278S expression sequence, optimized using OrfOpt
cggtcacgcttgggactgccataggctggcccggtgatgccggccacgatgcgtccggcgtagaggatcgagatctcgatcccgcgaaattaatacgactcactatagggagaccacaacggtttccctctagaaataattttgtttaactttaagaaggagatataccatgaaattagaaattttttcttggtgggcaggtgattgtggcccagctctcgaagccttgatccggttgtataaacagaaatacccaggtgtagaggtcattaatgctaccgtcaccgggggtgccggtgtcaacgccaaagccgtccttaaaacgcgtatgctcggcggggacccaccagatacctttcaagtacatgcagggcaggagctgatcggcacatgggtcgtcgccgaccgtatggaagatcttacctcattgtttcggcaggagggctggcttcaagcgttcccaaaaggtttaatcgatctcctcagttacaaaggtggcatttggtcagtcccagtcaacatccaccgttctaacgtaatgtggtacatcccggcaaaattaaaagaatggggcgtgaccccgccaaaaacatgggcagaatttttagcgacagcgcaaacattaaagcggaaaggccttgaggcaccattggcactcggtgagaattggacacagcaacatctctgggaaagcgtcgccctcgccacactgggtgccgatggttggaataatctctggagtggtaagctcaaattcacggatccaaaagcagtcgccgtatgggaaacattcggtaaggtattagatgcagcgaacaaggatgcagccgggctttcatggcaacaagcagtagaccgtgtagtacaggggaaagctgcattcaatatcatgggggactgggcagcaggttacatgagtacgaccttaaaactgaagccaggtaccgacttcgcatggacaccttctccgggcacttcagggatctttatgatgctgtctagcagtttcggcttgccaaagggggcgaagaatcgtcaaaatgctattaactggttgaaactcgtcgggtcaaaagaggggcaggacaccttcaacccgctcaaaggttccatcgctgctcgtctcgattctgatcctgccaaatataatgcatacggccaaagtgcaatgaaggactggaagtcaaatcggatcgtaggctccctcgtccacggcgcagtcgcgccagaatccttcatgtcgcagtttgggacggtaatggagattttcttgcaatcccgtaacccgcaggcagccgctaatgccgcacaagctatcgccaatcaggtcggtttaggtcgtgggggttcacatcatcatcatcatcattaatgaaagggcgatatccagcacactggcggccgttactagtggatccggctgctaacaaagcccgaaaggaagctgagttggctgctgccaccgctgagcaataactagcataaccccttggggcctctaaacgggtcttgaggggttttttgctgaaaggaggaactatatccggagcgactcccacggcacgttggcaagctcg

SEQ ID NO: 100 - DNA, 1577 bp, Artificial Sequence
  Exemplary tsGBP2.13C.D278L expression sequence, optimized using OrfOpt
cggtcacgcttgggactgccataggctggcccggtgatgccggccacgatgcgtccggcgtagaggatcgagatctcgatcccgcgaaattaatacgactcactatagggagaccacaacggtttccctctagaaataattttgtttaactttaagaaggagatataccatgaaattagaaattttttcttggtgggcaggtgattgtggcccagctctcgaagccttgatccggttgtataaacagaaatacccaggtgtagaggtcattaatgctaccgtcaccgggggtgccggtgtcaacgccaaagccgtccttaaaacgcgtatgctcggcggggacccaccagatacctttcaagtacatgcagggcaggagctgatcggcacatgggtcgtcgccgaccgtatggaagatcttacctcattgtttcggcaggagggctggcttcaagcgttcccaaaaggtttaatcgatctcctcagttacaaaggtggcatttggtcagtcccagtcaacatccaccgttctaacgtaatgtggtacatcccggcaaaattaaaagaatggggcgtgaccccgccaaaaacatgggcagaatttttagcgacagcgcaaacattaaagcggaaaggccttgaggcaccattggcactcggtgagaattggacacagcaacatctctgggaaagcgtcgccctcgccacactgggtgccgatggttggaataatctctggagtggtaagctcaaattcacggatccaaaagcagtcgccgtatgggaaacattcggtaaggtattagatgcagcgaacaaggatgcagccgggctttcatggcaacaagcagtagaccgtgtagtacaggggaaagctgcattcaatatcatgggggactgggcagcaggttacatgagtacgaccttaaaactgaagccaggtaccgacttcgcatggacaccttctccgggcacttcagggatctttatgatgctgtctctgagtttcggcttgccaaagggggcgaagaatcgtcaaaatgctattaactggttgaaactcgtcgggtcaaaagaggggcaggacaccttcaacccgctcaaaggttccatcgctgctcgtctcgattctgatcctgccaaatataatgcatacggccaaagtgcaatgaaggactggaagtcaaatcggatcgtaggctccctcgtccacggcgcagtcgcgccagaatccttcatgtcgcagtttgggacggtaatggagattttcttgcaatcccgtaacccgcaggcagccgctaatgccgcacaagctatcgccaatcaggtcggtttaggtcgtgggggttcacatcatcatcatcatcattaatgaaagggcgatatccagcacactggcggccgttactagtggatccggctgctaacaaagcccgaaaggaagctgagttggctgctgccaccgctgagcaataactagcataaccccttggggcctctaaacgggtcttgaggggttttttgctgaaaggaggaactatatccggagcgactcccacggcacgttggcaagctcg

SEQ ID NO: 101 - DNA, 1577 bp, Artificial Sequence
  Exemplary tsGBP2.13C.K312M expression sequence, optimized using OrfOpt
cggtcacgcttgggactgccataggctggcccggtgatgccggccacgatgcgtccggcgtagaggatcgagatctcgatcccgcgaaattaatacgactcactatagggagaccacaacggtttccctctagaaataattttgtttaactttaagaaggagatataccatgaaattagaaattttttcttggtgggcaggtgattgtggcccagctctcgaagccttgatccggttgtataaacagaaatacccaggtgtagaggtcattaatgctaccgtcaccgggggtgccggtgtcaacgccaaagccgtccttaaaacgcgtatgctcggcggggacccaccagatacctttcaagtacatgcagggcaggagctgatcggcacatgggtcgtcgccgaccgtatggaagatcttacctcattgtttcggcaggagggctggcttcaagcgttcccaaaaggtttaatcgatctcctcagttacaaaggtggcatttggtcagtcccagtcaacatccaccgttctaacgtaatgtggtacatcccggcaaaattaaaagaatggggcgtgaccccgccaaaaacatgggcagaatttttagcgacagcgcaaacattaaagcggaaaggccttgaggcaccattggcactcggtgagaattggacacagcaacatctctgggaaagcgtcgccctcgccacactgggtgccgatggttggaataatctctggagtggtaagctcaaattcacggatccaaaagcagtcgccgtatgggaaacattcggtaaggtattagatgcagcgaacaaggatgcagccgggctttcatggcaacaagcagtagaccgtgtagtacaggggaaagctgcattcaatatcatgggggactgggcagcaggttacatgagtacgaccttaaaactgaagccaggtaccgacttcgcatggacaccttctccgggcacttcagggatctttatgatgctgtctgatagtttcggcttgccaaagggggcgaagaatcgtcaaaatgctattaactggttgaaactcgtcgggtcaaaagaggggcaggacaccttcaacccgctcatgggttccatcgctgctcgtctcgattctgatcctgccaaatataatgcatacggccaaagtgcaatgaaggactggaagtcaaatcggatcgtaggctccctcgtccacggcgcagtcgcgccagaatccttcatgtcgcagtttgggacggtaatggagattttcttgcaatcccgtaacccgcaggcagccgctaatgccgcacaagctatcgccaatcaggtcggtttaggtcgtgggggttcacatcatcatcatcatcattaatgaaagggcgatatccagcacactggcggccgttactagtggatccggctgctaacaaagcccgaaaggaagctgagttggctgctgccaccgctgagcaataactagcataaccccttggggcctctaaacgggtcttgaggggttttttgctgaaaggaggaactatatccggagcgactcccacggcacgttggcaagctcg

SEQ ID NO: 102 - DNA, 1649 bp, Artificial Sequence
  Exemplary tsGBP2.13C.bZif expression sequence, optimized using OrfOpt
cggtcacgcttgggactgccataggctggcccggtgatgccggccacgatgcgtccggcgtagaggatcgagatctcgatcccgcgaaattaatacgactcactatagggagaccacaacggtttccctctagaaataattttgtttaactttaagaaggagatataccatgaaattagaaattttttcttggtgggcaggtgattgcggcccagctctcgaagccttgatccggttgtataaacagaaatacccaggtgtagaggtcattaatgctaccgtcaccgggggtgccggtgtcaacgccaaagccgtccttaaaacgcgtatgctcggcggggacccaccagatacctttcaagtacatgcagggcaggagctgatcggcacatgggtcgtcgccgaccgtatggaagatcttacctcattgtttcggcaggagggctggcttcaagcgttcccaaaaggtttaatcgatctcctcagttacaaaggtggcatttggtcagtcccagtcaacatccaccgttctaacgtaatgtggtacatcccggcaaaattaaaagaatggggcgtgaccccgccaaaaacatgggcagaatttttagcgacagcgcaaacattaaagcggaaaggccttgaggcaccattggcactcggtgagaattggacacagcaacatctctgggaaagcgtcgccctcgccacactgggtgccgatggttggaataatctctggagtggtaagctcaaattcacggatccaaaagcagtcgccgtatgggaaacattcggtaaggtattagatgcagcgaacaaggatgcagccgggctttcatggcaacaagcagtagaccgtgtagtacaggggaaagctgcattcaatatcatgggggactgggcagcaggttacatgagtacgaccttaaaactgaagccaggtaccgacttcgcatggacaccttctccgggcacttcagggatctttatgatgctgtctgatagtttcggcttgccaaagggggcgaagaatcgtcaaaatgctattaactggttgaaactcgtcgggtcaaaagaggggcaggacaccttcaacccgctcaaaggttccatcgctgctcgtctcgattctgatcctgccaaatataatgcatacggccaaagtgcaatgaaggactggaagtcaaatcggatcgtaggctccctcgtccacggcgcagtcgcgccagaatccttcatgtcgcagtttgggacggtaatggagattttcttgcaatcccgtaacccgcaggcagccgctaatgccgcacaagctatcgccaatcaggtcggtttaggtcgtggcggcagcggcggcagcaccggcgaaaaaccgtataaatgcccggaatgcggcaaaagctttagccgcagcgggggttcacatcatcatcatcatcattaatgaaagggcgatatccagcacactggcggccgttactagtggatccggctgctaacaaagcccgaaaggaagctgagttggctgctgccaccgctgagcaataactagcataaccccttggggcctctaaacgggtcttgaggggttttttgctgaaaggaggaactatatccggagcgactcccacggcacgttggcaagctcg

SEQ ID NO: 103 - DNA, 1649 bp, Artificial Sequence
  Exemplary tsGBP2.244C.bZif expression sequence, optimized using OrfOpt
cggtcacgcttgggactgccataggctggcccggtgatgccggccacgatgcgtccggcgtagaggatcgagatctcgatcccgcgaaattaatacgactcactatagggagaccacaacggtttccctctagaaataattttgtttaactttaagaaggagatataccatgaaattagaaattttttcttggtgggcaggtgatgaaggcccagctctcgaagccttgatccggttgtataaacagaaatacccaggtgtagaggtcattaatgctaccgtcaccgggggtgccggtgtcaacgccaaagccgtccttaaaacgcgtatgctcggcggggacccaccagatacctttcaagtacatgcagggcaggagctgatcggcacatgggtcgtcgccgaccgtatggaagatcttacctcattgtttcggcaggagggctggcttcaagcgttcccaaaaggtttaatcgatctcctcagttacaaaggtggcatttggtcagtcccagtcaacatccaccgttctaacgtaatgtggtacatcccggcaaaattaaaagaatggggcgtgaccccgccaaaaacatgggcagaatttttagcgacagcgcaaacattaaagcggaaaggccttgaggcaccattggcactcggtgagaattggacacagcaacatctctgggaaagcgtcgccctcgccacactgggtgccgatggttggaataatctctggagtggtaagctcaaattcacggatccaaaagcagtcgccgtatgggaaacattcggtaaggtattagatgcagcgaacaaggatgcagccgggctttcatggcaacaagcagtagaccgtgtagtacaggggaaagctgcattcaatatcatgggggactgcgcagcaggttacatgagtacgaccttaaaactgaagccaggtaccgacttcgcatggacaccttctccgggcacttcagggatctttatgatgctgtctgatagtttcggcttgccaaagggggcgaagaatcgtcaaaatgctattaactggttgaaactcgtcgggtcaaaagaggggcaggacaccttcaacccgctcaaaggttccatcgctgctcgtctcgattctgatcctgccaaatataatgcatacggccaaagtgcaatgaaggactggaagtcaaatcggatcgtaggctccctcgtccacggcgcagtcgcgccagaatccttcatgtcgcagtttgggacggtaatggagattttcttgcaatcccgtaacccgcaggcagccgctaatgccgcacaagctatcgccaatcaggtcggtttaggtcgtggcggcagcggcggcagcaccggcgaaaaaccgtataaatgcccggaatgcggcaaaagctttagccgcagcgggggttcacatcatcatcatcatcattaatgaaagggcgatatccagcacactggcggccgttactagtggatccggctgctaacaaagcccgaaaggaagctgagttggctgctgccaccgctgagcaataactagcataaccccttggggcctctaaacgggtcttgaggggttttttgctgaaaggaggaactatatccggagcgactcccacggcacgttggcaagctcg

SEQ ID NO: 104 - DNA, 1649 bp, Artificial Sequence
  Exemplary tsGBP2.13C_244F.bZif expression sequence, optimized using OrfOpt
cggtcacgcttgggactgccataggctggcccggtgatgccggccacgatgcgtccggcgtagaggatcgagatctcgatcccgcgaaattaatacgactcactatagggagaccacaacggtttccctctagaaataattttgtttaactttaagaaggagatataccatgaaattagaaattttttcttggtgggcaggtgattgcggcccagctctcgaagccttgatccggttgtataaacagaaatacccaggtgtagaggtcattaatgctaccgtcaccgggggtgccggtgtcaacgccaaagccgtccttaaaacgcgtatgctcggcggggacccaccagatacctttcaagtacatgcagggcaggagctgatcggcacatgggtcgtcgccgaccgtatggaagatcttacctcattgtttcggcaggagggctggcttcaagcgttcccaaaaggtttaatcgatctcctcagttacaaaggtggcatttggtcagtcccagtcaacatccaccgttctaacgtaatgtggtacatcccggcaaaattaaaagaatggggcgtgaccccgccaaaaacatgggcagaatttttagcgacagcgcaaacattaaagcggaaaggccttgaggcaccattggcactcggtgagaattggacacagcaacatctctgggaaagcgtcgccctcgccacactgggtgccgatggttggaataatctctggagtggtaagctcaaattcacggatccaaaagcagtcgccgtatgggaaacattcggtaaggtattagatgcagcgaacaaggatgcagccgggctttcatggcaacaagcagtagaccgtgtagtacaggggaaagctgcattcaatatcatgggggactttgcagcaggttacatgagtacgaccttaaaactgaagccaggtaccgacttcgcatggacaccttctccgggcacttcagggatctttatgatgctgtctgatagtttcggcttgccaaagggggcgaagaatcgtcaaaatgctattaactggttgaaactcgtcgggtcaaaagaggggcaggacaccttcaacccgctcaaaggttccatcgctgctcgtctcgattctgatcctgccaaatataatgcatacggccaaagtgcaatgaaggactggaagtcaaatcggatcgtaggctccctcgtccacggcgcagtcgcgccagaatccttcatgtcgcagtttgggacggtaatggagattttcttgcaatcccgtaacccgcaggcagccgctaatgccgcacaagctatcgccaatcaggtcggtttaggtcgtggcggcagcggcggcagcaccggcgaaaaaccgtataaatgcccggaatgcggcaaaagctttagccgcagcgggggttcacatcatcatcatcatcattaatgaaagggcgatatccagcacactggcggccgttactagtggatccggctgctaacaaagcccgaaaggaagctgagttggctgctgccaccgctgagcaataactagcataaccccttggggcctctaaacgggtcttgaggggttttttgctgaaaggaggaactatatccggagcgactcccacggcacgttggcaagctcg

SEQ ID NO: 105 - protein, 18 aa, Artificial Sequence
  bZif
TGEKPYKCPECGKSFSRS

SEQ ID NO: 106 - protein, 32 aa, Artificial Sequence
  ZF-QNK
TGEKPYKCPECGKSFSRSDHLSRHQRTHQNKK

SEQ ID NO: 107 - protein, 6 aa, Artificial Sequence
  Hexahistidine Tag
HHHHHH

SEQ ID NO: 108 - protein, 6 aa, Artificial Sequence
  Hexalysine Tag
KKKKKK

SEQ ID NO: 109 - protein, 394 aa, Artificial Sequence
  ttGBP1 (with signal peptide replaced with M)
MKLEIFSWWAGDEGPALEALIRLYKQKYPGVEVINATVTGGAGVNARAVLKTRMLGGDPPDTFQVHAGMELIGTWVVANRMEDLSALFRQEGWLQAFPKGLIDLISYKGGIWSVPVNIHRSNVMWYLPAKLKGWGVNPPRTWDKFLATAQTLKQKGLEAPLALGENWTQQHLWESVALAVLGPDDWNNLWNGKLKFTDPKAVRAWEVFGRVLDAANKDAAGLSWQQAVDRVVQGKAAFNIMGDWAAGYMTTTLKLKPGTDFAWAPSPGTQGVFMMLSDSFGLPKGAKNRQNAINWLRLVGSKEGQDTSNPLKGSIAARLDSDPSKYNAYGQSAMRDWRSNRIVGSLVHGAVAPESFMSQFGTVMEIFLQTRNPQAAANAAQAIADQVGLGRLGQ

SEQ ID NO: 110 - protein, 391 aa, Artificial Sequence
  tsGBP2  (with signal peptide replaced with M)
MKLEIFSWWAGDEGPALEALIRLYKQKYPGVEVINATVTGGAGVNAKAVLKTRMLGGDPPDTFQVHAGQELIGTWVVADRMEDLTSLFRQEGWLQAFPKGLIDLLSYKGGIWSVPVNIHRSNVMWYIPAKLKEWGVTPPKTWAEFLATAQTLKRKGLEAPLALGENWTQQHLWESVALATLGADGWNNLWSGKLKFTDPKAVAVWETFGKVLDAANKDAAGLSWQQAVDRVVQGKAAFNIMGDWAAGYMSTTLKLKPGTDFAWTPSPGTSGIFMMLSDSFGLPKGAKNRQNAINWLKLVGSKEGQDTFNPLKGSIAARLDSDPAKYNAYGQSAMKDWKSNRIVGSLVHGAVAPESFMSQFGTVMEIFLQSRNPQAAANAAQAIANQVGLGR

SEQ ID NO: 111 - protein, 390 aa, Artificial Sequence
  dmGBP3 (with signal peptide replaced with M)
MKLEIFSWWSGDEGPALEALVKLYKQKYPSVDVVNATVAGGAGTNAKAVLKTRMLGGDPPDSFQAHAGQELIGTWVVANRMEDLSSLFKSEGWTTKFPKDLLPLISSKGGIWSVPVNVHRSNVMWYIPANLKKWGVTAPKTWDQFLTTAKTLKTKNVTPLALGENWTQQHLWESVAVGTLGAQGWQNLWSGKLKFTDPKVVKVWDTFGKVLDATNKDASGLSWQQATDRVVNGQAAFNIMGDWAAGYLSTTKKLKPGTGFGWAPSPSTSGTFIFLADSFGLPKGAKDRAEALSWLKLLGSKQGQDTFNPLKGSIAARVDSDLSKYSTYSQSAAKDWKSNKIVGSLTHGAVAPESFTSTFGTVIDAFVASRNAQVAAATTQQLADKAGLGK

SEQ ID NO: 112 - protein, 393 aa, Artificial Sequence
  tnGBP4 (with signal peptide replaced with M)
MLEIFSWWTAGGEAEALEALIKVFNKYYPDVEVINATVAGGAGTNAKAVLKTRILGGNPPDSFQVHAGMELIDTYVIPGYMTPITNLLEQWGVMDKFPKGILEMASYEGEIYSIPVNVHRGNVVFYNKKIAEEIGMNEPPKTWDEFIMYLQKAKEKGYVGLALGDKNKWTALHLFETILLGVLGPNDYNGLWKGEVSFNDPRIRRAFEIMNKLLDYVNEDHAALAWQDATRLVYEGKALANVMGDWAEGYLKSVGWEPGKDFGWFAVPETQNAFMVVSDTFGLPKNAPHKENAVKWLKVVASVEGQDAFNPIKGSIPARLDADRSKYDIYLQWSMEDFATKALTPSIAHGSAAPEGFVTTLNDIINRFVTTRDIDSALEELLMAAEDEGYLVE

SEQ ID NO: 113 - protein, 390 aa, Artificial Sequence
  koGBP5 (with signal peptide replaced with M)
MLEIFSWWTGGGEEEGLLALFDVFHKYYPDVEIINATVAGGAGTNAKAVLKTRMLGGNPPDSFQVHGGMELIDTYVVTGMMEPITDLLEEWGIIDKFPEDILKIASYKGEVYSIPVNVHRGNVVFYNKAILEEVGIEKVPSTWPEFIEVLKKIKKAGYIPLALGDKNKWTATHLFEDILLSTLGPYNYNGLWNGRTSFEHQGVKEALEIFKELMNYVNPNHASLTWQDATLLVFEGKAAFNVMGDWAEGYLKTLGWTPGKEFGWMVVPGTKGSFMVVTDTFGLPKNAPHRENAIKWLKIISSVEGQDTFNPIKGSIPARIDADRSLYDDYLIWSMDDFATNALCPSIIHGSAAPEAFVTALNDTINMFITRKDVKKALKEIIYAAEDYLE

SEQ ID NO: 114 - protein, 386 aa, Artificial Sequence
  bhGBP6 (with signal peptide replaced with M)
MLEIFSWWTGAGEEDGLLALIELFEEKHPEIEVDNAAVAGGAGTNAKAVLTSRMQGNDPPGTFQVHGGAELNDSWVAAGQMDPLNDLFEAEGWADKFPEELIELVSKDGNIYSVPVNIHRGNVLWYNTEIFEEHGLEVPTTFEEFFDVADALQEAGVTPLALGDREPWAATHLFETVLLGTLGADDYNKLWSGEVGMDDPRVEEAAEIFIRMLDYVNEDHSSRNWQDASQLVAQGEAAMNVMGDWAKGYFVNDLNLAVKEDFGWAATPGTEGTFMVITDTFGLPTGVENPEVVKSFLAVLGSQEGQDAFNPLKGSIPARVDADVSKYDEYGQETIEDFKSAELSPSLAHGSAANEGFLTQVNQAINIFVTQKDVDSFVDSLKQYQP

SEQ ID NO: 115 - protein, 427 aa, Artificial Sequence
  smGBP7 (with signal peptide replaced with M)
MELVIYHWWTAGGEREAINAVFQVFKQKYPNIQIVENPVAGGAGSVMKSVIIGLLAAGTPPDTFQVHAGAELKEYVDAGYLAPIDDIWSKLGLDKVIPSTLQVMAKFNGHYYAVPIDVHRSNVLWYNPKIFNELGIINKFGDPRNWSVDTLLQVARYIKQQRPDIAPIALASRNKWPVTHLFEVLLANAGGPETYVKFFTGKFNYNDPNDPVVQTVKKVLTVMATMAKEGLFNSNHPELTWDQAAALVAEGKAAMFIHGDWVAGYYIANNYKYGKDWAAAPFPKNIFILLSDAFELPKNAPHPEAAKDWLMVVGSKEAQEKFNLIKGSIPARTDVSPKYPDPYRPETAEDFQKSTLIPSAVHGGIAKEAFMTDLHNILTSMLTAVSVGTPVDNAVNTALAQILQSVKTSGLASFWKGYTIDYFITKR

SEQ ID NO: 116 - protein, 391 aa, Artificial Sequence
  asGBP8 (with signal peptide replaced with M)
MKLEITSWWTSGSEADALNVLIDGVKAAKPGLSVDNAAVSGGGGANARQALAARLQAGSPPDAWQVHPAGQLKSYVDGGQVADLTDLWTEGDWASQMPKDVAEAQQVDGKYYTVPIGVHRGNVLWTNPAVLSKANVTIDADAGIDGLISSLEQVQASGTTPLALGDKDIFASSQLLESLIMSRAGADNWTKLFTSEYSFDAPEVKQALEDYKTILSFANKDHSAITWDEAAKKMADGEAAVNLMGDWAYGELLNAGKKPGTDFAWVAFPGKEDIFDYVGDGFSIPANNIPHAEAARAWLKTLMDPKIQTEFAAKKGSIPAVTSADISGLSEYQQEAAKSLASGAVVSSLAHAQAAGAEFAQTYADAVSTFNGSGNTDAFIASMTQAQKTQL

SEQ ID NO: 117 - protein, 309 aa, Artificial Sequence
  ecGGBP  (with signal peptide removed)
ADTRIGVTIYKYDDNFMSVVRKAIEQDAKAAPDVQLLMNDSQNDQSKQNDQIDVLLAKGVKALAINLVDPAAAGTVIEKARGQNVPVVFFNKEPSRKALDSYDKAYYVGTDSKESGIIQGDLIAKHWAANQGWDLNKDGQIQFVLLKGEPGHPDAEARTTYVIKELNDKGIKTEQLQLDTAMWDTAQAKDKMDAWLSGPNANKIEVVIANNDAMAMGAVEALKAHNKSSIPVFGVDALPEALALVKSGALAGTVLNDANNQAKATFDLAKNQADGKGAADGTNWKIDNKVVRVPYVGVDKDNLAEFSKK

SEQ ID NO: 118 - protein, 360 aa, Thermoanaerobacterium thermosaccharolyticum
MKKILTYLVLVVLVLSALLTGCGNSNTTSSNSSSSSSQQSDKTASSDSGKQLNIGVAIYKFDDTFMTGVRNAMTAEAQGKAKLNMVDSQNSQPTQNDQVDLFITKKMNALAINPVDRTAAGTIIDKAKQANIPVVFFNREPLPEDMKKWDKVYYVGAKAEQSGILQGQIMADYWKAHPEADKNHDGVMQYVMLMGQPGHQDAILRTQYSIQTVKDAGIKVQELAKDYANWDRVTAHDKMAAWLSSFGDKIEAVFCNNDDMALGAIEALKSAGYFTGNKYIPVVGVDATAPGIQAIKDGTLLGTVLNDAKNQAKATFNIAYELAQGITPTKDNIGYDITDGKYVWIPYKKITKDNISDAEQ

SEQ ID NO: 119 - protein, 332 aa, Salmonella typhimurium
MNKKVLTLSAVMASLLFGAHAHAADTRIGVTIYKYDDNFMSVVRKAIEKDGKSAPDVQLLMNDSQNDQSKQNDQIDVLLAKGVKALAINLVDPAAAGTVIEKARGQNVPVVFFNKEPSRKALDSYDKAYYVGTDSKESGVIQGDLIAKHWQANQGWDLNKDGKIQYVLLKGEPGHPDAEARTTYVVKELNDKGIQTEQLALDTAMWDTAQAKDKMDAWLSGPNANKIEVVIANNDAMAMGAVEALKAHNKSSIPVFGVDALPEALALVKSGAMAGTVLNDANNQAKATFDLAKNLAEGKGAADGTSWKIENKIVRVPYVGVDKDNLSEFTQK

SEQ ID NO: 120 - protein, 356 aa, Caldicellulosiruptor hydrothermalis
MFNKKKFWVVLVSMVLIISLVLVGCGKKSTNDSSNGTSEENKPYIGVAIYKFDDTFMTGVRNAIAKEGEGKAKLDFVDCQNSQSTQNDKIDLFITKKVDALAINPVDRTAAGVLIDKAKQANIPVVFFNREPLPEDMKKWDKVYYVGAKAEQSGTLQGEIMAEYWKSHPEADKNHNGIMEYVMITGEPGHQDAILRTEYSIKAVEAAGIKTKALAQDTAMWDRVKGQEKMQAFLASFGDRIEAVFCNNDDMALGAIEALKAAGYFKNGKYIPVVGVDATTPGLQALEEGTLLGTVLNDAKAQGKATFNLAYVLAKGEKPTKENVGFDITDGKYIWVPYQKVTKDNLEEMKKYVNEQ

SEQ ID NO: 121 - protein, 356 aa, Caldicellulosiruptor obsidiansis
MLNKKKFWVVLVSIVLAISLVLVGCGKKSTNENSGGTSEDNKPYIGVAIYKFDDTFMTGVRNAIAKEGEGKAKLDFVDCQNSQSTQNDKIDLFITKKVDALAINPVDRTAAGVLIDKAKQANIPVVFFNREPLPEDMKKWDKVYYVGAKAEQSGTLQGEIMAEYWKSHPEADKNHDGIMQYVMITGEPGHQDAILRTEYSIKAVEAAGIRVKCLAQDTAMWDRVKGQEKMQAFLASFGDKIEAVFCNNDDMALGAIEALKAAGYFKDGKYVPVVGVDATTPGLQALEEGTLLGTVLNDAKAQGKATFNLAYVLAKGEKPTKENVGFEITDGKYIWVPYQKVTKDNLEEMKKYVNEQ

SEQ ID NO: 122 - protein, 350 aa, Paenibacillus sp.
MKKKWLFVLMAGMMLTTAACNNGGSSSTGSDSTGGDAVGGSTPQVGVAIYKFDDTFMTGVRNAMSDAANGVAKLDIVDSQNAQPTQNEKIDLFISKKYSSMIINPVDRTAAGVIIDKAKTANTPVVFLNREPIAEDMNKWDKVYYVGAKAEESGTISGQLIVDYWKANPKADKNGDGKLQYVLLQGEPGHQDAELRTKFSVQAIQDAGIEVEALAVDTAMWDRVKGQEKMQTFLASHGDKIEAVLANNDDMALGAIEALKAAGYFSGDKYMPVVGVDATAPAVQALEDGTLLGTVLNDAKSQGKASVAIAAALSKGEAPNKENTGFDITDGKYVWIAYKKITKDNIADAK

SEQ ID NO: 123 - protein, 354 aa, Clostridium saccharolyticum
MKRLRKGIFLFFFIVWTAFPLYGCAPMEQKKDVGESATSEAGTEGVPEETGPKIGVSIYRYDDTFMKLYRQELKQYLEETYHAEVIMRNAGGDQKEQDKQVNQFISDGCDGIIVNPVEIPAAQELADACSRAGIPLVFINREPKEEEQKRWREKQMAVSCVGTDSRQAGTYQGEIILETLNKGDFNGDGVVSYVMLMGEKGNEDSQYRTEYSIKALEEGGMKTEELFSGNGNWNKDEGKKLAKQALASWGNRIEVFFCNNDSMANGALEAVEEAGRIPGKDIYLVGVDALQDTVTYIKEGRMTGTVLNDHEGQSQMAADTLKKMIDGESVETRYQVDYIKVTAISTFQTLKGED

SEQ ID NO: 124 - protein, 354 aa, Butyrivibrio proteoclasticus
MKKKMICYMIIAALALSLMAGCSNTQESEPVQESVAYSSYSDAKVGVCIYQKSDNFMSLFSSELVKYLVSRGFSKDNIILYDSNNDENVQLSQVEELIASGINALIINPVNSSVAHSITDMASASNIPLVYINREPSGDEENRWEMYQLNVCYVGCDARQSGIYQGEILLSLGKNKLDHNGDGKIQYFMIEGAPENIDAGYRTLYSVSALQNSEMEMDCLLDEVGNWDETTASLLVSKGIQNGLKPEVIICNNDAMALGAIKAAEKSGLVPGEDVYIVGVDALPEAIEMIKAGKLAGTVYNDYVLQSHKSADAVINYLKGIDNEHYIGCDYVKVDIDNAESIAGLTNTDEEDID

SEQ ID NO: 125 - protein, 383 aa, Roseburia intestinalis
MKRKVVSVILATAMVASMVAGCGGSNNASTNNAGTTTDAAASDASSDTSNDAAATEAADAGDAAADAATDADASLADKKVGVCIYQFSDNFMTLFRTELENYLVEKGFSKDNITIVDGANDQATQTGQIDNFITEGVDVLIINPVNSSSAATITDKVVAAGIPLVYINREPDEEEQKRWSDNNWDVTYVGCDARQSGTFQGEMISDLGLDTVDLNGNGKIDYVMVEGDPENVDAQYRTEYSVKALEDAGLEVNCLSDQVGNWQQDQAQQIVANALGQYGNDVEVVFCNNDAMALGALQAIQSAGRTVGTDIYLVGVDALSEALEDVLAGTMTGTVFNDHFSQSHSAADAAINYITGAGNDHYIGCDYVKVTKDNAQDVLDMVK

SEQ ID NO: 126 - protein, 350 aa, Faecalibacterium prausnitzii
MKMISRRDFLKASAVVGATAAMTACGGSSSTSTAASSVASSTAASAAATNGSANIGVCIYQFADNFMTLYRADLEGYLKDMGYSVTIMDGKNDQNTQTEQINTFLQQGVDVLVINPVQTTSAQTIVDTVSPSGTPIVFINREPEESVLDSYKGKCCYVGADARQSGTYQGELILATDTQGDINGDGKITYIMCKGDPENIDAQYRTEYSIKALTDAGKEVECLYEYLDNWDQTTAQQDVANALSQYGEKIEVVFCNNDAMALGALQSIQQAGRTVGKDVYLVGVDALVEAVQNVVDGNMTGTVLNDDVGQATKAAEATKLFVEGKDVEKYYWVDYVKVTKDNASQYLKED

SEQ ID NO: 127 - protein, 338 aa, Clostridium ljungdahlii
MIVKKCMKSIAVTGLLTIILGTGCSNSLSSNKNEPVIGFVAYEFNNTWITELKNEIYKVSSGKARVDIWNGDNIQTVENDKINLFINRKVNVLDINPVDVNAAGQIIEKCKKANIPTVFVNRQPKKEDMEKWNKVYYVGAKAEQSGTIQGQMLVNYFKGHPTQDGTIRYIMLKGETRNQDAEKRTQYSIKALKDSGFKVQKVAEDTAMWDRTKAQEKMTSFISSYGPNFDCVIANNDDMALGAVDALKAAGYFNGGKYVPVVGVDATAPAVKAVEDGTLFGTVLNDAAKQGDAAFDLSYILSKGKIPDESNFKYKVTDGKYIWIDYKMITKENVQDAK

SEQ ID NO: 128 - protein, 336 aa, Clostridium autoethanogenum
MKKCMKSIAVTGLLTIILGTGCSNSLSSNKNEPVIGFVAYEFNNTWITELKNEMYKVSNGKARVDIWNGNNIQTVENDKISLFINRKVDVLDINPVDVNAAGQIIEKCKKANIPTVFVNRQPKKEDVEKWNKVYYVGAKAEQSGTIQGQMLVNYFKGHPTQDGTIRYIMLKGEMRNQDAEKRTQYSIKALEDSGFKVQKVAEDTAMWDRTKAQEKMTSFISSYGPNFDCVIANNDDMALGAVDALKAAGYFNGGKYVPVVGVDATAPAVKAVEDGTLFGTVLNDAAKQGDAAFDLSYILSKGKIPDESNFKYKITDGKYIWIDYKMITKENVQDAK

SEQ ID NO: 129 - protein, 367 aa, Roseburia intestinalis
MCGAEKVRHMLMGEQVLKKWKKSKKMTVAFGGILVMSVVIGGCGGREDAKKSIKIGISVYDQYDTFVSEMMKDFNDYATKKEEETGVAINIDTYNASASQSTQNSQVENMITEGCDVICVNLVDRTDPTAIIDLAEKNNIPVIFFNRELVEEDLERWTRLYYVGAQAFESGIMQGELAAEAFLTDQSLDKNGDGIFQYVVLEGEAGHQDAIVRTEYSVSTMIDSGVEVEKLGYAIANWNRAQAQTKMAQLMSQFGDSIELVIANNDDMALGAIDALKASGLTKDEWPAVIGIDGTDVGLEAVKNKEMIGTVYNDKEGQADAMLNLAYELSTGSDLSDLNLIDGKYIRLPYARVTCDDVDSYMEGDTE

SEQ ID NO: 130 - protein, 360 aa, Erysipelothrix rhusiopathiae
MKKLSKLILVSLLALTLFGCSSKGGAEGNANEGGKTYNIGVAIYKFDDNFMTLYREELASYFKEVGEKDGNTYKLDIQDGKQDQANQTEQINNFIAQGKDLIIANMVDPTAAGSIINSAKAKEIPVVFINREPETQELEIWPGKTTYVGADATQSGTIQGYMIANLENKGDIDGDGSVSYITLMGDPANVDAKQRTEYSVKGLEEKGVKTNALAQPYQANWDTAKGQEFTANALEQFGNKLEVVFANNDGMAVGAVTAIEAAGRKVGEDIFVVGVDAIPDAIELLKGGKLTGTVLNDHFNQSHTAVDVALELLQGKDVSAYYWHDYVGVTKPEEAELKRAEARKETVEEAVKRYAERDAQ

SEQ ID NO: 131 - protein, 338 aa, Eubacterium rectale
MMILCFALILSFVSCSNTRVDEKKQIYIGVTCYDQKDTFIGELIETFKKECASLDTDKYDISMTIMDAAGSQRAQDDQVQEMIEDGCNVLCINLADRTDLSHIINAAMEKDIPIIFFNREPVDEDLNRWDKLYYVGAKAKQSGQMQGELIADYIKNNPGVDKNGDGRIQYVILEGEMGHQDAIVRTESVTESMKNNGLQIEKLSCQIANWNRAQAQNRMTQLIGQYKNSIELVIANNDAMALGAIDAYEKLGVTESNVPAFFGVDGTDDGLEAVQQSKLAATVYNDKEGQAMAMAQLAYLAATGGSMKNIKFEDKKYVYLPYEKVTPDNVNEFVKDEQ

SEQ ID NO: 132 - protein, 9 aa, Artificial Sequence
  GGSHHHHHH motif
GGSHHHHHH

SEQ ID NO: 133 - protein, 7 aa, Artificial Sequence
  Conserved sequence
  misc_feature (3)..(6): Xaa can be any naturally occurring amino acid
WWXXXXE

SEQ ID NO: 134 - protein, 6 aa, Artificial Sequence
  Conserved sequence
  misc_feature (3)..(5): Xaa can be any naturally occurring amino acid
WWXXXE

SEQ ID NO: 135 - protein, 5 aa, Artificial Sequence
  Conserved sequence
  misc_feature (1)..(1): Xaa can be any naturally occurring amino acid
  misc_feature (4)..(4): Xaa can be any naturally occurring amino acid
XQVXH

SEQ ID NO: 136 - protein, 5 aa, Artificial Sequence
  Conserved sequence
  misc_feature (3)..(3): Xaa can be any naturally occurring amino acid
HRXNV

SEQ ID NO: 137 - protein, 4 aa, Artificial Sequence
  Conserved sequence
  misc_feature (4)..(4): Xaa can be any naturally occurring amino acid
GDWX

SEQ ID NO: 138 - protein, 6 aa, Artificial Sequence
  Conserved sequence
  misc_feature (2)..(2): Xaa can be any naturally occurring amino acid
  misc_feature (4)..(5): Xaa can be any naturally occurring amino acid
DXFXXP

SEQ ID NO: 139 - protein, 6 aa, Artificial Sequence
  Conserved sequence
  misc_feature (5)..(5): Xaa can be any naturally occurring amino acid
KGSIXA

SEQ ID NO: 140 - protein, 109 aa, Escherichia coli
MSDKIIHLTDDSFDTDVLKADGAILVDFWAEWCGPCKMIAPILDEIADEYQGKLTVAKLNIDQNPGTAPKYGIRGIPTLLLFKNGEVAATKVGALSKGQLKEFLDANLA

SEQ ID NO: 141 - protein, 118 aa, Artificial Sequence
  Adaptor0
MSAKIIHLTDDSFDTDVLKADGAILVAFWAEWCGPCKMIAPILDEIADEYQGKLTVAMLNIDQNPGTAPKYGIRGIPTLLLFKNGEVAATKVGALSKGQLKEFLDANLAGGSHHHHHH

SEQ ID NO: 142 - protein, 118 aa, Artificial Sequence
  Adaptor1.0
MSAKIIHLTDDSFDTDVLKADGAILVAFWAEWCGPCKMIAPILDEIADEYQGKLTVAMLNIDQNPGTAPKYGICGIPTLLLFKNGEVAATKVGALSKGQLKEFLDANLAGGSHHHHHH

SEQ ID NO: 143 - protein, 118 aa, Artificial Sequence; identical to SEQ ID NO: 142
  Adaptor2.0a

SEQ ID NO: 144 - protein, 118 aa, Artificial Sequence; identical to SEQ ID NO: 142
  Adaptor2.0b

SEQ ID NO: 145 - protein, 118 aa, Artificial Sequence
  Adaptor3.0
MSAKIIHLTDCSFDTDVLKADGAILVAFWAEWCGPCKMIAPILDEIADEYQGKLTVAMLNIDQNPGTAPKYGIRGIPTLLLFKNGEVAATKVGALSKGQLKEFLDANLAGGSHHHHHH

SEQ ID NO: 146 - protein, 118 aa, Artificial Sequence
  Adaptor4.0
MSAKIIHLTDDSFDCDVLKADGAILVAFWAEWCGPCKMIAPILDEIADEYQGKLTVAMLNIDQNPGTAPKYGIRGIPTLLLFKNGEVAATKVGALSKGQLKEFLDANLAGGSHHHHHH

SEQ ID NO: 147 - protein, 118 aa, Artificial Sequence
  Adaptor5.0
MSAKIIHLTDDSFDTDVLKACGAILVAFWAEWCGPCKMIAPILDEIADEYQGKLTVAMLNIDQNPGTAPKYGIRGIPTLLLFKNGEVAATKVGALSKGQLKEFLDANLAGGSHHHHHH

SEQ ID NO: 148 - protein, 118 aa, Artificial Sequence
  Adaptor6.0
MSAKIIHLTDDSFDTDVLKADGAILVAFWAECCGPCKMIAPILDEIADEYQGKLTVAMLNIDQNPGTAPKYGIRGIPTLLLFKNGEVAATKVGALSKGQLKEFLDANLAGGSHHHHHH

SEQ ID NO: 149 - protein, 118 aa, Artificial Sequence
  Adaptor7.0
MSAKIIHLTDDSFDTDVLKADGAILVAFWAEWCGPCKCIAPILDEIADEYQGKLTVAMLNIDQNPGTAPKYGIRGIPTLLLFKNGEVAATKVGALSKGQLKEFLDANLAGGSHHHHHH

SEQ ID NO: 150 - protein, 118 aa, Artificial Sequence
  Adaptor8.0
MSAKIIHLTDDSFDTDVLKADGAILVAFWAEWCGPCKMIAPILDCIADEYQGKLTVAMLNIDQNPGTAPKYGIRGIPTLLLFKNGEVAATKVGALSKGQLKEFLDANLAGGSHHHHHH

SEQ ID NO: 151 - protein, 118 aa, Artificial Sequence
  Adaptor9.0
MSAKIIHLTDDSFDTDVLKADGAILVAFWAEWCGPCKMIAPILDEIADEYQGCLTVAMLNIDQNPGTAPKYGIRGIPTLLLFKNGEVAATKVGALSKGQLKEFLDANLAGGSHHHHHH

SEQ ID NO: 152 - protein, 118 aa, Artificial Sequence
  Adaptor10.0
MSAKIIHLTDDSFDTDVLKADGAILVAFWAEWCGPCKMIAPILDEIADEYQGKLTVAMLNIDCNPGTAPKYGIRGIPTLLLFKNGEVAATKVGALSKGQLKEFLDANLAGGSHHHHHH

SEQ ID NO: 153 - protein, 118 aa, Artificial Sequence
  Adaptor11.0
MSAKIIHLTDDSFDTDVLKADGAILVAFWAEWCGPCKMIAPILDEIADEYQGKLTVAMLNIDQNPGTAPKCGIRGIPTLLLFKNGEVAATKVGALSKGQLKEFLDANLAGGSHHHHHH

SEQ ID NO: 154 - protein, 118 aa, Artificial Sequence
  Adaptor12.0
MSAKIIHLTDDSFDTDVLKADGAILVAFWAEWCGPCKMIAPILDEIADEYQGKLTVAMLNIDQNPGTAPKYGIRGIPTLLLFKNGECAATKVGALSKGQLKEFLDANLAGGSHHHHHH

SEQ ID NO: 155 - protein, 118 aa, Artificial Sequence
  Adaptor13.0
MSAKIIHLTDDSFDTDVLKADGAILVAFWAEWCGPCKMIAPILDEIADEYQGKLTVAMLNIDQNPGTAPKYGIRGIPTLLLFKNGEVAATKCGALSKGQLKEFLDANLAGGSHHHHHH

SEQ ID NO: 156 - protein, 118 aa, Artificial Sequence
  Adaptor14.0
MSAKIIHLTDDSFDTDVLKADGAILVAFWAEWCGPCKMIAPILDEIADEYQGKLTVAMLNIDQNPGTAPKYGIRGIPTLLLFKNGEVAATKVGALSCGQLKEFLDANLAGGSHHHHHH

SEQ ID NO: 157 - protein, 118 aa, Artificial Sequence
  Adaptor15.0
MSAKIIHLTDDSFDTDVLKADGAILVAFWAEWCGPCKMIAPILDEIADEYQGKLTVAMLNIDQNPGTAPKYGIRGIPTLLLFKNGEVAATKVGALSKGCLKEFLDANLAGGSHHHHHH

SEQ ID NO: 158 - protein, 118 aa, Artificial Sequence
  Adaptor16.0
MSAKIIHLTDDSFDTDVLKADGAILVAFWAEWCGPCKMIAPILDEIADEYQGKLTVAMLNIDQNPGTAPKYGIRGIPTLLLFKNGEVAATKVGALSKGQLKEFLDCNLAGGSHHHHHH